European Patent Application EP 4 434 542 A1, published September 25, 2024. Title: SARS-CoV-2 IMMUNOGENIC POLYPEPTIDES AND USES THEREOF. Applicant: Fundacio Privada Institut de Recerca de la SIDA - Caixa. Application EP. The sequence listing filed with the application follows.

SEQUENCE LISTING (123 sequences)

SEQ ID NO: 1 - protein, 1188 aa, synthetic construct
VNLTTRTQLPPAYTNSFTRGVYYPDKVFRSSVLHSTQDLFLPFFSNVTWFHAIHVSGTNGTKRFDNPVLPFNDGVYFASTEKSNIIRGWIFGTTLDSKTQSLLIVNNATNVVIKVCEFQFCNDPFLGVYYHKNNKSWMESEFRVYSSANNCTFEYVSQPFLMDLEGKQGNFKNLREFVFKNIDGYFKIYSKHTPINLVRDLPQGFSALEPLVDLPIGINITRFQTLLALHRSYLTPGDSSSGWTAGAAAYYVGYLQPRTFLLKYNENGTITDAVDCALDPLSETKCTLKSFTVEKGIYQTSNFRVQPTESIVRFPNITNLCPFGEVFNATRFASVYAWNRKRISNCVADYSVLYNSASFSTFKCYGVSPTKLNDLCFTNVYADSFVIRGDEVRQIAPGQTGKIADYNYKLPDDFTGCVIAWNSNNLDSKVGGNYNYLYRLFRKSNLKPFERDISTEIYQAGSTPCNGVEGFNCYFPLQSYGFQPTNGVGYQPYRVVVLSFELLHAPATVCGPKKSTNLVKNKCVNFNFNGLTGTGVLTESNKKFLPFQQFGRDIADTTDAVRDPQTLEILDITPCSFGGVSVITPGTNTSNQVAVLYQDVNCTEVPVAIHADQLTPTWRVYSTGSNVFQTRAGCLIGAEHVNNSYECDIPIGAGICASYQTQTNSPVASQSIIAYTMSLGAENSVAYSNNSIAIPTNFTISVTTEILPVSMTKTSVDCTMYICGDSTECSNLLLQYGSFCTQLNRALTGIAVEQDKNTQEVFAQVKQIYKTPPIKDFGGFNFSQILPDPSKPSKRSFIEDLLFNKVTLADAGFIKQYGDCLGDIAARDLICAQKFNGLTVLPPLLTDEMIAQYTSALLAGTITSGWTFGAGAALQIPFAMQMAYRFNGIGVTQNVLYENQKLIANQFNSAIGKIQDSLSSTASALGKLQDVVNQNAQALNTLVKQLSSNFGAISSVLNDILSRLDKHEAEVQIDRLITGRLQSLQTYVTQQLIRAAEIRASANLAATKMSECVLGQSKRVDFCGKGYHLMSFPQSAPHGVVFLHVTYVPAQEKNFTTAPAICHDGKAHFPREGVFVSNGTHWFVTQRNFYEPQIITTDNTFVSGNCDVVIGIVNNTVYDPLQPELDSFKEELDKYFKNHTSPDVDLGDISGINASVVNIQKEIDRLNEVAKNLNESLIDLQELGKYEQ

SEQ ID NO: 2 - protein, 1188 aa, synthetic construct
VNLTTRTQLPPAYTNSFTRGVYYPDKVFRSSVLHSTQDLFLPFFSNVTWFHAIHVSGTNGTKRFDNPVLPFNDGVYFASTEKSNIIRGWIFGTTLDSKTQSLLIVNNATNVVIKVCEFQFCNDPFLGVYYHKNNKSWMESEFRVYSSANNCTFEYVSQPFLMDLEGKQGNFKNLREFVFKNIDGYFKIYSKHTPINLVRDLPQGFSALEPLVDLPIGINITRFQTLLALHRSYLTPGDSSSGWTAGAAAYYVGYLQPRTFLLKYNENGTITDAVDCALDPLSETKCTLKSFTVEKGIYQTSNFRVQPTESIVRFPNITNLCPFGEVFNATRFASVYAWNRKRISNCVADYSVLYNSASFSTFKCYGVSPTKLNDLCFTNVYADSFVIRGDEVRQIAPGQTGKIADYNYKLPDDFTGCVIAWNSNNLDSKVGGNYNYLYRLFRKSNLKPFERDISTEIYQAGSTPCNGVEGFNCYFPLQSYGFQPTNGVGYQPYRVVVLSFELLHAPATVCGPKKSTNLVKNKCVNFNFNGLTGTGVLTESNKKFLPFQQFGRDIADTTDAVRDPQTLEILDITPCSFGGVSVITPGTNTSNQVAVLYQDVNCTEVPVAIHADQLTPTWRVYSTGSNVFQTRAGCLIGAEHVNNSYECDIPIGAGICASYQTQTNSPVASQSIIAYTMSLGAENSVAYSNNSIAIPTNFTISVTTEILPVSMTKTSVDCTMYICGDSTECSNLLLQYGSFCTQLNRALTGIAVEQDKNTQEVFAQVKQIYKTPPIKDFGGFNFSQILPDPSKPSKRSFIEDLLFNKVTLADAGFIKQYGDCLGDIAARDLICAQKFNGLTVLPPLLTDEMIAQYTSALLAGTITSGWTFGAGAALQIPFAMQMAYRFNGIGVTQNVLYENQKLIANQFNSAIGKIQDSLSSTASALGKLQDVVNQNAQALNTLVKQLSSNFGAISSVLNDILSRLLKVEAEVQIDRLITGRLQSLQTYVTQQLIRAAEIRASANLAATKMSECVLGQSKRVDFCGKGYHLMSFPQSAPHGVVFLHVTYVPAQEKNFTTAPAICHDGKAHFPREGVFVSNGTHWFVTQRNFYEPQIITTDNTFVSGNCDVVIGIVNNTVYDPLQPELDSFKEELDKYFKNHTSPDVDLGDISGINASVVNIQKEIDRLNEVAKNLNESLIDLQELGKYEQ

SEQ ID NO: 3 - protein, 1188 aa, synthetic construct
VNLTTRTQLPPAYTNSFTRGVYYPDKVFRSSVLHSTQDLFLPFFSNVTWFHAIHVSGTNGTKRFDNPVLPFNDGVYFASTEKSNIIRGWIFGTTLDSKTQSLLIVNNATNVVIKVCEFQFCNDPFLGVYYHKNNKSWMESEFRVYSSANNCTFEYVSQPFLMDLEGKQGNFKNLREFVFKNIDGYFKIYSKHTPINLVRDLPQGFSALEPLVDLPIGINITRFQTLLALHRSYLTPGDSSSGWTAGAAAYYVGYLQPRTFLLKYNENGTITDAVDCALDPLSETKCTLKSFTVEKGIYQTSNFRVQPTESIVRFPNITNLCPFGEVFNATRFASVYAWNRKRISNCVADYSVLYNSASFSTFKCYGVSPTKLNDLCFTNVYADSFVIRGDEVRQIAPGQTGKIADYNYKLPDDFTGCVIAWNSNNLDSKVGGNYNYLYRLFRKSNLKPFERDISTEIYQAGSTPCNGVEGFNCYFPLQSYGFQPTNGVGYQPYRVVVLSFELLHAPATVCGPKKSTNLVKNKCVNFNFNGLTGTGVLTESNKKFLPFQQFGRDIADTTDAVRDPQTLEILDITPCSFGGVSVITPGTNTSNQVAVLYQDVNCTEVPVAIHADQLTPTWRVYSTGSNVFQTRAGCLIGAEHVNNSYECDIPIGAGICASYQTQTNSPVASQSIIAYTMSLGAENSVAYSNNSIAIPTNFTISVTTEILPVSMTKTSVDCTMYICGDSTECSNLLLQYGSFCTQLNRALTGIAVEQDKNTQEVFAQVKQIYKTPPIKDFGGFNFSQILPDPSKPSKRSFIEDLLFNKVTLADAGFIKQYGDCLGDIAARDLICAQKFNGLTVLPPLLTDEMIAQYTSALLAGTITSGWTFGAGAALQIPFAMQMAYRFNGIGVTQNVLYENQKLIANQFNSAIGKIQDSLSSTASALGKLQDVVNQNAQALNTLVKQLSSNFGAISSVLNDILFRLDKVEAEVQIDRLITGRLQSLQTYVTQQLIRAAEIRASANLAATKMSECVLGQSKRVDFCGKGYHLMSFPQSAPHGVVFLHVTYVPAQEKNFTTAPAICHDGKAHFPREGVFVSNGTHWFVTQRNFYEPQIITTDNTFVSGNCDVVIGIVNNTVYDPLQPELDSFKEELDKYFKNHTSPDVDLGDISGINASVVNIQKEIDRLNEVAKNLNESLIDLQELGKYEQ

SEQ ID NO: 4 - protein, 1188 aa, synthetic construct
VNLTTRTQLPPAYTNSFTRGVYYPDKVFRSSVLHSTQDLFLPFFSNVTWFHAIHVSGTNGTKRFDNPVLPFNDGVYFASTEKSNIIRGWIFGTTLDSKTQSLLIVNNATNVVIKVCEFQFCNDPFLGVYYHKNNKSWMESEFRVYSSANNCTFEYVSQPFLMDLEGKQGNFKNLREFVFKNIDGYFKIYSKHTPINLVRDLPQGFSALEPLVDLPIGINITRFQTLLALHRSYLTPGDSSSGWTAGAAAYYVGYLQPRTFLLKYNENGTITDAVDCALDPLSETKCTLKSFTVEKGIYQTSNFRVQPTESIVRFPNITNLCPFGEVFNATRFASVYAWNRKRISNCVADYSVLYNSASFSTFKCYGVSPTKLNDLCFTNVYADSFVIRGDEVRQIAPGQTGKIADYNYKLPDDFTGCVIAWNSNNLDSKVGGNYNYLYRLFRKSNLKPFERDISTEIYQAGSTPCNGVEGFNCYFPLQSYGFQPTNGVGYQPYRVVVLSFEYLHAPATVCGPKKSTNLVKNKCVNFNFNGLTGTGVLTESNKKFLPFQQFGRDIADTTDAVRDPQTLEILDITPCSFGGVSVITPGTNTSNQVAVLYQDVNCTEVPVAIHADQLTPTWRVYSTGSNVFQTRAGCLIGAEHVNNSYECDIPIGAGICASYQTQTNSPVASQSIIAYTMSLGAENSVAYSNNSIAIPTNFTISVTTEILPVSMTKTSVDCTMYICGDSTECSNLLLQYGSFCTQLNRALTGIAVEQDKNTQEVFAQVKQIYKTPPIKDFGGFNFSQILPDPSKPSKRSFIEDLLFNKVTLADAGFIKQYGDCLGDIAARDLICAQKFNGLTVLPPLLTDEMIAQYTSALLAGTITSGWTFGAGAALQIPFAMQMAYRFNGIGVTQNVLYENQKLIANQFNSAIGKIQDSLSSTASALGKLQDVVNQNAQALNTLVKQLSSNFGAISSVLNDILSRLDKVEAEVQIDRLITGRLQSLQTYVTQQLIRAAEIRASANLAATKMSECVLGQSKRVDFCGKGYHLMSFPQSAPHGVVFLHVTYVPAQEKNFTTAPAICHDGKAHFPREGVFVSNGTHWFVTQRNFYEPQIITTDNTFVSGNCDVVIGIVNNTVYDPLQPELDSFKEELDKYFKNHTSPDVDLGDISGINASVVNIQKEIDRLNEVAKNLNESLIDLQELGKYEQ

SEQ ID NO: 5 - protein, 1188 aa, synthetic construct
VNLTTRTQLPPAYTNSFTRGVYYPDKVFRSSVLHSTQDLFLPFFSNVTWFHAIHVSGTNGTKRFDNPVLPFNDGVYFASTEKSNIIRGWIFGTTLDSKTQSLLIVNNATNVVIKVCEFQFCNDPFLGVYYHKNNKSWMESEFRVYSSANNCTFEYVSQPFLMDLEGKQGNFKNLREFVFKNIDGYFKIYSKHTPINLVRDLPQGFSALEPLVDLPIGINITRFQTLLALHRSYLTPGDSSSGWTAGAAAYYVGYLQPRTFLLKYNENGTITDAVDCALDPLSETKCTLKSFTVEKGIYQTSNFRVQPTESIVRFPNITNLCPFGEVFNATRFASVYAWNRKRISNCVADYSVLYNSASFSTFKCYGVSPTKLNDLCFTNVYADSFVIRGDEVRQIAPGQTRKIADYNYKLPDDFTGCVIAWNSNNLDSKVGGNYNYLYRLFRKSNLKPFERDISTEIYQAGSTPCNGVEGFNCYFPLQSYGFQPTNGVGYQPYRVVVLSFELLHAPATVCGPKKSTNLVKNKCVNFNFNGLTGTGVLTESNKKFLPFQQFGRDIADTTDAVRDPQTLEILDITPCSFGGVSVITPGTNTSNQVAVLYQDVNCTEVPVAIHADQLTPTWRVYSTGSNVFQTRAGCLIGAEHVNNSYECDIPIGAGICASYQTQTNSPVASQSIIAYTMSLGAENSVAYSNNSIAIPTNFTISVTTEILPVSMTKTSVDCTMYICGDSTECSNLLLQYGSFCTQLNRALTGIAVEQDKNTQEVFAQVKQIYKTPPIKDFGGFNFSQILPDPSKPSKRSFIEDLLFNKVTLADAGFIKQYGDCLGDIAARDLICAQKFNGLTVLPPLLTDEMIAQYTSALLAGTITSGWTFGAGAALQIPFAMQMAYRFNGIGVTQNVLYENQKLIANQFNSAIGKIQDSLSSTASALGKLQDVVNQNAQALNTLVKQLSSNFGAISSVLNDILSRLDKVEAEVQIDRLITGRLQSLQTYVTQQLIRAAEIRASANLAATKMSECVLGQSKRVDFCGKGYHLMSFPQSAPHGVVFLHVTYVPAQEKNFTTAPAICHDGKAHFPREGVFVSNGTHWFVTQRNFYEPQIITTDNTFVSGNCDVVIGIVNNTVYDPLQPELDSFKEELDKYFKNHTSPDVDLGDISGINASVVNIQKEIDRLNEVAKNLNESLIDLQELGKYEQ

SEQ ID NO: 6 - protein, 1188 aa, synthetic construct
VNLTTRTQLPPAYTNSFTRGVYYPDKVFRSSVLHSTQDLFLPFFSNVTWFHAIHVSGTNGTKRFDNPVLPFNDGVYFASTEKSNIIRGWIFGTTLDSKTQSLLIVNNATNVVIKVCEFQFCNDPFLGVYYHKNNKSWMESEFRVYSSANNCTFEYVSQPFLMDLEGKQGNFKNLREFVFKNIDGYFKIYSKHTPINLVRDLPQGFSALEPLVDLPIGINITRFQTLLALHRSYLTPGDSSSGWTAGAAAYYVGYLQPRTFLLKYNENGTITDAVDCALDPLSETKCTLKSFTVEKGIYQTSNFRVQPTESIVRFPNITNLCPFGEVFNATRFASVYAWNRKRISNCVADYSVLYNSASFSTFKCYGVSPTRLNDLCFTNVYADSFVIRGDEVRQIAPGQTGKIADYNYKLPDDFTGCVIAWNSNNLDSKVGGNYNYLYRLFRKSNLKPFERDISTEIYQAGSTPCNGVEGFNCYFPLQSYGFQPTNGVGYQPYRVVVLSFELLHAPATVCGPKKSTNLVKNKCVNFNFNGLTGTGVLTESNKKFLPFQQFGRDIADTTDAVRDPQTLEILDITPCSFGGVSVITPGTNTSNQVAVLYQDVNCTEVPVAIHADQLTPTWRVYSTGSNVFQTRAGCLIGAEHVNNSYECDIPIGAGICASYQTQTNSPVASQSIIAYTMSLGAENSVAYSNNSIAIPTNFTISVTTEILPVSMTKTSVDCTMYICGDSTECSNLLLQYGSFCTQLNRALTGIAVEQDKNTQEVFAQVKQIYKTPPIKDFGGFNFSQILPDPSKPSKRSFIEDLLFNKVTLADAGFIKQYGDCLGDIAARDLICAQKFNGLTVLPPLLTDEMIAQYTSALLAGTITSGWTFGAGAALQIPFAMQMAYRFNGIGVTQNVLYENQKLIANQFNSAIGKIQDSLSSTASALGKLQDVVNQNAQALNTLVKQLSSNFGAISSVLNDILSRLDKVEAEVQIDRLITGRLQSLQTYVTQQLIRAAEIRASANLAATKMSECVLGQSKRVDFCGKGYHLMSFPQSAPHGVVFLHVTYVPAQEKNFTTAPAICHDGKAHFPREGVFVSNGTHWFVTQRNFYEPQIITTDNTFVSGNCDVVIGIVNNTVYDPLQPELDSFKEELDKYFKNHTSPDVDLGDISGINASVVNIQKEIDRLNEVAKNLNESLIDLQELGKYEQ

SEQ ID NO: 7 - protein, 1188 aa, synthetic construct
VNLTTRTQLPPAYTNSFTRGVYYPDKVFRSSVLHSTQDLFLPFFSNVTWFHAIHVSGTNGTKRFDNPVLPFNDGVYFASTEKSNIIRGWIFGTTLDSKTQSLLIVNNATNVVIKVCEFQFCNDPFLGVYYHKNNKSWMESEFRVYSSANNCTFEYVSQPFLMDLEGKQGNFKNLREFVFKNIDGYFKIYSKHTPINLVRDLPQGFSALEPLVDLPIGINITRFQTLLALHRSYLTPGDSSSGWTAGAAAYYVGYLQPRTFLLKYNENGTITDAVDCALDPLSETKCTLKSFTVEKGIYQTSNFRVQPTESIVRFPNITNLCPFGEVFNATRFASVYAWNRKRISNCVADYSVLYNSASFSTFKCYGVSPTKLNDLCFTNVYADSFVIRGDEVRQIAPGQTGKIADYNYKLPDDFTGCVIAWNSNNLDSKVGGNYNYLYRLFRKSNLKPFERDISTEIYQAGSTPCNGVEGFNCYFPLQSYGFQPTNGVGYQPYRVVVLSFELLHAPATVCGPKKSTNLVKNKCVNFNFNGLTGTGVLTESNKKFLPFQQFGRDIADTTDAVRDPQTLEILDITPCSFGGVSVITPGTNTSNQVAVLYQDVNCTEVPVAIHADQLTPTWRVYSTGSNVFQTRAGCLIGAEHVNNSYECDIPIGAGICASYQTQTNSPVASQSIIAYTMSLGAENSVAYSNNSIAIPTNFTISVTTEILPVSMTKTSVDCTMYICGDSTECSNLLLQYGSFCTQLNRALTGIAVEQDKNTQEVFAQVKQIYKTPPIKDFGGFNFSQILPDPSKPSKRSFIEDLLFNKVTLADAGFIKQYGDCLGDIAARDLICAQKFNGLTVLPPLLTDEMIAQYTSALLAGTITSGWTFGAGAALQIPFAMQMAYRFNGIGVTQNVLYENQKLIANQFNSAIGKIQDSLSSTASALGKLQDVVNQNAQALNTLVKQLSSNFGAISSVLNDILSRLDKWEAEVQIDRLITGRLQSLQTYVTQQLIRAAEIRASANLAATKMSECVLGQSKRVDFCGKGYHLMSFPQSAPHGVVFLHVTYVPAQEKNFTTAPAICHDGKAHFPREGVFVSNGTHWFVTQRNFYEPQIITTDNTFVSGNCDVVIGIVNNTVYDPLQPELDSFKEELDKYFKNHTSPDVDLGDISGINASVVNIQKEIDRLNEVAKNLNESLIDLQELGKYEQ

SEQ ID NO: 8 - protein, 1188 aa, synthetic construct
VNLTTRTQLPPAYTNSFTRGVYYPDKVFRSSVLHSTQDLFLPFFSNVTWFHAIHVSGTNGTKRFDNPVLPFNDGVYFASTEKSNIIRGWIFGTTLDSKTQSLLIVNNATNVVIKVCEFQFCNDPFLGVYYHKNNKSWMESEFRVYSSANNCTFEYVSQPFLMDLEGKQGNFKNLREFVFKNIDGYFKIYSKHTPINLVRDLPQGFSALEPLVDLPIGINITRFQTLLALHRSYLTPGDSSSGWTAGAAAYYVGYLQPRTFLLKYNENGTITDAVDCALDPLSETKCTLKSFTVEKGIYQTSNFRVQPTESIVRFPNITNLCPFGEVFNATRFASVYAWNRKRISNCVADYSVLYNSASFSTFKCYGVSPTKLNDLCFTNVYADSFVIRGDEVRQIAPGQTGKIADYNYKLPIDFTGCVIAWNSNNLDSKVGGNYNYLYRLFRKSNLKPFERDISTEIYQAGSTPCNGVEGFNCYFPLQSYGFQPTNGVGYQPYRVVVLSFELLHAPATVCGPKKSTNLVKNKCVNFNFNGLTGTGVLTESNKKFLPFQQFGRDIADTTDAVRDPQTLEILDITPCSFGGVSVITPGTNTSNQVAVLYQDVNCTEVPVAIHADQLTPTWRVYSTGSNVFQTRAGCLIGAEHVNNSYECDIPIGAGICASYQTQTNSPVASQSIIAYTMSLGAENSVAYSNNSIAIPTNFTISVTTEILPVSMTKTSVDCTMYICGDSTECSNLLLQYGSFCTQLNRALTGIAVEQDKNTQEVFAQVKQIYKTPPIKDFGGFNFSQILPDPSKPSKRSFIEDLLFNKVTLADAGFIKQYGDCLGDIAARDLICAQKFNGLTVLPPLLTDEMIAQYTSALLAGTITSGWTFGAGAALQIPFAMQMAYRFNGIGVTQNVLYENQKLIANQFNSAIGKIQDSLSSTASALGKLQDVVNQNAQALNTLVKQLSSNFGAISSVLNDILSRLDKVEAEVQIDRLITGRLQSLQTYVTQQLIRAAEIRASANLAATKMSECVLGQSKRVDFCGKGYHLMSFPQSAPHGVVFLHVTYVPAQEKNFTTAPAICHDGKAHFPREGVFVSNGTHWFVTQRNFYEPQIITTDNTFVSGNCDVVIGIVNNTVYDPLQPELDSFKEELDKYFKNHTSPDVDLGDISGINASVVNIQKEIDRLNEVAKNLNESLIDLQELGKYEQ

SEQ ID NO: 9 - protein, 1188 aa, synthetic construct
VNLTTRTQLPPAYTNSFTRGVYYPDKVFRSSVLHSTQDLFLPFFSNVTWFHAIHVSGTNGTKRFDNPVLPFNDGVYFASTEKSNIIRGWIFGTTLDSKTQSLLIVNNATNVVIKVCEFQFCNDPFLGVYYHKNNKSWMESEFRVYSSANNCTFEYVSQPFLMDLEGKQGNFKNLREFVFKNIDGYFKIYSKHTPINLVRDLPQGFSALEPLVDLPIGINITRFQTLLALHRSYLTPGDSSSGWTAGAAAYYVGYLQPRTFLLKYNENGTITDAVDCALDPLSETKCTLKSFTVEKGIYQTSNFRVQPTESIVRFPNITNLCPFGEVFNATRFASVYAWNRKRISNCVADYSVLYNSASFSTFKCYGVSPTKLNDLCFTNVYADSFVIRGDEVRQIAPGQTGKIARYNYKLPDDFTGCVIAWNSNNLDSKVGGNYNYLYRLFRKSNLKPFERDISTEIYQAGSTPCNGVEGFNCYFPLQSYGFQPTNGVGYQPYRVVVLSFELLHAPATVCGPKKSTNLVKNKCVNFNFNGLTGTGVLTESNKKFLPFQQFGRDIADTTDAVRDPQTLEILDITPCSFGGVSVITPGTNTSNQVAVLYQDVNCTEVPVAIHADQLTPTWRVYSTGSNVFQTRAGCLIGAEHVNNSYECDIPIGAGICASYQTQTNSPVASQSIIAYTMSLGAENSVAYSNNSIAIPTNFTISVTTEILPVSMTKTSVDCTMYICGDSTECSNLLLQYGSFCTQLNRALTGIAVEQDKNTQEVFAQVKQIYKTPPIKDFGGFNFSQILPDPSKPSKRSFIEDLLFNKVTLADAGFIKQYGDCLGDIAARDLICAQKFNGLTVLPPLLTDEMIAQYTSALLAGTITSGWTFGAGAALQIPFAMQMAYRFNGIGVTQNVLYENQKLIANQFNSAIGKIQDSLSSTASALGKLQDVVNQNAQALNTLVKQLSSNFGAISSVLNDILSRLDKVEAEVQIDRLITGRLQSLQTYVTQQLIRAAEIRASANLAATKMSECVLGQSKRVDFCGKGYHLMSFPQSAPHGVVFLHVTYVPAQEKNFTTAPAICHDGKAHFPREGVFVSNGTHWFVTQRNFYEPQIITTDNTFVSGNCDVVIGIVNNTVYDPLQPELDSFKEELDKYFKNHTSPDVDLGDISGINASVVNIQKEIDRLNEVAKNLNESLIDLQELGKYEQ

SEQ ID NO: 10 - protein, 1188 aa, synthetic construct
VNLTTRTQLPPAYTNSFTRGVYYPDKVFRSSVLHSTQDLFLPFFSNVTWFHAIHVSGTNGTKRFDNPVLPFNDGVYFASTEKSNIIRGWIFGTTLDSKTQSLLIVNNATNVVIKVCEFQFCNDPFLGVYYHKNNKSWMESEFRVYSSANNCTFEYVSQPFLMDLEGKQGNFKNLREFVFKNIDGYFKIYSKHTPINLVRDLPQGFSALEPLVDLPIGINITRFQTLLALHRSYLTPGDSSSGWTAGAAAYYVGYLQPRTFLLKYNENGTITDAVDCALDPLSETKCTLKSFTVEKGIYQTSNFRVQPTESIVRFPNITNLCPFGEVFNATRFASVYAWNRKRISNCVADYSVLYNSWSFSTFKCYGVSPTKLNDLCFTNVYADSFVIRGDEVRQIAPGQTGKIADYNYKLPDDFTGCVIAWNSNNLDSKVGGNYNYLYRLFRKSNLKPFERDISTEIYQAGSTPCNGVEGFNCYFPLQSYGFQPTNGVGYQPYRVVVLSFELLHAPATVCGPKKSTNLVKNKCVNFNFNGLTGTGVLTESNKKFLPFQQFGRDIADTTDAVRDPQTLEILDITPCSFGGVSVITPGTNTSNQVAVLYQDVNCTEVPVAIHADQLTPTWRVYSTGSNVFQTRAGCLIGAEHVNNSYECDIPIGAGICASYQTQTNSPVASQSIIAYTMSLGAENSVAYSNNSIAIPTNFTISVTTEILPVSMTKTSVDCTMYICGDSTECSNLLLQYGSFCTQLNRALTGIAVEQDKNTQEVFAQVKQIYKTPPIKDFGGFNFSQILPDPSKPSKRSFIEDLLFNKVTLADAGFIKQYGDCLGDIAARDLICAQKFNGLTVLPPLLTDEMIAQYTSALLAGTITSGWTFGAGAALQIPFAMQMAYRFNGIGVTQNVLYENQKLIANQFNSAIGKIQDSLSSTASALGKLQDVVNQNAQALNTLVKQLSSNFGAISSVLNDILSRLDKVEAEVQIDRLITGRLQSLQTYVTQQLIRAAEIRASANLAATKMSECVLGQSKRVDFCGKGYHLMSFPQSAPHGVVFLHVTYVPAQEKNFTTAPAICHDGKAHFPREGVFVSNGTHWFVTQRNFYEPQIITTDNTFVSGNCDVVIGIVNNTVYDPLQPELDSFKEELDKYFKNHTSPDVDLGDISGINASVVNIQKEIDRLNEVAKNLNESLIDLQELGKYEQ

SEQ ID NO: 11 - protein, 1188 aa, synthetic construct
VNLTTRTQLPPAYTNSFTRGVYYPDKVFRSSVLHSTQDLFLPFFSNVTWFHAIHVSGTNGTKRFDNPVLPFNDGVYFASTEKSNIIRGWIFGTTLDSKTQSLLIVNNATNVVIKVCEFQFCNDPFLGVYYHKNNKSWMESEFRVYSSANNCTFEYVSQPFLMDLEGKQGNFKNLREFVFKNIDGYFKIYSKHTPINLVRDLPQGFSALEPLVDLPIGINITRFQTLLALHRSYLTPGDSSSGWTAGAAAYYVGYLQPRTFLLKYNENGTITDAVDCALDPLSETKCTLKSFTVEKGIYQTSNFRVQPTESIVRFPNITNLCPFGEVFNATRFASVYAWNRKRISNCVADYSVLYNSASFSTFKCYGVSPTKLNDLCFTNVYADSFVIRGDEVRQIAPGQTGKIAYYNYKLPDDFTGCVIAWNSNNLDSKVGGNYNYLYRLFRKSNLKPFERDISTEIYQAGSTPCNGVEGFNCYFPLQSYGFQPTNGVGYQPYRVVVLSFELLHAPATVCGPKKSTNLVKNKCVNFNFNGLTGTGVLTESNKKFLPFQQFGRDIADTTDAVRDPQTLEILDITPCSFGGVSVITPGTNTSNQVAVLYQDVNCTEVPVAIHADQLTPTWRVYSTGSNVFQTRAGCLIGAEHVNNSYECDIPIGAGICASYQTQTNSPVASQSIIAYTMSLGAENSVAYSNNSIAIPTNFTISVTTEILPVSMTKTSVDCTMYICGDSTECSNLLLQYGSFCTQLNRALTGIAVEQDKNTQEVFAQVKQIYKTPPIKDFGGFNFSQILPDPSKPSKRSFIEDLLFNKVTLADAGFIKQYGDCLGDIAARDLICAQKFNGLTVLPPLLTDEMIAQYTSALLAGTITSGWTFGAGAALQIPFAMQMAYRFNGIGVTQNVLYENQKLIANQFNSAIGKIQDSLSSTASALGKLQDVVNQNAQALNTLVKQLSSNFGAISSVLNDILSRLDKVEAEVQIDRLITGRLQSLQTYVTQQLIRAAEIRASANLAATKMSECVLGQSKRVDFCGKGYHLMSFPQSAPHGVVFLHVTYVPAQEKNFTTAPAICHDGKAHFPREGVFVSNGTHWFVTQRNFYEPQIITTDNTFVSGNCDVVIGIVNNTVYDPLQPELDSFKEELDKYFKNHTSPDVDLGDISGINASVVNIQKEIDRLNEVAKNLNESLIDLQELGKYEQ

SEQ ID NO: 12 - protein, 1188 aa, synthetic construct
VNLTTRTQLPPAYTNSFTRGVYYPDKVFRSSVLHSTQDLFLPFFSNVTWFHAIHVSGTNGTKRFDNPVLPFNDGVYFASTEKSNIIRGWIFGTTLDSKTQSLLIVNNATNVVIKVCEFQFCNDPFLGVYYHKNNKSWMESEFRVYSSANNCTFEYVSQPFLMDLEGKQGNFKNLREFVFKNIDGYFKIYSKHTPINLVRDLPQGFSALEPLVDLPIGINITRFQTLLALHRSYLTPGDSSSGWTAGAAAYYVGYLQPRTFLLKYNENGTITDAVDCALDPLSETKCTLKSFTVEKGIYQTSNFRVQPTESIVRFPNITNLCPFGEVFNATRFASVYAWNRKRISNCVADYSVLYNSWSFSTFKCYGVSPTKLNDLCFTNVYADSFVIRGDEVRQIAPGQTGKIARYNYKLPDDFTGCVIAWNSNNLDSKVGGNYNYLYRLFRKSNLKPFERDISTEIYQAGSTPCNGVEGFNCYFPLQSYGFQPTNGVGYQPYRVVVLSFELLHAPATVCGPKKSTNLVKNKCVNFNFNGLTGTGVLTESNKKFLPFQQFGRDIADTTDAVRDPQTLEILDITPCSFGGVSVITPGTNTSNQVAVLYQDVNCTEVPVAIHADQLTPTWRVYSTGSNVFQTRAGCLIGAEHVNNSYECDIPIGAGICASYQTQTNSPVASQSIIAYTMSLGAENSVAYSNNSIAIPTNFTISVTTEILPVSMTKTSVDCTMYICGDSTECSNLLLQYGSFCTQLNRALTGIAVEQDKNTQEVFAQVKQIYKTPPIKDFGGFNFSQILPDPSKPSKRSFIEDLLFNKVTLADAGFIKQYGDCLGDIAARDLICAQKFNGLTVLPPLLTDEMIAQYTSALLAGTITSGWTFGAGAALQIPFAMQMAYRFNGIGVTQNVLYENQKLIANQFNSAIGKIQDSLSSTASALGKLQDVVNQNAQALNTLVKQLSSNFGAISSVLNDILSRLDKVEAEVQIDRLITGRLQSLQTYVTQQLIRAAEIRASANLAATKMSECVLGQSKRVDFCGKGYHLMSFPQSAPHGVVFLHVTYVPAQEKNFTTAPAICHDGKAHFPREGVFVSNGTHWFVTQRNFYEPQIITTDNTFVSGNCDVVIGIVNNTVYDPLQPELDSFKEELDKYFKNHTSPDVDLGDISGINASVVNIQKEIDRLNEVAKNLNESLIDLQELGKYEQ

SEQ ID NO: 13 - protein, 1188 aa, synthetic construct
VNLTTRTQLPPAYTNSFTRGVYYPDKVFRSSVLHSTQDLFLPFFSNVTWFHAIHVSGTNGTKRFDNPVLPFNDGVYFASTEKSNIIRGWIFGTTLDSKTQSLLIVNNATNVVIKVCEFQFCNDPFLGVYYHKNNKSWMESEFRVYSSANNCTFEYVSQPFLMDLEGKQGNFKNLREFVFKNIDGYFKIYSKHTPINLVRDLPQGFSALEPLVDLPIGINITRFQTLLALHRSYLTPGDSSSGWTAGAAAYYVGYLQPRTFLLKYNENGTITDAVDCALDPLSETKCTLKSFTVEKGIYQTSNFRVQPTESIVRFPNITNLCPFGEVFNATRFASVYAWNRKRISNCVADYSVLYNSASFSTFKCYGVSPTKLNDLCFTNVYADSFVIRGDEVRQIAPGQTGKIADYNYKLPDDFTGCVIAWNSNNLDSKVGGNYNYLYRLFRKSNLKPFERDISTEIYQAGSTPCNGVEGFNCYFPLQSYGFQPTNGVGYQPYRVVVLSFELLHAPATVCGPKKSTNLVKNKCVNFNFNGLTGTGVLTESNKKFLPFQQFGRDIADTTDAVRDPQTLEILDITPCSFGGVSVITPGTNTSNQVAVLYQDVNCTEVPVAIHADQLTPTWRVYSTGSNVFQTRAGCLIGAEHVNNSYECDIPIGAGICASYQTQTNSPVASQSIIAYTMSLGAENSVQYSNNSIAIPTNFTISVTTEILPVSMTKTSVDCTMYICGDSTECSNLLLQYGEFCTQLNRALTGIAVEQDKNTQEVFAQVKQIYKTPPIKDFGGFNFSQILPDPSKPSKRSFIEDLLFNKVTLADAGFIKQYGDCLGDIAARDKICAQKFNGLTVLPPLLTDEMIAQYTSALLAGTITSGWTFGAGAALQIPFAMQMAYRFNGIGVTQNVLYENQKLIANQFNSAIGKIQDSLSSTASALGKLQDVVNQNAQALNTLEKQLSSNFGAISSVLNDILSRLDPPEAEVQIDRLITGRLQSLQTYVTQQLIRAAEIRASANLAATKMRECVLGQSKRVDFCGKGYHLMSFPQSAPHGVVFLHVTYVPAQEKNFTTAPAICHDGKAHFPREGVFVSNGTHWFVTQRNFYEPRIITTDNTFVSGNCDVVIGIVNNTVYDPLQPELDSFKEELDKYFKNHTSPDVDLGDISGINASVVNIQKEIDRLNEVAKNLNESLIDLQELGKYEQ

SEQ ID NO: 14 - protein, 1188 aa, synthetic construct; identical to SEQ ID NO: 13

SEQ ID NO: 15 - protein, 1188 aa, synthetic construct
VNLTTRTQLPPAYTNSFTRGVYYPDKVFRSSVLHSTQDLFLPFFSNVTWFHAIHVSGTNGTKRFDNPVLPFNDGVYFASTEKSNIIRGWIFGTTLDSKTQSLLIVNNATNVVIKVCEFQFCNDPFLGVYYHKNNKSWMESEFRVYSSANNCTFEYVSQPFLMDLEGKQGNFKNLREFVFKNIDGYFKIYSKHTPINLVRDLPQGFSALEPLVDLPIGINITRFQTLLALHRSYLTPGDSSSGWTAGAAAYYVGYLQPRTFLLKYNENGTITDAVDCALDPLSETKCTLKSFTVEKGIYQTSNFRVQPTESIVRFPNITNLCPFGEVFNATRFASVYAWNRKRISNCVADYSVLYNSASFSTFKCYGVSPTKLNDLCFTNVYADSFVIRGDEVRQIAPGQTGKIADYNYKLPDDFTGCVIAWNSNNLDSKVGGNYNYLYRLFRKSNLKPFERDISTEIYQAGSTPCNGVEGFNCYFPLQSYGFQPTNGVGYQPYRVVVLSFELLHAPATVCGPKKSTNLVKNKCVNFNFNGLTGTGVLTESNKKFLPFQQFGRDIADTTDAVRDPQTLEILDITPCSFGGVSVITPGTNTSNQVAVLYQDVNCTEVPVAIHADQLTPTWRVYSTGSNVFQTRAGCLIGAEHVNNSYECDIPIGAGICASYQTQTNSPVASQSIIAYTMSLGAENSVAYSNNSIAIPTNFTISVTTEILPVSMTKTSVDCTMYICGDSTECSNLLLKYGSFCTQLNRALTGIAVEQDKNTQEVFAQVKQIYKTPPIKDFGGFNFSQILPDPSKPSKRSFIEDLLFNKVTLADAGFIKQYGDCLGDIAARDKICAQKFNGLTVLPPLLTDEMIAQYTSALLAGTITSGWTFGAGNALQIPFAMQMAYRFNGIGVTQNVLYENQKLIANQFNSAIGKIQDSLSSTASALGRLQDVVNQNAQALNTLVKQLSSNFGAISSVLNDILSRLDPPEAEVQIDRLITGRLQSLQTYVTQQLIRAAEIRASANLAATKMSECVLGQSKRVDFCGRGYHLMSFPQSAPHGVVFLHVTYVPAQEKNFTTAPAICHDGKAHFPREGVFVSNGTHWFVTQRNFYEPQIITTDNTFVSGNCDVVIGIVNNTVYDPLQPELDSFKEELDKYFKNHTSPDVDLGDISGINASVVNIQKEIDRLNEVAKNLNESLIDLQELGKYEQ

SEQ ID NO: 16 - protein, 1188 aa, synthetic construct
VNLTTRTQLPPAYTNSFTRGVYYPDKVFRSSVLHSTQDLFLPFFSNVTWFHAIHVSGTNGTKRFDNPVLPFNDGVYFASTEKSNIIRGWIFGTTLDSKTQSLLIVNNATNVVIKVCEFQFCNDPFLGVYYHKNNKSWMESEFRVYSSANNCTFEYVSQPFLMDLEGKQGNFKNLREFVFKNIDGYFKIYSKHTPINLVRDLPQGFSALEPLVDLPIGINITRFQTLLALHRSYLTPGDSSSGWTAGAAAYYVGYLQPRTFLLKYNENGTITDAVDCALDPLSETKCTLKSFTVEKGIYQTSNFRVQPTESIVRFPNITNLCPFGEVFNATRFASVYAWNRKRISNCVADYSVLYNSASFSTFKCYGVSPTKLNDLCFTNVYADSFVIRGDEVRQIAPGQTGKIADYNYKLPDDFTGCVIAWNSNNLDSKVGGNYNYLYRLFRKSNLKPFERDISTEIYQAGSTPCNGVEGFNCYFPLQSYGFQPTNGVGYQPYRVVVLSFELLHAPATVCGPKKSTNLVKNKCVNFNFNGLTGTGVLTESNKKFLPFQQFGRDIADTTDAVRDPQTLEILDITPCSFGGVSVITPGTNTSNQVAVLYQDVNCTEVPVAIHADQLTPTWRVYSTGSNVFQTRAGCLIGAEHVNNSYECDIPIGAGICASYQTQTNSPVASQSIIAYTMSLGAENSVAYSNNSIAIPTNFTISVTTEILPVSMTKTSVDCTMYICGDSTECSNLLLQYGEFCTQLNRALTGIAVEQDKNTQEVFAQVKQIYKTPPIKDFGGFNFSQILPDPSKPSKRSFIEDLLFNKVTLADAGFIKQYGDCLGDIAARDKICAQKFNGLTVLPPLLTDEMIAQYTSALLAGTITSGWTFGAGAALQIPFAMQMAYRFNGIGVTQNVLYENQKLIANQFNSAIGKIQDSLSSTASALGKLQDVVNQNAQALNTLEKQLSSNFGAISSVLNDILSRLDPPEAEVQIDRLITGRLQSLQTYVTQQLIRAAEIRASANLAATKMSECVLGQSKRVDFCGKGYHLMSFPQSAPHGVVFLHVTYVPAQEKNFTTAPAICHDGKAHFPREGVFVSNGTHWFVTQRNFYEPQIITTDNTFVSGNCDVVIGIVNNTVYDPLQPELDSFKEELDKYFKNHTSPDVDLGDISGINASVVNIQKEIDRLNEVAKNLNESLIDLQELGKYEQ

SEQ ID NO: 17 - protein, 1188 aa, synthetic construct
VNLTTRTQLPPAYTNSFTRGVYYPDKVFRSSVLHSTQDLFLPFFSNVTWFHAIHVSGTNGTKRFDNPVLPFNDGVYFASTEKSNIIRGWIFGTTLDSKTQSLLIVNNATNVVIKVCEFQFCNDPFLGVYYHKNNKSWMESEFRVYSSANNCTFEYVSQPFLMDLEGKQGNFKNLREFVFKNIDGYFKIYSKHTPINLVRDLPQGFSALEPLVDLPIGINITRFQTLLALHRSYLTPGDSSSGWTAGAAAYYVGYLQPRTFLLKYNENGTITDAVDCALDPLSETKCTLKSFTVEKGIYQTSNFRVQPTESIVRFPNITNLCPFGEVFNATRFASVYAWNRKRISNCVADYSVLYNSASFSTFKCYGVSPTKLNDLCFTNVYADSFVIRGDEVRQIAPGQTGKIADYNYKLPDDFTGCVIAWNSNNLDSKVGGNYNYLYRLFRKSNLKPFERDISTEIYQAGSTPCNGVEGFNCYFPLQSYGFQPTNGVGYQPYRVVVLSFELLHAPATVCGPKKSTNLVKNKCVNFNFNGLTGTGVLTESNKKFLPFQQFGRDIADTTDAVRDPQTLEILDITPCSFGGVSVITPGTNTSNQVAVLYQDVNCTEVPVAIHADQLTPTWRVYSTGSNVFQTRAGCLIGAEHVNNSYECDIPIGAGICASYQTQTNSPVASQSIIAYTMSLGAENSVAYSNNSIAIPTNFTISVTTEILPVSMTKTSVDCTMYICGDSTECSNLLLKYGSFCTQLNRALTGIAVEQDKNTQEVFAQVKQIYKTPPIKDFGGFNFSQILPDPSKPSKRSFIEDLLFNKVTLADAGFIKQYGDCLGDIAARDLIQAQKFNGLTVLPPLLTDEMIAQYTSALLAGTITSGWTFGAGAALQIPFAMQMAYRFNGIGVTQNVLYENQKLIANQFNSAIGKIQDSLSSTASALGKLQDVVNQNAQALNELVKQLSSNFGAISSVLNDILSRLDPPEAEVQIDRLITGRLQSLQTYVTQQLIRAAEIRASANLAATKMSECVLGQSKRVDFCGKGYHLMSFPQSAPHGVVFLHVTYVPAQEKNFTTAPAICHDGKAHFPREGVFVSNGTHWFVTQRNFYEPQIITTDNTFVSGNCDVVIGIVNNTVYDPLQPELDSFKEELDKYFKNHTSPDVDLGDISGINASVVNIQKEIDRLNEVAKNLNESLIDLQELGKYEQ

SEQ ID NO: 18 - protein, 1188 aa, synthetic construct
VNLTTRTQLPPAYTNSFTRGVYYPDKVFRSSVLHSTQDLFLPFFSNVTWFHAIHVSGTNGTKRFDNPVLPFNDGVYFASTEKSNIIRGWIFGTTLDSKTQSLLIVNNATNVVIKVCEFQFCNDPFLGVYYHKNNKSWMESEFRVYSSANNCTFEYVSQPFLMDLEGKQGNFKNLREFVFKNIDGYFKIYSKHTPINLVRDLPQGFSALEPLVDLPIGINITRFQTLLALHRSYLTPGDSSSGWTAGAAAYYVGYLQPRTFLLKYNENGTITDAVDCALDPLSETKCTLKSFTVEKGIYQTSNFRVQPTESIVRFPNITNLCPFGEVFNATRFASVYAWNRKRISNCVADYSVLYNSASFSTFKCYGVSPTKLNDLCFTNVYADSFVIRGDEVRQIAPGQTGKIADYNYKLPDDFTGCVIAWNSNNLDSKVGGNYNYLYRLFRKSNLKPFERDISTEIYQAGSTPCNGVEGFNCYFPLQSYGFQPTNGVGYQPYRVVVLSFELLHAPATVCGPKKSTNLVKNKCVNFNFNGLTGTGVLTESNKKFLPFQQFGRDIADTTDAVRDPQTLEILDITPCSFGGVSVITPGTNTSNQVAVLYQDVNCTEVPVAIHADQLTPTWRVYSTGSNVFQTRAGCLIGAEHVNNSYECDIPIGAGICASYQTQTNSPVASQSIIAYTMSLGAENSVQYSNNSIAIPTNFTISVTTEILPVSMTKTSVDCTMYICGDSTECSNLLLQYGSFCTQLNRALTGIAVEQDKNTQEVFAQVKQIYKTPPIKDFGGFNFSQILPDPSKPSKRSFIEDLLFNKVTLADAGFIKQYGDCLGDIAARDLICAQKFNGLTVLPPLLTDEMIAQYTSALLAGTITSGWTFGAGAALQIPFAMQMAYRFNGIGVTQNVLYENQKLIANQFNSAIGKIQDSLSSTASALGKLQDVVNQNAQALNTLVKQLSSNFGAISSVLNDILSRLDPPEAEVQIDRLITGRLQSLQTYVTQQLIRAAEIRASANLAATKMRECVLGQSKRVDFCGKGYHLMSFPQSAPHGVVFLHVTYVPAQEKNFTTAPAICHDGKAHFPREGVFVSNGTHWFVTQRNFYEPRIITTDNTFVSGNCDVVIGIVNNTVYDPLQPELDSFKEELDKYFKNHTSPDVDLGDISGINASVVNIQKEIDRLNEVAKNLNESLIDLQELGKYEQ

SEQ ID NO: 19 - protein, 1188 aa, synthetic construct
VNLTTRTQLPPAYTNSFTRGVYYPDKVFRSSVLHSTQDLFLPFFSNVTWFHAIHVSGTNGTKRFDNPVLPFNDGVYFASTEKSNIIRGWIFGTTLDSKTQSLLIVNNATNVVIKVCEFQFCNDPFLGVYYHKNNKSWMESEFRVYSSANNCTFEYVSQPFLMDLEGKQGNFKNLREFVFKNIDGYFKIYSKHTPINLVRDLPQGFSALEPLVDLPIGINITRFQTLLALHRSYLTPGDSSSGWTAGAAAYYVGYLQPRTFLLKYNENGTITDAVDCALDPLSETKCTLKSFTVEKGIYQTSNFRVQPTESIVRFPNITNLCPFGEVFNATRFASVYAWNRKRISNCVADYSVLYNSASFSTFKCYGVSPTKLNDLCFTNVYADSFVIRGDEVRQIAPGQTGKIADYNYKLPDDFTGCVIAWNSNNLDSKVGGNYNYLYRLFRKSNLKPFERDISTEIYQAGSTPCNGVEGFNCYFPLQSYGFQPTNGVGYQPYRVVVLSFELLHAPATVCGPKKSTNLVKNKCVNFNFNGLTGTGVLTESNKKFLPFQQFGRDIADTTDAVRDPQTLEILDITPCSFGGVSVITPGTNTSNQVAVLYQDVNCTEVPVAIHADQLTPTWRVYSTGSNVFQTRAGCLIGAEHVNNSYECDIPIGAGICASYQTQTNSPVASQSIIAYTMSLGAENSVAYSNNSIAIPTNFTISVTTEILPVSMTKTSVDCTMYICGDSTECSNLLLQYGEFCTQLNRALTGIAVEQDKNTQEVFAQVKQIYKTPPIKDFGGFNFSQILPDPSKPSKRSFIEDLLFNKVTLADAGFIKQYGDCLGDIAARDLICAQKFNGLTVLPPLLTDEMIAQYTSALLAGTITSGWTFGAGAALQIPFAMQMAYRFNGIGVRQNVLYENQKLIANQFNSAIGKIQDSLSSTASALGRLQDVVNQNAQALNTLVKQLSSNFGAISSVLNDILSRLDPPEAEVQIDRLITGRLQSLQTYVTQQLIRAAEIRASANLAATKMSECVLGQSKRVDFCGKGYHLMSFPQSAPHGVVFLHVTYVPAQEKNFTTAPAICHDGKAHFPREGVFVSNGTHWFVTQRNFYEPQIITTDNTFVSGNCDVVIGIVNNTVYDPLQPELDSFKEELDKYFKNHTSPDVDLGDISGINASVVNIQKEIDRLNEVAKNLNESLIDLQELGKYEQ

SEQ ID NO: 20 - protein, 1188 aa, synthetic construct
VNLTTRTQLPPAYTNSFTRGVYYPDKVFRSSVLHSTQDLFLPFFSNVTWFHAIHVSGTNGTKRFDNPVLPFNDGVYFASTEKSNIIRGWIFGTTLDSKTQSLLIVNNATNVVIKVCEFQFCNDPFLGVYYHKNNKSWMESEFRVYSSANNCTFEYVSQPFLMDLEGKQGNFKNLREFVFKNIDGYFKIYSKHTPINLVRDLPQGFSALEPLVDLPIGINITRFQTLLALHRSYLTPGDSSSGWTAGAAAYYVGYLQPRTFLLKYNENGTITDAVDCALDPLSETKCTLKSFTVEKGIYQTSNFRVQPTESIVRFPNITNLCPFGEVFNATRFASVYAWNRKRISNCVADYSVLYNSASFSTFKCYGVSPTKLNDLCFTNVYADSFVIRGDEVRQIAPGQTGKIADYNYKLPDDFTGCVIAWNSNNLDSKVGGNYNYLYRLFRKSNLKPFERDISTEIYQAGSTPCNGVEGFNCYFPLQSYGFQPTNGVGYQPYRVVVLSFELLHAPATVCGPKKSTNLVKNKCVNFNFNGLTGTGVLTESNKKFLPFQQFGRDIADTTDAVRDPQTLEILDITPCSFGGVSVITPGTNTSNQVAVLYQDVNCTEVPVAIHADQLTPTWRVYSTGSNVFQTRAGCLIGAEHVNNSYECDIPIGAGICASYQTQTNSPVASQSIIAYTMSLGAENSVAYSNNSIAIPTNFTISVTTEILPVSMTKTSVDCTMYICGDSTECSNLLLQYGSFCTQLNRALTGIAVEQDKNTQEVFAQVKQIYKTPPIKDFGGFNFSQILPDPSKPSKRSFIEDLLFNKVTLADAGFIKQYGDCLGDIAARDKICAQKFNGLTVLPPLLTDEMIAQYTSALLAGTITSGWTFGAGAALQIPFAMQMAYRFNGIGVTQNVLYENQKLIANQFNSAIGKIQDSLSSTASALGKLQDVVNQNAQALNTLVKQLSSNFGAISSVLNDILSRLDPPEAEVQIDRLITGRLQSLQTYVTQQLIRAAEIRASANLAATKMSECVLGQSKRVDFCGKGYHLMSFPQSAPHGVVFLHVTYVPAQEKNFTTAPAICHDGKAHFPREGVFVSNGTHWFVTQRNFYEPQIITTDNTFVSGNCDVVIGIVNNTVYDPLQPELDSFKEELDKYFKNHTSPDVDLGDISGINASVVNIQKEIDRLNEVAKNLNESLIDLQELGKYEQ

SEQ ID NO: 21 - protein, 1188 aa, synthetic construct
VNLTTRTQLPPAYTNSFTRGVYYPDKVFRSSVLHSTQDLFLPFFSNVTWFHAIHVSGTNGTKRFDNPVLPFNDGVYFASTEKSNIIRGWIFGTTLDSKTQSLLIVNNATNVVIKVCEFQFCNDPFLGVYYHKNNKSWMESEFRVYSSANNCTFEYVSQPFLMDLEGKQGNFKNLREFVFKNIDGYFKIYSKHTPINLVRDLPQGFSALEPLVDLPIGINITRFQTLLALHRSYLTPGDSSSGWTAGAAAYYVGYLQPRTFLLKYNENGTITDAVDCALDPLSETKCTLKSFTVEKGIYQTSNFRVQPTESIVRFPNITNLCPFGEVFNATRFASVYAWNRKRISNCVADYSVLYNSASFSTFKCYGVSPTKLNDLCFTNVYADSFVIRGDEVRQIAPGQTGKIADYNYKLPDDFTGCVIAWNSNNLDSKVGGNYNYLYRLFRKSNLKPFERDISTEIYQAGSTPCNGVEGFNCYFPLQSYGFQPTNGVGYQPYRVVVLSFELLHAPATVCGPKKSTNLVKNKCVNFNFNGLTGTGVLTESNKKFLPFQQFGRDIADTTDAVRDPQTLEILDITPCSFGGVSVITPGTNTSNQVAVLYQDVNCTEVPVAIHADQLTPTWRVYSTGSNVFQTRAGCLIGAEHVNNSYECDIPIGAGICASYQTQTNSPVASQSIIAYTMSLGAENSVAYSNNSIAIPTNFTISVTTEILPVSMTKTSVDCTMYICGDSTECSNLLLQYGSFCTQLNRALTGIAVEQDKNTQEVFAQVKQIYKTPPIKDFGGFNFSQILPDPSKPSKRSFIEDLLFNKVTLADAGFIKQYGDCLGDIAARDLICAQKFNGLTVLPPLLTDEMIAQYTSALLAGTITSGWTFGAGAALQIPFAMQMAYRFNGIGVTQNVLYENQKLIANQFNSAIGKIQDSLSSTASALGKLQDVVNQNAQALNELVKQLSSNFGAISSVLNDILSRLDPPEAEVQIDRLITGRLQSLQTYVTQQLIRAAEIRASANLAATKMSECVLGQSKRVDFCGKGYHLMSFPQSAPHGVVFLHVTYVPAQEKNFTTAPAICHDGKAHFPREGVFVSNGTHWFVTQRNFYEPQIITTDNTFVSGNCDVVIGIVNNTVYDPLQPELDSFKEELDKYFKNHTSPDVDLGDISGINASVVNIQKEIDRLNEVAKNLNESLIDLQELGKYEQ

SEQ ID NO: 22 - protein, 27 aa, synthetic construct
GYIPEAPRDGQAYVRKDGEWVLLSTFL

SEQ ID NO: 23 - protein, 8 aa, synthetic construct
HHHHHHHH

SEQ ID NO: 24 - protein, 8 aa, synthetic construct
WSHPQFEK

SEQ ID NO: 25 - protein, 8 aa, synthetic construct
LEVLFQGP

SEQ ID NO: 26 - protein, 5 aa, synthetic construct
GSASS

SEQ ID NO: 27 - protein, 1278 aa, synthetic construct
VNLTTRTQLPPAYTNSFTRGVYYPDKVFRSSVLHSTQDLFLPFFSNVTWFHAIHVSGTNGTKRFDNPVLPFNDGVYFASTEKSNIIRGWIFGTTLDSKTQSLLIVNNATNVVIKVCEFQFCNDPFLGVYYHKNNKSWMESEFRVYSSANNCTFEYVSQPFLMDLEGKQGNFKNLREFVFKNIDGYFKIYSKHTPINLVRDLPQGFSALEPLVDLPIGINITRFQTLLALHRSYLTPGDSSSGWTAGAAAYYVGYLQPRTFLLKYNENGTITDAVDCALDPLSETKCTLKSFTVEKGIYQTSNFRVQPTESIVRFPNITNLCPFGEVFNATRFASVYAWNRKRISNCVADYSVLYNSASFSTFKCYGVSPTKLNDLCFTNVYADSFVIRGDEVRQIAPGQTGKIADYNYKLPDDFTGCVIAWNSNNLDSKVGGNYNYLYRLFRKSNLKPFERDISTEIYQAGSTPCNGVEGFNCYFPLQSYGFQPTNGVGYQPYRVVVLSFELLHAPATVCGPKKSTNLVKNKCVNFNFNGLTGTGVLTESNKKFLPFQQFGRDIADTTDAVRDPQTLEILDITPCSFGGVSVITPGTNTSNQVAVLYQDVNCTEVPVAIHADQLTPTWRVYSTGSNVFQTRAGCLIGAEHVNNSYECDIPIGAGICASYQTQTNSPGSASSVASQSIIAYTMSLGAENSVAYSNNSIAIPTNFTISVTTEILPVSMTKTSVDCTMYICGDSTECSNLLLQYGSFCTQLNRALTGIAVEQDKNTQEVFAQVKQIYKTPPIKDFGGFNFSQILPDPSKPSKRSFIEDLLFNKVTLADAGFIKQYGDCLGDIAARDLICAQKFNGLTVLPPLLTDEMIAQYTSALLAGTITSGWTFGAGAALQIPFAMQMAYRFNGIGVTQNVLYENQKLIANQFNSAIGKIQDSLSSTASALGKLQDVVNQNAQALNTLVKQLSSNFGAISSVLNDILSRLDKHEAEVQIDRLITGRLQSLQTYVTQQLIRAAEIRASANLAATKMSECVLGQSKRVDFCGKGYHLMSFPQSAPHGVVFLHVTYVPAQEKNFTTAPAICHDGKAHFPREGVFVSNGTHWFVTQRNFYEPQIITTDNTFVSGNCDVVIGIVNNTVYDPLQPELDSFKEELDKYFKNHTSPDVDLGDISGINASVVNIQKEIDRLNEVAKNLNESLIDLQELGKYEQGGGGTGGGYIPEAPRDGQAYVRKDGEWVLLSTFLGRSLEVLFQGPGHHHHHHHHSAWSHPQFEKGGGSGGGGSGGSAWSHPQFEK

SEQ ID NO: 28 - protein, 1278 aa, synthetic construct
VNLTTRTQLPPAYTNSFTRGVYYPDKVFRSSVLHSTQDLFLPFFSNVTWFHAIHVSGTNGTKRFDNPVLPFNDGVYFASTEKSNIIRGWIFGTTLDSKTQSLLIVNNATNVVIKVCEFQFCNDPFLGVYYHKNNKSWMESEFRVYSSANNCTFEYVSQPFLMDLEGKQGNFKNLREFVFKNIDGYFKIYSKHTPINLVRDLPQGFSALEPLVDLPIGINITRFQTLLALHRSYLTPGDSSSGWTAGAAAYYVGYLQPRTFLLKYNENGTITDAVDCALDPLSETKCTLKSFTVEKGIYQTSNFRVQPTESIVRFPNITNLCPFGEVFNATRFASVYAWNRKRISNCVADYSVLYNSASFSTFKCYGVSPTKLNDLCFTNVYADSFVIRGDEVRQIAPGQTGKIADYNYKLPDDFTGCVIAWNSNNLDSKVGGNYNYLYRLFRKSNLKPFERDISTEIYQAGSTPCNGVEGFNCYFPLQSYGFQPTNGVGYQPYRVVVLSFELLHAPATVCGPKKSTNLVKNKCVNFNFNGLTGTGVLTESNKKFLPFQQFGRDIADTTDAVRDPQTLEILDITPCSFGGVSVITPGTNTSNQVAVLYQDVNCTEVPVAIHADQLTPTWRVYSTGSNVFQTRAGCLIGAEHVNNSYECDIPIGAGICASYQTQTNSPGSASSVASQSIIAYTMSLGAENSVAYSNNSIAIPTNFTISVTTEILPVSMTKTSVDCTMYICGDSTECSNLLLQYGSFCTQLNRALTGIAVEQDKNTQEVFAQVKQIYKTPPIKDFGGFNFSQILPDPSKPSKRSFIEDLLFNKVTLADAGFIKQYGDCLGDIAARDLICAQKFNGLTVLPPLLTDEMIAQYTSALLAGTITSGWTFGAGAALQIPFAMQMAYRFNGIGVTQNVLYENQKLIANQFNSAIGKIQDSLSSTASALGKLQDVVNQNAQALNTLVKQLSSNFGAISSVLNDILSRLLKVEAEVQIDRLITGRLQSLQTYVTQQLIRAAEIRASANLAATKMSECVLGQSKRVDFCGKGYHLMSFPQSAPHGVVFLHVTYVPAQEKNFTTAPAICHDGKAHFPREGVFVSNGTHWFVTQRNFYEPQIITTDNTFVSGNCDVVIGIVNNTVYDPLQPELDSFKEELDKYFKNHTSPDVDLGDISGINASVVNIQKEIDRLNEVAKNLNESLIDLQELGKYEQGGGGTGGGYIPEAPRDGQAYVRKDGEWVLLSTFLGRSLEVLFQGPGHHHHHHHHSAWSHPQFEKGGGSGGGGSGGSAWSHPQFEK

SEQ ID NO: 29 - protein, 1278 aa, synthetic construct
VNLTTRTQLPPAYTNSFTRGVYYPDKVFRSSVLHSTQDLFLPFFSNVTWFHAIHVSGTNGTKRFDNPVLPFNDGVYFASTEKSNIIRGWIFGTTLDSKTQSLLIVNNATNVVIKVCEFQFCNDPFLGVYYHKNNKSWMESEFRVYSSANNCTFEYVSQPFLMDLEGKQGNFKNLREFVFKNIDGYFKIYSKHTPINLVRDLPQGFSALEPLVDLPIGINITRFQTLLALHRSYLTPGDSSSGWTAGAAAYYVGYLQPRTFLLKYNENGTITDAVDCALDPLSETKCTLKSFTVEKGIYQTSNFRVQPTESIVRFPNITNLCPFGEVFNATRFASVYAWNRKRISNCVADYSVLYNSASFSTFKCYGVSPTKLNDLCFTNVYADSFVIRGDEVRQIAPGQTGKIADYNYKLPDDFTGCVIAWNSNNLDSKVGGNYNYLYRLFRKSNLKPFERDISTEIYQAGSTPCNGVEGFNCYFPLQSYGFQPTNGVGYQPYRVVVLSFELLHAPATVCGPKKSTNLVKNKCVNFNFNGLTGTGVLTESNKKFLPFQQFGRDIADTTDAVRDPQTLEILDITPCSFGGVSVITPGTNTSNQVAVLYQDVNCTEVPVAIHADQLTPTWRVYSTGSNVFQTRAGCLIGAEHVNNSYECDIPIGAGICASYQTQTNSPGSASSVASQSIIAYTMSLGAENSVAYSNNSIAIPTNFTISVTTEILPVSMTKTSVDCTMYICGDSTECSNLLLQYGSFCTQLNRALTGIAVEQDKNTQEVFAQVKQIYKTPPIKDFGGFNFSQILPDPSKPSKRSFIEDLLFNKVTLADAGFIKQYGDCLGDIAARDLICAQKFNGLTVLPPLLTDEMIAQYTSALLAGTITSGWTFGAGAALQIPFAMQMAYRFNGIGVTQNVLYENQKLIANQFNSAIGKIQDSLSSTASALGKLQDVVNQNAQALNTLVKQLSSNFGAISSVLNDILFRLDKVEAEVQIDRLITGRLQSLQTYVTQQLIRAAEIRASANLAATKMSECVLGQSKRVDFCGKGYHLMSFPQSAPHGVVFLHVTYVPAQEKNFTTAPAICHDGKAHFPREGVFVSNGTHWFVTQRNFYEPQIITTDNTFVSGNCDVVIGIVNNTVYDPLQPELDSFKEELDKYFKNHTSPDVDLGDISGINASVVNIQKEIDRLNEVAKNLNESLIDLQELGKYEQGGGGTGGGYIPEAPRDGQAYVRKDGEWVLLSTFLGRSLEVLFQGPGHHHHHHHHSAWSHPQFEKGGGSGGGGSGGSAWSHPQFEK

SEQ ID NO: 30 - protein, 1278 aa, synthetic construct
VNLTTRTQLPPAYTNSFTRGVYYPDKVFRSSVLHSTQDLFLPFFSNVTWFHAIHVSGTNGTKRFDNPVLPFNDGVYFASTEKSNIIRGWIFGTTLDSKTQSLLIVNNATNVVIKVCEFQFCNDPFLGVYYHKNNKSWMESEFRVYSSANNCTFEYVSQPFLMDLEGKQGNFKNLREFVFKNIDGYFKIYSKHTPINLVRDLPQGFSALEPLVDLPIGINITRFQTLLALHRSYLTPGDSSSGWTAGAAAYYVGYLQPRTFLLKYNENGTITDAVDCALDPLSETKCTLKSFTVEKGIYQTSNFRVQPTESIVRFPNITNLCPFGEVFNATRFASVYAWNRKRISNCVADYSVLYNSASFSTFKCYGVSPTKLNDLCFTNVYADSFVIRGDEVRQIAPGQTGKIADYNYKLPDDFTGCVIAWNSNNLDSKVGGNYNYLYRLFRKSNLKPFERDISTEIYQAGSTPCNGVEGFNCYFPLQSYGFQPTNGVGYQPYRVVVLSFEYLHAPATVCGPKKSTNLVKNKCVNFNFNGLTGTGVLTESNKKFLPFQQFGRDIADTTDAVRDPQTLEILDITPCSFGGVSVITPGTNTSNQVAVLYQDVNCTEVPVAIHADQLTPTWRVYSTGSNVFQTRAGCLIGAEHVNNSYECDIPIGAGICASYQTQTNSPGSASSVASQSIIAYTMSLGAENSVAYSNNSIAIPTNFTISVTTEILPVSMTKTSVDCTMYICGDSTECSNLLLQYGSFCTQLNRALTGIAVEQDKNTQEVFAQVKQIYKTPPIKDFGGFNFSQILPDPSKPSKRSFIEDLLFNKVTLADAGFIKQYGDCLGDIAARDLICAQKFNGLTVLPPLLTDEMIAQYTSALLAGTITSGWTFGAGAALQIPFAMQMAYRFNGIGVTQNVLYENQKLIANQFNSAIGKIQDSLSSTASALGKLQDVVNQNAQALNTLVKQLSSNFGAISSVLNDILSRLDKVEAEVQIDRLITGRLQSLQTYVTQQLIRAAEIRASANLAATKMSECVLGQSKRVDFCGKGYHLMSFPQSAPHGVVFLHVTYVPAQEKNFTTAPAICHDGKAHFPREGVFVSNGTHWFVTQRNFYEPQIITTDNTFVSGNCDVVIGIVNNTVYDPLQPELDSFKEELDKYFKNHTSPDVDLGDISGINASVVNIQKEIDRLNEVAKNLNESLIDLQELGKYEQGGGGTGGGYIPEAPRDGQAYVRKDGEWVLLSTFLGRSLEVLFQGPGHHHHHHHHSAWSHPQFEKGGGSGGGGSGGSAWSHPQFEK

SEQ ID NO: 31 - protein, 1278 aa, synthetic construct
VNLTTRTQLPPAYTNSFTRGVYYPDKVFRSSVLHSTQDLFLPFFSNVTWFHAIHVSGTNGTKRFDNPVLPFNDGVYFASTEKSNIIRGWIFGTTLDSKTQSLLIVNNATNVVIKVCEFQFCNDPFLGVYYHKNNKSWMESEFRVYSSANNCTFEYVSQPFLMDLEGKQGNFKNLREFVFKNIDGYFKIYSKHTPINLVRDLPQGFSALEPLVDLPIGINITRFQTLLALHRSYLTPGDSSSGWTAGAAAYYVGYLQPRTFLLKYNENGTITDAVDCALDPLSETKCTLKSFTVEKGIYQTSNFRVQPTESIVRFPNITNLCPFGEVFNATRFASVYAWNRKRISNCVADYSVLYNSASFSTFKCYGVSPTKLNDLCFTNVYADSFVIRGDEVRQIAPGQTRKIADYNYKLPDDFTGCVIAWNSNNLDSKVGGNYNYLYRLFRKSNLKPFERDISTEIYQAGSTPCNGVEGFNCYFPLQSYGFQPTNGVGYQPYRVVVLSFELLHAPATVCGPKKSTNLVKNKCVNFNFNGLTGTGVLTESNKKFLPFQQFGRDIADTTDAVRDPQTLEILDITPCSFGGVSVITPGTNTSNQVAVLYQDVNCTEVPVAIHADQLTPTWRVYSTGSNVFQTRAGCLIGAEHVNNSYECDIPIGAGICASYQTQTNSPGSASSVASQSIIAYTMSLGAENSVAYSNNSIAIPTNFTISVTTEILPVSMTKTSVDCTMYICGDSTECSNLLLQYGSFCTQLNRALTGIAVEQDKNTQEVFAQVKQIYKTPPIKDFGGFNFSQILPDPSKPSKRSFIEDLLFNKVTLADAGFIKQYGDCLGDIAARDLICAQKFNGLTVLPPLLTDEMIAQYTSALLAGTITSGWTFGAGAALQIPFAMQMAYRFNGIGVTQNVLYENQKLIANQFNSAIGKIQDSLSSTASALGKLQDVVNQNAQALNTLVKQLSSNFGAISSVLNDILSRLDKVEAEVQIDRLITGRLQSLQTYVTQQLIRAAEIRASANLAATKMSECVLGQSKRVDFCGKGYHLMSFPQSAPHGVVFLHVTYVPAQEKNFTTAPAICHDGKAHFPREGVFVSNGTHWFVTQRNFYEPQIITTDNTFVSGNCDVVIGIVNNTVYDPLQPELDSFKEELDKYFKNHTSPDVDLGDISGINASVVNIQKEIDRLNEVAKNLNESLIDLQELGKYEQGGGGTGGGYIPEAPRDGQAYVRKDGEWVLLSTFLGRSLEVLFQGPGHHHHHHHHSAWSHPQFEKGGGSGGGGSGGSAWSHPQFEK

SEQ ID NO: 32 - protein, 1278 aa, synthetic construct
VNLTTRTQLPPAYTNSFTRGVYYPDKVFRSSVLHSTQDLFLPFFSNVTWFHAIHVSGTNGTKRFDNPVLPFNDGVYFASTEKSNIIRGWIFGTTLDSKTQSLLIVNNATNVVIKVCEFQFCNDPFLGVYYHKNNKSWMESEFRVYSSANNCTFEYVSQPFLMDLEGKQGNFKNLREFVFKNIDGYFKIYSKHTPINLVRDLPQGFSALEPLVDLPIGINITRFQTLLALHRSYLTPGDSSSGWTAGAAAYYVGYLQPRTFLLKYNENGTITDAVDCALDPLSETKCTLKSFTVEKGIYQTSNFRVQPTESIVRFPNITNLCPFGEVFNATRFASVYAWNRKRISNCVADYSVLYNSASFSTFKCYGVSPTRLNDLCFTNVYADSFVIRGDEVRQIAPGQTGKIADYNYKLPDDFTGCVIAWNSNNLDSKVGGNYNYLYRLFRKSNLKPFERDISTEIYQAGSTPCNGVEGFNCYFPLQSYGFQPTNGVGYQPYRVVVLSFELLHAPATVCGPKKSTNLVKNKCVNFNFNGLTGTGVLTESNKKFLPFQQFGRDIADTTDAVRDPQTLEILDITPCSFGGVSVITPGTNTSNQVAVLYQDVNCTEVPVAIHADQLTPTWRVYSTGSNVFQTRAGCLIGAEHVNNSYECDIPIGAGICASYQTQTNSPGSASSVASQSIIAYTMSLGAENSVAYSNNSIAIPTNFTISVTTEILPVSMTKTSVDCTMYICGDSTECSNLLLQYGSFCTQLNRALTGIAVEQDKNTQEVFAQVKQIYKTPPIKDFGGFNFSQILPDPSKPSKRSFIEDLLFNKVTLADAGFIKQYGDCLGDIAARDLICAQKFNGLTVLPPLLTDEMIAQYTSALLAGTITSGWTFGAGAALQIPFAMQMAYRFNGIGVTQNVLYENQKLIANQFNSAIGKIQDSLSSTASALGKLQDVVNQNAQALNTLVKQLSSNFGAISSVLNDILSRLDKVEAEVQIDRLITGRLQSLQTYVTQQLIRAAEIRASANLAATKMSECVLGQSKRVDFCGKGYHLMSFPQSAPHGVVFLHVTYVPAQEKNFTTAPAICHDGKAHFPREGVFVSNGTHWFVTQRNFYEPQIITTDNTFVSGNCDVVIGIVNNTVYDPLQPELDSFKEELDKYFKNHTSPDVDLGDISGINASVVNIQKEIDRLNEVAKNLNESLIDLQELGKYEQGGGGTGGGYIPEAPRDGQAYVRKDGEWVLLSTFLGRSLEVLFQGPGHHHHHHHHSAWSHPQFEKGGGSGGGGSGGSAWSHPQFEK

SEQ ID NO: 33 - protein, 1278 aa, synthetic construct
VNLTTRTQLPPAYTNSFTRGVYYPDKVFRSSVLHSTQDLFLPFFSNVTWFHAIHVSGTNGTKRFDNPVLPFNDGVYFASTEKSNIIRGWIFGTTLDSKTQSLLIVNNATNVVIKVCEFQFCNDPFLGVYYHKNNKSWMESEFRVYSSANNCTFEYVSQPFLMDLEGKQGNFKNLREFVFKNIDGYFKIYSKHTPINLVRDLPQGFSALEPLVDLPIGINITRFQTLLALHRSYLTPGDSSSGWTAGAAAYYVGYLQPRTFLLKYNENGTITDAVDCALDPLSETKCTLKSFTVEKGIYQTSNFRVQPTESIVRFPNITNLCPFGEVFNATRFASVYAWNRKRISNCVADYSVLYNSASFSTFKCYGVSPTKLNDLCFTNVYADSFVIRGDEVRQIAPGQTGKIADYNYKLPDDFTGCVIAWNSNNLDSKVGGNYNYLYRLFRKSNLKPFERDISTEIYQAGSTPCNGVEGFNCYFPLQSYGFQPTNGVGYQPYRVVVLSFELLHAPATVCGPKKSTNLVKNKCVNFNFNGLTGTGVLTESNKKFLPFQQFGRDIADTTDAVRDPQTLEILDITPCSFGGVSVITPGTNTSNQVAVLYQDVNCTEVPVAIHADQLTPTWRVYSTGSNVFQTRAGCLIGAEHVNNSYECDIPIGAGICASYQTQTNSPGSASSVASQSIIAYTMSLGAENSVAYSNNSIAIPTNFTISVTTEILPVSMTKTSVDCTMYICGDSTECSNLLLQYGSFCTQLNRALTGIAVEQDKNTQEVFAQVKQIYKTPPIKDFGGFNFSQILPDPSKPSKRSFIEDLLFNKVTLADAGFIKQYGDCLGDIAARDLICAQKFNGLTVLPPLLTDEMIAQYTSALLAGTITSGWTFGAGAALQIPFAMQMAYRFNGIGVTQNVLYENQKLIANQFNSAIGKIQDSLSSTASALGKLQDVVNQNAQALNTLVKQLSSNFGAISSVLNDILSRLDKWEAEVQIDRLITGRLQSLQTYVTQQLIRAAEIRASANLAATKMSECVLGQSKRVDFCGKGYHLMSFPQSAPHGVVFLHVTYVPAQEKNFTTAPAICHDGKAHFPREGVFVSNGTHWFVTQRNFYEPQIITTDNTFVSGNCDVVIGIVNNTVYDPLQPELDSFKEELDKYFKNHTSPDVDLGDISGINASVVNIQKEIDRLNEVAKNLNESLIDLQELGKYEQGGGGTGGGYIPEAPRDGQAYVRKDGEWVLLSTFLGRSLEVLFQGPGHHHHHHHHSAWSHPQFEKGGGSGGGGSGGSAWSHPQFEK

SEQ ID NO: 34 - protein, 1278 aa, synthetic construct
VNLTTRTQLPPAYTNSFTRGVYYPDKVFRSSVLHSTQDLFLPFFSNVTWFHAIHVSGTNGTKRFDNPVLPFNDGVYFASTEKSNIIRGWIFGTTLDSKTQSLLIVNNATNVVIKVCEFQFCNDPFLGVYYHKNNKSWMESEFRVYSSANNCTFEYVSQPFLMDLEGKQGNFKNLREFVFKNIDGYFKIYSKHTPINLVRDLPQGFSALEPLVDLPIGINITRFQTLLALHRSYLTPGDSSSGWTAGAAAYYVGYLQPRTFLLKYNENGTITDAVDCALDPLSETKCTLKSFTVEKGIYQTSNFRVQPTESIVRFPNITNLCPFGEVFNATRFASVYAWNRKRISNCVADYSVLYNSASFSTFKCYGVSPTKLNDLCFTNVYADSFVIRGDEVRQIAPGQTGKIADYNYKLPIDFTGCVIAWNSNNLDSKVGGNYNYLYRLFRKSNLKPFERDISTEIYQAGSTPCNGVEGFNCYFPLQSYGFQPTNGVGYQPYRVVVLSFELLHAPATVCGPKKSTNLVKNKCVNFNFNGLTGTGVLTESNKKFLPFQQFGRDIADTTDAVRDPQTLEILDITPCSFGGVSVITPGTNTSNQVAVLYQDVNCTEVPVAIHADQLTPTWRVYSTGSNVFQTRAGCLIGAEHVNNSYECDIPIGAGICASYQTQTNSPGSASSVASQSIIAYTMSLGAENSVAYSNNSIAIPTNFTISVTTEILPVSMTKTSVDCTMYICGDSTECSNLLLQYGSFCTQLNRALTGIAVEQDKNTQEVFAQVKQIYKTPPIKDFGGFNFSQILPDPSKPSKRSFIEDLLFNKVTLADAGFIKQYGDCLGDIAARDLICAQKFNGLTVLPPLLTDEMIAQYTSALLAGTITSGWTFGAGAALQIPFAMQMAYRFNGIGVTQNVLYENQKLIANQFNSAIGKIQDSLSSTASALGKLQDVVNQNAQALNTLVKQLSSNFGAISSVLNDILSRLDKVEAEVQIDRLITGRLQSLQTYVTQQLIRAAEIRASANLAATKMSECVLGQSKRVDFCGKGYHLMSFPQSAPHGVVFLHVTYVPAQEKNFTTAPAICHDGKAHFPREGVFVSNGTHWFVTQRNFYEPQIITTDNTFVSGNCDVVIGIVNNTVYDPLQPELDSFKEELDKYFKNHTSPDVDLGDISGINASVVNIQKEIDRLNEVAKNLNESLIDLQELGKYEQGGGGTGGGYIPEAPRDGQAYVRKDGEWVLLSTFLGRSLEVLFQGPGHHHHHHHHSAWSHPQFEKGGGSGGGGSGGSAWSHPQFEK

SEQ ID NO: 35 - protein, 1278 aa, synthetic construct
VNLTTRTQLPPAYTNSFTRGVYYPDKVFRSSVLHSTQDLFLPFFSNVTWFHAIHVSGTNGTKRFDNPVLPFNDGVYFASTEKSNIIRGWIFGTTLDSKTQSLLIVNNATNVVIKVCEFQFCNDPFLGVYYHKNNKSWMESEFRVYSSANNCTFEYVSQPFLMDLEGKQGNFKNLREFVFKNIDGYFKIYSKHTPINLVRDLPQGFSALEPLVDLPIGINITRFQTLLALHRSYLTPGDSSSGWTAGAAAYYVGYLQPRTFLLKYNENGTITDAVDCALDPLSETKCTLKSFTVEKGIYQTSNFRVQPTESIVRFPNITNLCPFGEVFNATRFASVYAWNRKRISNCVADYSVLYNSASFSTFKCYGVSPTKLNDLCFTNVYADSFVIRGDEVRQIAPGQTGKIARYNYKLPDDFTGCVIAWNSNNLDSKVGGNYNYLYRLFRKSNLKPFERDISTEIYQAGSTPCNGVEGFNCYFPLQSYGFQPTNGVGYQPYRVVVLSFELLHAPATVCGPKKSTNLVKNKCVNFNFNGLTGTGVLTESNKKFLPFQQFGRDIADTTDAVRDPQTLEILDITPCSFGGVSVITPGTNTSNQVAVLYQDVNCTEVPVAIHADQLTPTWRVYSTGSNVFQTRAGCLIGAEHVNNSYECDIPIGAGICASYQTQTNSPGSASSVASQSIIAYTMSLGAENSVAYSNNSIAIPTNFTISVTTEILPVSMTKTSVDCTMYICGDSTECSNLLLQYGSFCTQLNRALTGIAVEQDKNTQEVFAQVKQIYKTPPIKDFGGFNFSQILPDPSKPSKRSFIEDLLFNKVTLADAGFIKQYGDCLGDIAARDLICAQKFNGLTVLPPLLTDEMIAQYTSALLAGTITSGWTFGAGAALQIPFAMQMAYRFNGIGVTQNVLYENQKLIANQFNSAIGKIQDSLSSTASALGKLQDVVNQNAQALNTLVKQLSSNFGAISSVLNDILSRLDKVEAEVQIDRLITGRLQSLQTYVTQQLIRAAEIRASANLAATKMSECVLGQSKRVDFCGKGYHLMSFPQSAPHGVVFLHVTYVPAQEKNFTTAPAICHDGKAHFPREGVFVSNGTHWFVTQRNFYEPQIITTDNTFVSGNCDVVIGIVNNTVYDPLQPELDSFKEELDKYFKNHTSPDVDLGDISGINASVVNIQKEIDRLNEVAKNLNESLIDLQELGKYEQGGGGTGGGYIPEAPRDGQAYVRKDGEWVLLSTFLGRSLEVLFQGPGHHHHHHHHSAWSHPQFEKGGGSGGGGSGGSAWSHPQFEK

SEQ ID NO: 36 - protein, 1278 aa, synthetic construct
VNLTTRTQLPPAYTNSFTRGVYYPDKVFRSSVLHSTQDLFLPFFSNVTWFHAIHVSGTNGTKRFDNPVLPFNDGVYFASTEKSNIIRGWIFGTTLDSKTQSLLIVNNATNVVIKVCEFQFCNDPFLGVYYHKNNKSWMESEFRVYSSANNCTFEYVSQPFLMDLEGKQGNFKNLREFVFKNIDGYFKIYSKHTPINLVRDLPQGFSALEPLVDLPIGINITRFQTLLALHRSYLTPGDSSSGWTAGAAAYYVGYLQPRTFLLKYNENGTITDAVDCALDPLSETKCTLKSFTVEKGIYQTSNFRVQPTESIVRFPNITNLCPFGEVFNATRFASVYAWNRKRISNCVADYSVLYNSWSFSTFKCYGVSPTKLNDLCFTNVYADSFVIRGDEVRQIAPGQTGKIADYNYKLPDDFTGCVIAWNSNNLDSKVGGNYNYLYRLFRKSNLKPFERDISTEIYQAGSTPCNGVEGFNCYFPLQSYGFQPTNGVGYQPYRVVVLSFELLHAPATVCGPKKSTNLVKNKCVNFNFNGLTGTGVLTESNKKFLPFQQFGRDIADTTDAVRDPQTLEILDITPCSFGGVSVITPGTNTSNQVAVLYQDVNCTEVPVAIHADQLTPTWRVYSTGSNVFQTRAGCLIGAEHVNNSYECDIPIGAGICASYQTQTNSPGSASSVASQSIIAYTMSLGAENSVAYSNNSIAIPTNFTISVTTEILPVSMTKTSVDCTMYICGDSTECSNLLLQYGSFCTQLNRALTGIAVEQDKNTQEVFAQVKQIYKTPPIKDFGGFNFSQILPDPSKPSKRSFIEDLLFNKVTLADAGFIKQYGDCLGDIAARDLICAQKFNGLTVLPPLLTDEMIAQYTSALLAGTITSGWTFGAGAALQIPFAMQMAYRFNGIGVTQNVLYENQKLIANQFNSAIGKIQDSLSSTASALGKLQDVVNQNAQALNTLVKQLSSNFGAISSVLNDILSRLDKVEAEVQIDRLITGRLQSLQTYVTQQLIRAAEIRASANLAATKMSECVLGQSKRVDFCGKGYHLMSFPQSAPHGVVFLHVTYVPAQEKNFTTAPAICHDGKAHFPREGVFVSNGTHWFVTQRNFYEPQIITTDNTFVSGNCDVVIGIVNNTVYDPLQPELDSFKEELDKYFKNHTSPDVDLGDISGINASVVNIQKEIDRLNEVAKNLNESLIDLQELGKYEQGGGGTGGGYIPEAPRDGQAYVRKDGEWVLLSTFLGRSLEVLFQGPGHHHHHHHHSAWSHPQFEKGGGSGGGGSGGSAWSHPQFEK

SEQ ID NO: 37 - protein, 1278 aa, synthetic construct
VNLTTRTQLPPAYTNSFTRGVYYPDKVFRSSVLHSTQDLFLPFFSNVTWFHAIHVSGTNGTKRFDNPVLPFNDGVYFASTEKSNIIRGWIFGTTLDSKTQSLLIVNNATNVVIKVCEFQFCNDPFLGVYYHKNNKSWMESEFRVYSSANNCTFEYVSQPFLMDLEGKQGNFKNLREFVFKNIDGYFKIYSKHTPINLVRDLPQGFSALEPLVDLPIGINITRFQTLLALHRSYLTPGDSSSGWTAGAAAYYVGYLQPRTFLLKYNENGTITDAVDCALDPLSETKCTLKSFTVEKGIYQTSNFRVQPTESIVRFPNITNLCPFGEVFNATRFASVYAWNRKRISNCVADYSVLYNSASFSTFKCYGVSPTKLNDLCFTNVYADSFVIRGDEVRQIAPGQTGKIAYYNYKLPDDFTGCVIAWNSNNLDSKVGGNYNYLYRLFRKSNLKPFERDISTEIYQAGSTPCNGVEGFNCYFPLQSYGFQPTNGVGYQPYRVVVLSFELLHAPATVCGPKKSTNLVKNKCVNFNFNGLTGTGVLTESNKKFLPFQQFGRDIADTTDAVRDPQTLEILDITPCSFGGVSVITPGTNTSNQVAVLYQDVNCTEVPVAIHADQLTPTWRVYSTGSNVFQTRAGCLIGAEHVNNSYECDIPIGAGICASYQTQTNSPGSASSVASQSIIAYTMSLGAENSVAYSNNSIAIPTNFTISVTTEILPVSMTKTSVDCTMYICGDSTECSNLLLQYGSFCTQLNRALTGIAVEQDKNTQEVFAQVKQIYKTPPIKDFGGFNFSQILPDPSKPSKRSFIEDLLFNKVTLADAGFIKQYGDCLGDIAARDLICAQKFNGLTVLPPLLTDEMIAQYTSALLAGTITSGWTFGAGAALQIPFAMQMAYRFNGIGVTQNVLYENQKLIANQFNSAIGKIQDSLSSTASALGKLQDVVNQNAQALNTLVKQLSSNFGAISSVLNDILSRLDKVEAEVQIDRLITGRLQSLQTYVTQQLIRAAEIRASANLAATKMSECVLGQSKRVDFCGKGYHLMSFPQSAPHGVVFLHVTYVPAQEKNFTTAPAICHDGKAHFPREGVFVSNGTHWFVTQRNFYEPQIITTDNTFVSGNCDVVIGIVNNTVYDPLQPELDSFKEELDKYFKNHTSPDVDLGDISGINASVVNIQKEIDRLNEVAKNLNESLIDLQELGKYEQGGGGTGGGYIPEAPRDGQAYVRKDGEWVLLSTFLGRSLEVLFQGPGHHHHHHHHSAWSHPQFEKGGGSGGGGSGGSAWSHPQFEK

SEQ ID NO: 38 - protein, 1278 aa, synthetic construct
VNLTTRTQLPPAYTNSFTRGVYYPDKVFRSSVLHSTQDLFLPFFSNVTWFHAIHVSGTNGTKRFDNPVLPFNDGVYFASTEKSNIIRGWIFGTTLDSKTQSLLIVNNATNVVIKVCEFQFCNDPFLGVYYHKNNKSWMESEFRVYSSANNCTFEYVSQPFLMDLEGKQGNFKNLREFVFKNIDGYFKIYSKHTPINLVRDLPQGFSALEPLVDLPIGINITRFQTLLALHRSYLTPGDSSSGWTAGAAAYYVGYLQPRTFLLKYNENGTITDAVDCALDPLSETKCTLKSFTVEKGIYQTSNFRVQPTESIVRFPNITNLCPFGEVFNATRFASVYAWNRKRISNCVADYSVLYNSWSFSTFKCYGVSPTKLNDLCFTNVYADSFVIRGDEVRQIAPGQTGKIARYNYKLPDDFTGCVIAWNSNNLDSKVGGNYNYLYRLFRKSNLKPFERDISTEIYQAGSTPCNGVEGFNCYFPLQSYGFQPTNGVGYQPYRVVVLSFELLHAPATVCGPKKSTNLVKNKCVNFNFNGLTGTGVLTESNKKFLPFQQFGRDIADTTDAVRDPQTLEILDITPCSFGGVSVITPGTNTSNQVAVLYQDVNCTEVPVAIHADQLTPTWRVYSTGSNVFQTRAGCLIGAEHVNNSYECDIPIGAGICASYQTQTNSPGSASSVASQSIIAYTMSLGAENSVAYSNNSIAIPTNFTISVTTEILPVSMTKTSVDCTMYICGDSTECSNLLLQYGSFCTQLNRALTGIAVEQDKNTQEVFAQVKQIYKTPPIKDFGGFNFSQILPDPSKPSKRSFIEDLLFNKVTLADAGFIKQYGDCLGDIAARDLICAQKFNGLTVLPPLLTDEMIAQYTSALLAGTITSGWTFGAGAALQIPFAMQMAYRFNGIGVTQNVLYENQKLIANQFNSAIGKIQDSLSSTASALGKLQDVVNQNAQALNTLVKQLSSNFGAISSVLNDILSRLDKVEAEVQIDRLITGRLQSLQTYVTQQLIRAAEIRASANLAATKMSECVLGQSKRVDFCGKGYHLMSFPQSAPHGVVFLHVTYVPAQEKNFTTAPAICHDGKAHFPREGVFVSNGTHWFVTQRNFYEPQIITTDNTFVSGNCDVVIGIVNNTVYDPLQPELDSFKEELDKYFKNHTSPDVDLGDISGINASVVNIQKEIDRLNEVAKNLNESLIDLQELGKYEQGGGGTGGGYIPEAPRDGQAYVRKDGEWVLLSTFLGRSLEVLFQGPGHHHHHHHHSAWSHPQFEKGGGSGGGGSGGSAWSHPQFEK

SEQ ID NO: 39 - protein, 1278 aa, synthetic construct
VNLTTRTQLPPAYTNSFTRGVYYPDKVFRSSVLHSTQDLFLPFFSNVTWFHAIHVSGTNGTKRFDNPVLPFNDGVYFASTEKSNIIRGWIFGTTLDSKTQSLLIVNNATNVVIKVCEFQFCNDPFLGVYYHKNNKSWMESEFRVYSSANNCTFEYVSQPFLMDLEGKQGNFKNLREFVFKNIFGYFKIYSKHTPINLVRDLPQGFSALEPLVDLPILINITRFQTLLALHRSYLTPGDSSSGWTAGAAAYYVGYLQPRTFLLKYNENGTITDAVDCALDPLSETKCTLKSFTVEKGIYQTSNFRVQPTESIVRFPNITNLCPFGEVFNATRFASVYAWNRKRISNCVADYSVLYNSWSFSTFKCYGVSPTKLNDLCFTQVYADSFVIRGDEVRQIAPGQTGKIARYNYKLPDDFTGCVIAWNSNNLDSKVGGNYNYLYRLFRKSNLKPFERDISTEIYQAGSTPCNGVEGFNCYFPLQSYGFQPTNGVGYQPYRVVVLSFELLHAPATVCGPKKSTNLVKNKCVNFNFNGLTGTGVLTESNKKFLPFQQFGRDIADTTDAVRDPQTLEILDITPCSFGGVSVITPGTNTSNQVAVLYQDVNCTEVPVAIHADQLTPTWRVYSTGSNVFQTRAGCLIGAEHVNNSYECDIPIGAGICASYQTQTNSPGSASSVASQSIIAYTMSLGAENSVAYSNNSIAIPTNFTISVTTEILPVSMTKTSVDCTMYICGDSTECSNLLLQYGSFCTQLNRALTGIAVEQDKNTQEVFAQVKQIYKTPPIKDFGGFNFSQILPDPSKPSKRSFIEDLLFNKVTLADAGFIKQYGDCLGDIAARDLICAQKFNGLTVLPPLLTDEMIAQYTSALLAGTITSGWTFGAGAALQIPFAMQMAYRFNGIGVTQNVLYENQKLIANQFNSAIGKIQDSLSSTASALGKLQDVVNQNAQALNTLVKQLSSNFGAISSVLNDILSRLDKVEAEVQIDRLITGRLQSLQTYVTQQLIRAAEIRASANLAATKMSECVLGQSKRVDFCGKGYHLMSFPQSAPHGVVFLHVTYVPAQEKNFTTAPAICHDGKAHFPREGVFVSNGTHWFVTQRNFYEPQIITTDNTFVSGNCDVVIGIVNNTVYDPLQPELDSFKEELDKYFKNHTSPDVDLGDISGINASVVNIQKEIDRLNEVAKNLNESLIDLQELGKYEQGGGGTGGGYIPEAPRDGQAYVRKDGEWVLLSTFLGRSLEVLFQGPGHHHHHHHHSAWSHPQFEKGGGSGGGGSGGSAWSHPQFEK

SEQ ID NO: 40 - protein, 1278 aa, synthetic construct
VNLTTRTQLPPAYTNSFTRGVYYPDKVFRSSVLHSTQDLFLPFFSNVTWFHAIHVSGTNGTKRFDNPVLPFNDGVYFASTEKSNIIRGWIFGTTLDSKTQSLLIVNNATNVVIKVCEFQFCNDPFLGVYYHKNNKSWMESEFRVYSSANNCTFEYVSQPFLMDLEGKQGNFKNLREFVFKNIDGYFKIYSKHTPINLVRDLPQGFSALEPLVDLPIGINITRFQTLLALHRSYLTPGDSSSGWTAGAAAYYVGYLQPRTFLLKYNENGTITDAVDCALDPLSETKCTLKSFTVEKGIYQTSNFRVQPTESIVRFPNITNLCPFGEVFNATRFASVYAWNRKRISNCVADYSVLYNSASFSTFKCYGVSPTKLNDLCFTNVYADSFVIRGDEVRQIAPGQTGKIADYNYKLPDDFTGCVIAWNSNNLDSKVGGNYNYLYRLFRKSNLKPFERDISTEIYQAGSTPCNGVEGFNCYFPLQSYGFQPTNGVGYQPYRVVVLSFELLHAPATVCGPKKSTNLVKNKCVNFNFNGLTGTGVLTESNKKFLPFQQFGRDIADTTDAVRDPQTLEILDITPCSFGGVSVITPGTNTSNQVAVLYQDVNCTEVPVAIHADQLTPTWRVYSTGSNVFQTRAGCLIGAEHVNNSYECDIPIGAGICASYQTQTNSPGSASSVASQSIIAYTMSLGAENSVQYSNNSIAIPTNFTISVTTEILPVSMTKTSVDCTMYICGDSTECSNLLLQYGEFCTQLNRALTGIAVEQDKNTQEVFAQVKQIYKTPPIKDFGGFNFSQILPDPSKPSKRSFIEDLLFNKVTLADAGFIKQYGDCLGDIAARDKICAQKFNGLTVLPPLLTDEMIAQYTSALLAGTITSGWTFGAGAALQIPFAMQMAYRFNGIGVTQNVLYENQKLIANQFNSAIGKIQDSLSSTASALGKLQDVVNQNAQALNTLEKQLSSNFGAISSVLNDILSRLDPPEAEVQIDRLITGRLQSLQTYVTQQLIRAAEIRASANLAATKMRECVLGQSKRVDFCGKGYHLMSFPQSAPHGVVFLHVTYVPAQEKNFTTAPAICHDGKAHFPREGVFVSNGTHWFVTQRNFYEPRIITTDNTFVSGNCDVVIGIVNNTVYDPLQPELDSFKEELDKYFKNHTSPDVDLGDISGINASVVNIQKEIDRLNEVAKNLNESLIDLQELGKYEQGGGGTGGGYIPEAPRDGQAYVRKDGEWVLLSTFLGRSLEVLFQGPGHHHHHHHHSAWSHPQFEKGGGSGGGGSGGSAWSHPQFEK

SEQ ID NO: 41 - protein, 1278 aa, synthetic construct
VNLTTRTQLPPAYTNSFTRGVYYPDKVFRSSVLHSTQDLFLPFFSNVTWFHAIHVSGTNGTKRFDNPVLPFNDGVYFASTEKSNIIRGWIFGTTLDSKTQSLLIVNNATNVVIKVCEFQFCNDPFLGVYYHKNNKSWMESEFRVYSSANNCTFEYVSQPFLMDLEGKQGNFKNLREFVFKNIDGYFKIYSKHTPINLVRDLPQGFSALEPLVDLPIGINITRFQTLLALHRSYLTPGDSSSGWTAGAAAYYVGYLQPRTFLLKYNENGTITDAVDCALDPLSETKCTLKSFTVEKGIYQTSNFRVQPTESIVRFPNITNLCPFGEVFNATRFASVYAWNRKRISNCVADYSVLYNSASFSTFKCYGVSPTKLNDLCFTNVYADSFVIRGDEVRQIAPGQTGKIADYNYKLPDDFTGCVIAWNSNNLDSKVGGNYNYLYRLFRKSNLKPFERDISTEIYQAGSTPCNGVEGFNCYFPLQSYGFQPTNGVGYQPYRVVVLSFELLHAPATVCGPKKSTNLVKNKCVNFNFNGLTGTGVLTESNKKFLPFQQFGRDIADTTDAVRDPQTLEILDITPCSFGGVSVITPGTNTSNQVAVLYQDVNCTEVPVAIHADQLTPTWRVYSTGSNVFQTRAGCLIGAEHVNNSYECDIPIGAGICASYQTQTNSPGSASSVASQSIIAYTMSLGAENSVAYSNNSIAIPTNFTISVTTEILPVSMTKTSVDCTMYICGDSTECSNLLLKYGSFCTQLNRALTGIAVEQDKNTQEVFAQVKQIYKTPPIKDFGGFNFSQILPDPSKPSKRSFIEDLLFNKVTLADAGFIKQYGDCLGDIAARDKICAQKFNGLTVLPPLLTDEMIAQYTSALLAGTITSGWTFGAGNALQIPFAMQMAYRFNGIGVTQNVLYENQKLIANQFNSAIGKIQDSLSSTASALGRLQDVVNQNAQALNTLVKQLSSNFGAISSVLNDILSRLDPPEAEVQIDRLITGRLQSLQTYVTQQLIRAAEIRASANLAATKMSECVLGQSKRVDFCGRGYHLMSFPQSAPHGVVFLHVTYVPAQEKNFTTAPAICHDGKAHFPREGVFVSNGTHWFVTQRNFYEPQIITTDNTFVSGNCDVVIGIVNNTVYDPLQPELDSFKEELDKYFKNHTSPDVDLGDISGINASVVNIQKEIDRLNEVAKNLNESLIDLQELGKYEQGGGGTGGGYIPEAPRDGQAYVRKDGEWVLLSTFLGRSLEVLFQGPGHHHHHHHHSAWSHPQFEKGGGSGGGGSGGSAWSHPQFEK

SEQ ID NO: 42 - protein, 1278 aa, synthetic construct
VNLTTRTQLPPAYTNSFTRGVYYPDKVFRSSVLHSTQDLFLPFFSNVTWFHAIHVSGTNGTKRFDNPVLPFNDGVYFASTEKSNIIRGWIFGTTLDSKTQSLLIVNNATNVVIKVCEFQFCNDPFLGVYYHKNNKSWMESEFRVYSSANNCTFEYVSQPFLMDLEGKQGNFKNLREFVFKNIDGYFKIYSKHTPINLVRDLPQGFSALEPLVDLPIGINITRFQTLLALHRSYLTPGDSSSGWTAGAAAYYVGYLQPRTFLLKYNENGTITDAVDCALDPLSETKCTLKSFTVEKGIYQTSNFRVQPTESIVRFPNITNLCPFGEVFNATRFASVYAWNRKRISNCVADYSVLYNSASFSTFKCYGVSPTKLNDLCFTNVYADSFVIRGDEVRQIAPGQTGKIADYNYKLPDDFTGCVIAWNSNNLDSKVGGNYNYLYRLFRKSNLKPFERDISTEIYQAGSTPCNGVEGFNCYFPLQSYGFQPTNGVGYQPYRVVVLSFELLHAPATVCGPKKSTNLVKNKCVNFNFNGLTGTGVLTESNKKFLPFQQFGRDIADTTDAVRDPQTLEILDITPCSFGGVSVITPGTNTSNQVAVLYQDVNCTEVPVAIHADQLTPTWRVYSTGSNVFQTRAGCLIGAEHVNNSYECDIPIGAGICASYQTQTNSPGSASSVASQSIIAYTMSLGAENSVAYSNNSIAIPTNFTISVTTEILPVSMTKTSVDCTMYICGDSTECSNLLLQYGEFCTQLNRALTGIAVEQDKNTQEVFAQVKQIYKTPPIKDFGGFNFSQILPDPSKPSKRSFIEDLLFNKVTLADAGFIKQYGDCLGDIAARDKICAQKFNGLTVLPPLLTDEMIAQYTSALLAGTITSGWTFGAGAALQIPFAMQMAYRFNGIGVTQNVLYENQKLIANQFNSAIGKIQDSLSSTASALGKLQDVVNQNAQALNTLEKQLSSNFGAISSVLNDILSRLDPPEAEVQIDRLITGRLQSLQTYVTQQLIRAAEIRASANLAATKMSECVLGQSKRVDFCGKGYHLMSFPQSAPHGVVFLHVTYVPAQEKNFTTAPAICHDGKAHFPREGVFVSNGTHWFVTQRNFYEPQIITTDNTFVSGNCDVVIGIVNNTVYDPLQPELDSFKEELDKYFKNHTSPDVDLGDISGINASVVNIQKEIDRLNEVAKNLNESLIDLQELGKYEQGGGGTGGGYIPEAPRDGQAYVRKDGEWVLLSTFLGRSLEVLFQGPGHHHHHHHHSAWSHPQFEKGGGSGGGGSGGSAWSHPQFEK

SEQ ID NO: 43 - protein, 1278 aa, synthetic construct
VNLTTRTQLPPAYTNSFTRGVYYPDKVFRSSVLHSTQDLFLPFFSNVTWFHAIHVSGTNGTKRFDNPVLPFNDGVYFASTEKSNIIRGWIFGTTLDSKTQSLLIVNNATNVVIKVCEFQFCNDPFLGVYYHKNNKSWMESEFRVYSSANNCTFEYVSQPFLMDLEGKQGNFKNLREFVFKNIDGYFKIYSKHTPINLVRDLPQGFSALEPLVDLPIGINITRFQTLLALHRSYLTPGDSSSGWTAGAAAYYVGYLQPRTFLLKYNENGTITDAVDCALDPLSETKCTLKSFTVEKGIYQTSNFRVQPTESIVRFPNITNLCPFGEVFNATRFASVYAWNRKRISNCVADYSVLYNSASFSTFKCYGVSPTKLNDLCFTNVYADSFVIRGDEVRQIAPGQTGKIADYNYKLPDDFTGCVIAWNSNNLDSKVGGNYNYLYRLFRKSNLKPFERDISTEIYQAGSTPCNGVEGFNCYFPLQSYGFQPTNGVGYQPYRVVVLSFELLHAPATVCGPKKSTNLVKNKCVNFNFNGLTGTGVLTESNKKFLPFQQFGRDIADTTDAVRDPQTLEILDITPCSFGGVSVITPGTNTSNQVAVLYQDVNCTEVPVAIHADQLTPTWRVYSTGSNVFQTRAGCLIGAEHVNNSYECDIPIGAGICASYQTQTNSPGSASSVASQSIIAYTMSLGAENSVAYSNNSIAIPTNFTISVTTEILPVSMTKTSVDCTMYICGDSTECSNLLLKYGSFCTQLNRALTGIAVEQDKNTQEVFAQVKQIYKTPPIKDFGGFNFSQILPDPSKPSKRSFIEDLLFNKVTLADAGFIKQYGDCLGDIAARDLIQAQKFNGLTVLPPLLTDEMIAQYTSALLAGTITSGWTFGAGAALQIPFAMQMAYRFNGIGVTQNVLYENQKLIANQFNSAIGKIQDSLSSTASALGKLQDVVNQNAQALNELVKQLSSNFGAISSVLNDILSRLDPPEAEVQIDRLITGRLQSLQTYVTQQLIRAAEIRASANLAATKMSECVLGQSKRVDFCGKGYHLMSFPQSAPHGVVFLHVTYVPAQEKNFTTAPAICHDGKAHFPREGVFVSNGTHWFVTQRNFYEPQIITTDNTFVSGNCDVVIGIVNNTVYDPLQPELDSFKEELDKYFKNHTSPDVDLGDISGINASVVNIQKEIDRLNEVAKNLNESLIDLQELGKYEQGGGGTGGGYIPEAPRDGQAYVRKDGEWVLLSTFLGRSLEVLFQGPGHHHHHHHHSAWSHPQFEKGGGSGGGGSGGSAWSHPQFEK

SEQ ID NO: 44 - protein, 1278 aa, synthetic construct
VNLTTRTQLPPAYTNSFTRGVYYPDKVFRSSVLHSTQDLFLPFFSNVTWFHAIHVSGTNGTKRFDNPVLPFNDGVYFASTEKSNIIRGWIFGTTLDSKTQSLLIVNNATNVVIKVCEFQFCNDPFLGVYYHKNNKSWMESEFRVYSSANNCTFEYVSQPFLMDLEGKQGNFKNLREFVFKNIDGYFKIYSKHTPINLVRDLPQGFSALEPLVDLPIGINITRFQTLLALHRSYLTPGDSSSGWTAGAAAYYVGYLQPRTFLLKYNENGTITDAVDCALDPLSETKCTLKSFTVEKGIYQTSNFRVQPTESIVRFPNITNLCPFGEVFNATRFASVYAWNRKRISNCVADYSVLYNSASFSTFKCYGVSPTKLNDLCFTNVYADSFVIRGDEVRQIAPGQTGKIADYNYKLPDDFTGCVIAWNSNNLDSKVGGNYNYLYRLFRKSNLKPFERDISTEIYQAGSTPCNGVEGFNCYFPLQSYGFQPTNGVGYQPYRVVVLSFELLHAPATVCGPKKSTNLVKNKCVNFNFNGLTGTGVLTESNKKFLPFQQFGRDIADTTDAVRDPQTLEILDITPCSFGGVSVITPGTNTSNQVAVLYQDVNCTEVPVAIHADQLTPTWRVYSTGSNVFQTRAGCLIGAEHVNNSYECDIPIGAGICASYQTQTNSPGSASSVASQSIIAYTMSLGAENSVQYSNNSIAIPTNFTISVTTEILPVSMTKTSVDCTMYICGDSTECSNLLLQYGSFCTQLNRALTGIAVEQDKNTQEVFAQVKQIYKTPPIKDFGGFNFSQILPDPSKPSKRSFIEDLLFNKVTLADAGFIKQYGDCLGDIAARDLICAQKFNGLTVLPPLLTDEMIAQYTSALLAGTITSGWTFGAGAALQIPFAMQMAYRFNGIGVTQNVLYENQKLIANQFNSAIGKIQDSLSSTASALGKLQDVVNQNAQALNTLVKQLSSNFGAISSVLNDILSRLDPPEAEVQIDRLITGRLQSLQTYVTQQLIRAAEIRASANLAATKMRECVLGQSKRVDFCGKGYHLMSFPQSAPHGVVFLHVTYVPAQEKNFTTAPAICHDGKAHFPREGVFVSNGTHWFVTQRNFYEPRIITTDNTFVSGNCDVVIGIVNNTVYDPLQPELDSFKEELDKYFKNHTSPDVDLGDISGINASVVNIQKEIDRLNEVAKNLNESLIDLQELGKYEQGGGGTGGGYIPEAPRDGQAYVRKDGEWVLLSTFLGRSLEVLFQGPGHHHHHHHHSAWSHPQFEKGGGSGGGGSGGSAWSHPQFEK

SEQ ID NO: 45 - protein, 1278 aa, synthetic construct
VNLTTRTQLPPAYTNSFTRGVYYPDKVFRSSVLHSTQDLFLPFFSNVTWFHAIHVSGTNGTKRFDNPVLPFNDGVYFASTEKSNIIRGWIFGTTLDSKTQSLLIVNNATNVVIKVCEFQFCNDPFLGVYYHKNNKSWMESEFRVYSSANNCTFEYVSQPFLMDLEGKQGNFKNLREFVFKNIDGYFKIYSKHTPINLVRDLPQGFSALEPLVDLPIGINITRFQTLLALHRSYLTPGDSSSGWTAGAAAYYVGYLQPRTFLLKYNENGTITDAVDCALDPLSETKCTLKSFTVEKGIYQTSNFRVQPTESIVRFPNITNLCPFGEVFNATRFASVYAWNRKRISNCVADYSVLYNSASFSTFKCYGVSPTKLNDLCFTNVYADSFVIRGDEVRQIAPGQTGKIADYNYKLPDDFTGCVIAWNSNNLDSKVGGNYNYLYRLFRKSNLKPFERDISTEIYQAGSTPCNGVEGFNCYFPLQSYGFQPTNGVGYQPYRVVVLSFELLHAPATVCGPKKSTNLVKNKCVNFNFNGLTGTGVLTESNKKFLPFQQFGRDIADTTDAVRDPQTLEILDITPCSFGGVSVITPGTNTSNQVAVLYQDVNCTEVPVAIHADQLTPTWRVYSTGSNVFQTRAGCLIGAEHVNNSYECDIPIGAGICASYQTQTNSPGSASSVASQSIIAYTMSLGAENSVAYSNNSIAIPTNFTISVTTEILPVSMTKTSVDCTMYICGDSTECSNLLLQYGEFCTQLNRALTGIAVEQDKNTQEVFAQVKQIYKTPPIKDFGGFNFSQILPDPSKPSKRSFIEDLLFNKVTLADAGFIKQYGDCLGDIAARDLICAQKFNGLTVLPPLLTDEMIAQYTSALLAGTITSGWTFGAGAALQIPFAMQMAYRFNGIGVRQNVLYENQKLIANQFNSAIGKIQDSLSSTASALGRLQDVVNQNAQALNTLVKQLSSNFGAISSVLNDILSRLDPPEAEVQIDRLITGRLQSLQTYVTQQLIRAAEIRASANLAATKMSECVLGQSKRVDFCGKGYHLMSFPQSAPHGVVFLHVTYVPAQEKNFTTAPAICHDGKAHFPREGVFVSNGTHWFVTQRNFYEPQIITTDNTFVSGNCDVVIGIVNNTVYDPLQPELDSFKEELDKYFKNHTSPDVDLGDISGINASVVNIQKEIDRLNEVAKNLNESLIDLQELGKYEQGGGGTGGGYIPEAPRDGQAYVRKDGEWVLLSTFLGRSLEVLFQGPGHHHHHHHHSAWSHPQFEKGGGSGGGGSGGSAWSHPQFEK

SEQ ID NO: 46 - protein, 1278 aa, synthetic construct
VNLTTRTQLPPAYTNSFTRGVYYPDKVFRSSVLHSTQDLFLPFFSNVTWFHAIHVSGTNGTKRFDNPVLPFNDGVYFASTEKSNIIRGWIFGTTLDSKTQSLLIVNNATNVVIKVCEFQFCNDPFLGVYYHKNNKSWMESEFRVYSSANNCTFEYVSQPFLMDLEGKQGNFKNLREFVFKNIDGYFKIYSKHTPINLVRDLPQGFSALEPLVDLPIGINITRFQTLLALHRSYLTPGDSSSGWTAGAAAYYVGYLQPRTFLLKYNENGTITDAVDCALDPLSETKCTLKSFTVEKGIYQTSNFRVQPTESIVRFPNITNLCPFGEVFNATRFASVYAWNRKRISNCVADYSVLYNSASFSTFKCYGVSPTKLNDLCFTNVYADSFVIRGDEVRQIAPGQTGKIADYNYKLPDDFTGCVIAWNSNNLDSKVGGNYNYLYRLFRKSNLKPFERDISTEIYQAGSTPCNGVEGFNCYFPLQSYGFQPTNGVGYQPYRVVVLSFELLHAPATVCGPKKSTNLVKNKCVNFNFNGLTGTGVLTESNKKFLPFQQFGRDIADTTDAVRDPQTLEILDITPCSFGGVSVITPGTNTSNQVAVLYQDVNCTEVPVAIHADQLTPTWRVYSTGSNVFQTRAGCLIGAEHVNNSYECDIPIGAGICASYQTQTNSPGSASSVASQSIIAYTMSLGAENSVAYSNNSIAIPTNFTISVTTEILPVSMTKTSVDCTMYICGDSTECSNLLLQYGSFCTQLNRALTGIAVEQDKNTQEVFAQVKQIYKTPPIKDFGGFNFSQILPDPSKPSKRSFIEDLLFNKVTLADAGFIKQYGDCLGDIAARDKICAQKFNGLTVLPPLLTDEMIAQYTSALLAGTITSGWTFGAGAALQIPFAMQMAYRFNGIGVTQNVLYENQKLIANQFNSAIGKIQDSLSSTASALGKLQDVVNQNAQALNTLVKQLSSNFGAISSVLNDILSRLDPPEAEVQIDRLITGRLQSLQTYVTQQLIRAAEIRASANLAATKMSECVLGQSKRVDFCGKGYHLMSFPQSAPHGVVFLHVTYVPAQEKNFTTAPAICHDGKAHFPREGVFVSNGTHWFVTQRNFYEPQIITTDNTFVSGNCDVVIGIVNNTVYDPLQPELDSFKEELDKYFKNHTSPDVDLGDISGINASVVNIQKEIDRLNEVAKNLNESLIDLQELGKYEQGGGGTGGGYIPEAPRDGQAYVRKDGEWVLLSTFLGRSLEVLFQGPGHHHHHHHHSAWSHPQFEKGGGSGGGGSGGSAWSHPQFEK

SEQ ID NO: 47 - protein, 1278 aa, synthetic construct
VNLTTRTQLPPAYTNSFTRGVYYPDKVFRSSVLHSTQDLFLPFFSNVTWFHAIHVSGTNGTKRFDNPVLPFNDGVYFASTEKSNIIRGWIFGTTLDSKTQSLLIVNNATNVVIKVCEFQFCNDPFLGVYYHKNNKSWMESEFRVYSSANNCTFEYVSQPFLMDLEGKQGNFKNLREFVFKNIDGYFKIYSKHTPINLVRDLPQGFSALEPLVDLPIGINITRFQTLLALHRSYLTPGDSSSGWTAGAAAYYVGYLQPRTFLLKYNENGTITDAVDCALDPLSETKCTLKSFTVEKGIYQTSNFRVQPTESIVRFPNITNLCPFGEVFNATRFASVYAWNRKRISNCVADYSVLYNSASFSTFKCYGVSPTKLNDLCFTNVYADSFVIRGDEVRQIAPGQTGKIADYNYKLPDDFTGCVIAWNSNNLDSKVGGNYNYLYRLFRKSNLKPFERDISTEIYQAGSTPCNGVEGFNCYFPLQSYGFQPTNGVGYQPYRVVVLSFELLHAPATVCGPKKSTNLVKNKCVNFNFNGLTGTGVLTESNKKFLPFQQFGRDIADTTDAVRDPQTLEILDITPCSFGGVSVITPGTNTSNQVAVLYQDVNCTEVPVAIHADQLTPTWRVYSTGSNVFQTRAGCLIGAEHVNNSYECDIPIGAGICASYQTQTNSPGSASSVASQSIIAYTMSLGAENSVAYSNNSIAIPTNFTISVTTEILPVSMTKTSVDCTMYICGDSTECSNLLLQYGSFCTQLNRALTGIAVEQDKNTQEVFAQVKQIYKTPPIKDFGGFNFSQILPDPSKPSKRSFIEDLLFNKVTLADAGFIKQYGDCLGDIAARDLICAQKFNGLTVLPPLLTDEMIAQYTSALLAGTITSGWTFGAGAALQIPFAMQMAYRFNGIGVTQNVLYENQKLIANQFNSAIGKIQDSLSSTASALGKLQDVVNQNAQALNELVKQLSSNFGAISSVLNDILSRLDPPEAEVQIDRLITGRLQSLQTYVTQQLIRAAEIRASANLAATKMSECVLGQSKRVDFCGKGYHLMSFPQSAPHGVVFLHVTYVPAQEKNFTTAPAICHDGKAHFPREGVFVSNGTHWFVTQRNFYEPQIITTDNTFVSGNCDVVIGIVNNTVYDPLQPELDSFKEELDKYFKNHTSPDVDLGDISGINASVVNIQKEIDRLNEVAKNLNESLIDLQELGKYEQGGGGTGGGYIPEAPRDGQAYVRKDGEWVLLSTFLGRSLEVLFQGPGHHHHHHHHSAWSHPQFEKGGGSGGGGSGGSAWSHPQFEK

SEQ ID NO: 48 - protein, 19 aa, synthetic construct
MDWTWRFLFVVAAATGVQS

SEQ ID NO: 49 - protein, 19 aa, synthetic construct
MDWTWRFLFVVAAATGVQS

SEQ ID NO: 50 - DNA, 3897 bp, synthetic construct
  source 1..3897: mol_type = other DNA
atggattggacctggcggttcctgtttgtggtggctgctgctacaggcgtgcagagcgtgaacctgaccaccagaacacagctgcctccagcctacaccaacagcttcaccagaggcgtgtactaccccgacaaggtgttcagatccagcgtgctgcactctacccaggacctgttcctgcctttcttcagcaacgtgacctggttccacgccatccacgtgtccggcaccaatggcaccaagagattcgacaaccccgtgctgcccttcaacgacggggtgtactttgccagcaccgagaagtccaacatcatcagaggctggatcttcggcaccacactggacagcaagacccagagcctgctgatcgtgaacaacgccaccaacgtggtcatcaaagtgtgcgagttccagttctgcaacgaccccttcctgggcgtctactaccacaagaacaacaagagctggatggaaagcgagttccgggtgtacagcagcgccaacaactgcaccttcgagtacgtgtcccagcctttcctgatggacctggaaggcaagcagggcaacttcaagaacctgcgcgagttcgtgttcaagaacatcgacggctacttcaagatctacagcaagcacacccctatcaacctcgtgcgggatctgcctcagggcttctctgctctggaacccctggtggatctgcccatcggcatcaacatcacccggtttcagacactgctggccctgcacagaagctacctgacacctggcgatagcagctctggatggacagctggcgccgctgcctactatgtgggatacctgcagcctcggaccttcctgctgaagtacaacgagaacggcaccatcaccgacgccgtggattgtgctctggatcctctgagcgagacaaagtgcaccctgaagtccttcaccgtggaaaagggcatctaccagaccagcaacttccgggtgcagcccaccgaatccatcgtgcggttccccaatatcaccaatctgtgccccttcggcgaggtgttcaatgccaccagattcgcctctgtgtacgcctggaaccggaagcggatcagcaattgcgtggccgactactccgtgctgtacaactccgccagcttcagcaccttcaagtgctacggcgtgtcccctaccaagctgaacgacctgtgcttcacaaacgtgtacgccgacagcttcgtgatccggggagatgaagtgcggcagattgcccctggacagacaggcaagatcgccgactacaactacaagctgcccgacgacttcaccggctgtgtgattgcctggaacagcaacaacctggactccaaagtcggcggcaactacaattacctgtaccggctgttccggaagtccaatctgaagcccttcgagcgggacatctccaccgagatctatcaggccggcagcaccccttgtaacggcgtggaaggcttcaactgctacttcccactgcagtcctacggctttcagcccacaaatggcgtgggctaccagccttacagagtggtggtgctgagcttcgagctgctgcatgctcctgccacagtgtgcggccctaagaaaagcaccaatctcgtgaagaacaaatgcgtgaacttcaacttcaacggcctgaccggaaccggcgtgctgacagagagcaacaagaagttcctgccattccagcagttcggccgggatatcgccgataccacagatgccgtcagagatccccagacactggaaatcctggacatcaccccttgcagcttcggcggagtgtctgtgatcacccctggcaccaacaccagcaatcaggtggcagtgctgtaccaggacgtgaactgtaccgaagtgcccgtggccattcacgccgatcagctgacacctacatggcgggtgtactccaccggcagcaatgtgtttcagaccagagccggctgtctgatcggagccgagcacgtgaacaatagctacgagtgcgacatccccatcggcgctggcatctgcgcctcttaccagacacagacaaacagccctggcagcgcctcttctgtggccagccagagcatcattgcctacacaatgtctctgggcgccgagaacagcgtggcctactccaacaactctatcgctatccccaccaacttcaccatcagcgtgaccacagagatcctgcctgtgtccatgaccaagaccagcgtggactgcaccatgtacatctgcggcgattccaccgagtgctccaacctgctgctgcagtacggcagcttctgcacccagctgaatagagccctgaccgggatcgccgtggaacaggacaagaacacccaagaggtgttcgcccaagtgaagcagatctacaagacccctcctatcaaggacttcggcggcttcaatttcagccagattctgcccgatcctagcaagcccagcaagcggagcttcatcgaggacctgctgttcaacaaagtgacactggccgacgccggcttcatcaagcagtatggcgattgtctgggcgacattgccgccagggatctgatttgcgcccagaagtttaacggactgacagtgctgcctcctctgctgaccgatgagatgatcgcccagtacacatctgccctgctggccggcacaatcacaagcggctggacatttggagctggcgctgccctgcagatcccctttgctatgcagatggcctaccggttcaacggcatcggagtgacccagaatgtgctgtacgagaaccagaagctgatcgccaaccagttcaacagcgccatcggcaagatccaggacagcctgagcagcacagcaagcgccctgggaaagctgcaggacgtggtcaaccagaatgcccaggcactgaacaccctggtcaagcagctgtctagcaacttcggcgccatcagctctgtgctgaacgatatcctgagcagactggacaaacatgaggccgaggtgcagatcgacagactgatcacaggcagactgcagagcctccagacatacgtgacccagcagctgatcagagccgccgagattagagcctctgccaatctggccgccaccaagatgtctgagtgtgtgctgggccagagcaagagagtggacttttgcggcaagggctaccacctgatgagcttccctcagtctgcccctcacggcgtggtgtttctgcacgtgacatatgtgcccgctcaagagaagaatttcaccaccgctccagccatctgccacgacggcaaagcccactttcctagagaaggcgtgttcgtgtccaacggcacccattggttcgtgacacagcggaacttctacgagccccagatcatcaccaccgacaacaccttcgtgtctggcaactgcgacgtcgtgatcggcattgtgaacaataccgtgtacgaccctctgcagcccgagctggacagcttcaaagaggaactggacaagtactttaagaaccacacaagccccgacgtggacctgggcgatatcagcggaatcaatgccagcgtcgtgaacatccagaaagagatcgaccggctgaacgaggtggccaagaatttaaatgagagcctgatcgacctgcaagaactggggaagtacgagcaaggcggcggaggaacaggcggaggctatattcctgaggctcccagagatggccaggcctacgttagaaaggatggcgagtgggtgctgctgtccacctttctgggaagatctctggaagtgctgtttcaaggccctggccaccaccatcatcaccatcaccacagcgcttggagccatcctcagttcgagaaaggcggtggaagcggaggcggaggttctggcggatctgcttggtcacacccacagtttgagaagtgatga

SEQ ID NO: 51 - DNA, 3897 bp, synthetic construct
  source 1..3897: mol_type = other DNA
atggattggacctggcggttcctgtttgtggtggctgctgctacaggcgtgcagagcgtgaacctgaccaccagaacacagctgcctccagcctacaccaacagcttcaccagaggcgtgtactaccccgacaaggtgttcagatccagcgtgctgcactctacccaggacctgttcctgcctttcttcagcaacgtgacctggttccacgccatccacgtgtccggcaccaatggcaccaagagattcgacaaccccgtgctgcccttcaacgacggggtgtactttgccagcaccgagaagtccaacatcatcagaggctggatcttcggcaccacactggacagcaagacccagagcctgctgatcgtgaacaacgccaccaacgtggtcatcaaagtgtgcgagttccagttctgcaacgaccccttcctgggcgtctactaccacaagaacaacaagagctggatggaaagcgagttccgggtgtacagcagcgccaacaactgcaccttcgagtacgtgtcccagcctttcctgatggacctggaaggcaagcagggcaacttcaagaacctgcgcgagttcgtgttcaagaacatcgacggctacttcaagatctacagcaagcacacccctatcaacctcgtgcgggatctgcctcagggcttctctgctctggaacccctggtggatctgcccatcggcatcaacatcacccggtttcagacactgctggccctgcacagaagctacctgacacctggcgatagcagctctggatggacagctggcgccgctgcctactatgtgggatacctgcagcctcggaccttcctgctgaagtacaacgagaacggcaccatcaccgacgccgtggattgtgctctggatcctctgagcgagacaaagtgcaccctgaagtccttcaccgtggaaaagggcatctaccagaccagcaacttccgggtgcagcccaccgaatccatcgtgcggttccccaatatcaccaatctgtgccccttcggcgaggtgttcaatgccaccagattcgcctctgtgtacgcctggaaccggaagcggatcagcaattgcgtggccgactactccgtgctgtacaactccgccagcttcagcaccttcaagtgctacggcgtgtcccctaccaagctgaacgacctgtgcttcacaaacgtgtacgccgacagcttcgtgatccggggagatgaagtgcggcagattgcccctggacagacaggcaagatcgccgactacaactacaagctgcccgacgacttcaccggctgtgtgattgcctggaacagcaacaacctggactccaaagtcggcggcaactacaattacctgtaccggctgttccggaagtccaatctgaagcccttcgagcgggacatctccaccgagatctatcaggccggcagcaccccttgtaacggcgtggaaggcttcaactgctacttcccactgcagtcctacggctttcagcccacaaatggcgtgggctaccagccttacagagtggtggtgctgagcttcgagctgctgcatgctcctgccacagtgtgcggccctaagaaaagcaccaatctcgtgaagaacaaatgcgtgaacttcaacttcaacggcctgaccggaaccggcgtgctgacagagagcaacaagaagttcctgccattccagcagttcggccgggatatcgccgataccacagatgccgtcagagatccccagacactggaaatcctggacatcaccccttgcagcttcggcggagtgtctgtgatcacccctggcaccaacaccagcaatcaggtggcagtgctgtaccaggacgtgaactgtaccgaagtgcccgtggccattcacgccgatcagctgacacctacatggcgggtgtactccaccggcagcaatgtgtttcagaccagagccggctgtctgatcggagccgagcacgtgaacaatagctacgagtgcgacatccccatcggcgctggcatctgcgcctcttaccagacacagacaaacagccctggcagcgcctcttctgtggccagccagagcatcattgcctacacaatgtctctgggcgccgagaacagcgtggcctactccaacaactctatcgctatccccaccaacttcaccatcagcgtgaccacagagatcctgcctgtgtccatgaccaagaccagcgtggactgcaccatgtacatctgcggcgattccaccgagtgctccaacctgctgctgcagtacggcagcttctgcacccagctgaatagagccctgaccgggatcgccgtggaacaggacaagaacacccaagaggtgttcgcccaagtgaagcagatctacaagacccctcctatcaaggacttcggcggcttcaatttcagccagattctgcccgatcctagcaagcccagcaagcggagcttcatcgaggacctgctgttcaacaaagtgacactggccgacgccggcttcatcaagcagtatggcgattgtctgggcgacattgccgccagggatctgatttgcgcccagaagtttaacggactgacagtgctgcctcctctgctgaccgatgagatgatcgcccagtacacatctgccctgctggccggcacaatcacaagcggctggacatttggagctggcgctgccctgcagatcccctttgctatgcagatggcctaccggttcaacggcatcggagtgacccagaatgtgctgtacgagaaccagaagctgatcgccaaccagttcaacagcgccatcggcaagatccaggacagcctgagcagcacagcaagcgccctgggaaagctgcaggacgtggtcaaccagaatgcccaggcactgaacaccctggtcaagcagctgtctagcaacttcggcgccatcagctctgtgctgaacgatatcctgagcagactgttaaaagttgaggccgaggtgcagatcgacagactgatcacaggcagactgcagagcctccagacatacgtgacccagcagctgatcagagccgccgagattagagcctctgccaatctggccgccaccaagatgtctgagtgtgtgctgggccagagcaagagagtggacttttgcggcaagggctaccacctgatgagcttccctcagtctgcccctcacggcgtggtgtttctgcacgtgacatatgtgcccgctcaagagaagaatttcaccaccgctccagccatctgccacgacggcaaagcccactttcctagagaaggcgtgttcgtgtccaacggcacccattggttcgtgacacagcggaacttctacgagccccagatcatcaccaccgacaacaccttcgtgtctggcaactgcgacgtcgtgatcggcattgtgaacaataccgtgtacgaccctctgcagcccgagctggacagcttcaaagaggaactggacaagtactttaagaaccacacaagccccgacgtggacctgggcgatatcagcggaatcaatgccagcgtcgtgaacatccagaaagagatcgaccggctgaacgaggtggccaagaatttaaatgagagcctgatcgacctgcaagaactggggaagtacgagcaaggcggcggaggaacaggcggaggctatattcctgaggctcccagagatggccaggcctacgttagaaaggatggcgagtgggtgctgctgtccacctttctgggaagatctctggaagtgctgtttcaaggccctggccaccaccatcatcaccatcaccacagcgcttggagccatcctcagttcgagaaaggcggtggaagcggaggcggaggttctggcggatctgcttggtcacacccacagtttgagaagtgatga

SEQ ID NO: 52 - DNA, 3897 bp, synthetic construct
  source 1..3897: mol_type = other DNA
atggattggacctggcggttcctgtttgtggtggctgctgctacaggcgtgcagagcgtgaacctgaccaccagaacacagctgcctccagcctacaccaacagcttcaccagaggcgtgtactaccccgacaaggtgttcagatccagcgtgctgcactctacccaggacctgttcctgcctttcttcagcaacgtgacctggttccacgccatccacgtgtccggcaccaatggcaccaagagattcgacaaccccgtgctgcccttcaacgacggggtgtactttgccagcaccgagaagtccaacatcatcagaggctggatcttcggcaccacactggacagcaagacccagagcctgctgatcgtgaacaacgccaccaacgtggtcatcaaagtgtgcgagttccagttctgcaacgaccccttcctgggcgtctactaccacaagaacaacaagagctggatggaaagcgagttccgggtgtacagcagcgccaacaactgcaccttcgagtacgtgtcccagcctttcctgatggacctggaaggcaagcagggcaacttcaagaacctgcgcgagttcgtgttcaagaacatcgacggctacttcaagatctacagcaagcacacccctatcaacctcgtgcgggatctgcctcagggcttctctgctctggaacccctggtggatctgcccatcggcatcaacatcacccggtttcagacactgctggccctgcacagaagctacctgacacctggcgatagcagctctggatggacagctggcgccgctgcctactatgtgggatacctgcagcctcggaccttcctgctgaagtacaacgagaacggcaccatcaccgacgccgtggattgtgctctggatcctctgagcgagacaaagtgcaccctgaagtccttcaccgtggaaaagggcatctaccagaccagcaacttccgggtgcagcccaccgaatccatcgtgcggttccccaatatcaccaatctgtgccccttcggcgaggtgttcaatgccaccagattcgcctctgtgtacgcctggaaccggaagcggatcagcaattgcgtggccgactactccgtgctgtacaactccgccagcttcagcaccttcaagtgctacggcgtgtcccctaccaagctgaacgacctgtgcttcacaaacgtgtacgccgacagcttcgtgatccggggagatgaagtgcggcagattgcccctggacagacaggcaagatcgccgactacaactacaagctgcccgacgacttcaccggctgtgtgattgcctggaacagcaacaacctggactccaaagtcggcggcaactacaattacctgtaccggctgttccggaagtccaatctgaagcccttcgagcgggacatctccaccgagatctatcaggccggcagcaccccttgtaacggcgtggaaggcttcaactgctacttcccactgcagtcctacggctttcagcccacaaatggcgtgggctaccagccttacagagtggtggtgctgagcttcgagctgctgcatgctcctgccacagtgtgcggccctaagaaaagcaccaatctcgtgaagaacaaatgcgtgaacttcaacttcaacggcctgaccggaaccggcgtgctgacagagagcaacaagaagttcctgccattccagcagttcggccgggatatcgccgataccacagatgccgtcagagatccccagacactggaaatcctggacatcaccccttgcagcttcggcggagtgtctgtgatcacccctggcaccaacaccagcaatcaggtggcagtgctgtaccaggacgtgaactgtaccgaagtgcccgtggccattcacgccgatcagctgacacctacatggcgggtgtactccaccggcagcaatgtgtttcagaccagagccggctgtctgatcggagccgagcacgtgaacaatagctacgagtgcgacatccccatcggcgctggcatctgcgcctcttaccagacacagacaaacagccctggcagcgcctcttctgtggccagccagagcatcattgcctacacaatgtctctgggcgccgagaacagcgtggcctactccaacaactctatcgctatccccaccaacttcaccatcagcgtgaccacagagatcctgcctgtgtccatgaccaagaccagcgtggactgcaccatgtacatctgcggcgattccaccgagtgctccaacctgctgctgcagtacggcagcttctgcacccagctgaatagagccctgaccgggatcgccgtggaacaggacaagaacacccaagaggtgttcgcccaagtgaagcagatctacaagacccctcctatcaaggacttcggcggcttcaatttcagccagattctgcccgatcctagcaagcccagcaagcggagcttcatcgaggacctgctgttcaacaaagtgacactggccgacgccggcttcatcaagcagtatggcgattgtctgggcgacattgccgccagggatctgatttgcgcccagaagtttaacggactgacagtgctgcctcctctgctgaccgatgagatgatcgcccagtacacatctgccctgctggccggcacaatcacaagcggctggacatttggagctggcgctgccctgcagatcccctttgctatgcagatggcctaccggttcaacggcatcggagtgacccagaatgtgctgtacgagaaccagaagctgatcgccaaccagttcaacagcgccatcggcaagatccaggacagcctgagcagcacagcaagcgccctgggaaagctgcaggacgtggtcaaccagaatgcccaggcactgaacaccctggtcaagcagctgtctagcaacttcggcgccatcagctctgtgctgaacgatatcctgttcagactggacaaagttgaggccgaggtgcagatcgacagactgatcacaggcagactgcagagcctccagacatacgtgacccagcagctgatcagagccgccgagattagagcctctgccaatctggccgccaccaagatgtctgagtgtgtgctgggccagagcaagagagtggacttttgcggcaagggctaccacctgatgagcttccctcagtctgcccctcacggcgtggtgtttctgcacgtgacatatgtgcccgctcaagagaagaatttcaccaccgctccagccatctgccacgacggcaaagcccactttcctagagaaggcgtgttcgtgtccaacggcacccattggttcgtgacacagcggaacttctacgagccccagatcatcaccaccgacaacaccttcgtgtctggcaactgcgacgtcgtgatcggcattgtgaacaataccgtgtacgaccctctgcagcccgagctggacagcttcaaagaggaactggacaagtactttaagaaccacacaagccccgacgtggacctgggcgatatcagcggaatcaatgccagcgtcgtgaacatccagaaagagatcgaccggctgaacgaggtggccaagaatttaaatgagagcctgatcgacctgcaagaactggggaagtacgagcaaggcggcggaggaacaggcggaggctatattcctgaggctcccagagatggccaggcctacgttagaaaggatggcgagtgggtgctgctgtccacctttctgggaagatctctggaagtgctgtttcaaggccctggccaccaccatcatcaccatcaccacagcgcttggagccatcctcagttcgagaaaggcggtggaagcggaggcggaggttctggcggatctgcttggtcacacccacagtttgagaagtgatga

SEQ ID NO: 53 - DNA, 3897 bp, synthetic construct
  source 1..3897: mol_type = other DNA
atggattggacctggcggttcctgtttgtggtggctgctgctacaggcgtgcagagcgtgaacctgaccaccagaacacagctgcctccagcctacaccaacagcttcaccagaggcgtgtactaccccgacaaggtgttcagatccagcgtgctgcactctacccaggacctgttcctgcctttcttcagcaacgtgacctggttccacgccatccacgtgtccggcaccaatggcaccaagagattcgacaaccccgtgctgcccttcaacgacggggtgtactttgccagcaccgagaagtccaacatcatcagaggctggatcttcggcaccacactggacagcaagacccagagcctgctgatcgtgaacaacgccaccaacgtggtcatcaaagtgtgcgagttccagttctgcaacgaccccttcctgggcgtctactaccacaagaacaacaagagctggatggaaagcgagttccgggtgtacagcagcgccaacaactgcaccttcgagtacgtgtcccagcctttcctgatggacctggaaggcaagcagggcaacttcaagaacctgcgcgagttcgtgttcaagaacatcgacggctacttcaagatctacagcaagcacacccctatcaacctcgtgcgggatctgcctcagggcttctctgctctggaacccctggtggatctgcccatcggcatcaacatcacccggtttcagacactgctggccctgcacagaagctacctgacacctggcgatagcagctctggatggacagctggcgccgctgcctactatgtgggatacctgcagcctcggaccttcctgctgaagtacaacgagaacggcaccatcaccgacgccgtggattgtgctctggatcctctgagcgagacaaagtgcaccctgaagtccttcaccgtggaaaagggcatctaccagaccagcaacttccgggtgcagcccaccgaatccatcgtgcggttccccaatatcaccaatctgtgccccttcggcgaggtgttcaatgccaccagattcgcctctgtgtacgcctggaaccggaagcggatcagcaattgcgtggccgactactccgtgctgtacaactccgccagcttcagcaccttcaagtgctacggcgtgtcccctaccaagctgaacgacctgtgcttcacaaacgtgtacgccgacagcttcgtgatccggggagatgaagtgcggcagattgcccctggacagacaggcaagatcgccgactacaactacaagctgcccgacgacttcaccggctgtgtgattgcctggaacagcaacaacctggactccaaagtcggcggcaactacaattacctgtaccggctgttccggaagtccaatctgaagcccttcgagcgggacatctccaccgagatctatcaggccggcagcaccccttgtaacggcgtggaaggcttcaactgctacttcccactgcagtcctacggctttcagcccacaaatggcgtgggctaccagccttacagagtggtggtgctgagcttcgagtatctgcatgctcctgccacagtgtgcggccctaagaaaagcaccaatctcgtgaagaacaaatgcgtgaacttcaacttcaacggcctgaccggaaccggcgtgctgacagagagcaacaagaagttcctgccattccagcagttcggccgggatatcgccgataccacagatgccgtcagagatccccagacactggaaatcctggacatcaccccttgcagcttcggcggagtgtctgtgatcacccctggcaccaacaccagcaatcaggtggcagtgctgtaccaggacgtgaactgtaccgaagtgcccgtggccattcacgccgatcagctgacacctacatggcgggtgtactccaccggcagcaatgtgtttcagaccagagccggctgtctgatcggagccgagcacgtgaacaatagctacgagtgcgacatccccatcggcgctggcatctgcgcctcttaccagacacagacaaacagccctggcagcgcctcttctgtggccagccagagcatcattgcctacacaatgtctctgggcgccgagaacagcgtggcctactccaacaactctatcgctatccccaccaacttcaccatcagcgtgaccacagagatcctgcctgtgtccatgaccaagaccagcgtggactgcaccatgtacatctgcggcgattccaccgagtgctccaacctgctgctgcagtacggcagcttctgcacccagctgaatagagccctgaccgggatcgccgtggaacaggacaagaacacccaagaggtgttcgcccaagtgaagcagatctacaagacccctcctatcaaggacttcggcggcttcaatttcagccagattctgcccgatcctagcaagcccagcaagcggagcttcatcgaggacctgctgttcaacaaagtgacactggccgacgccggcttcatcaagcagtatggcgattgtctgggcgacattgccgccagggatctgatttgcgcccagaagtttaacggactgacagtgctgcctcctctgctgaccgatgagatgatcgcccagtacacatctgccctgctggccggcacaatcacaagcggctggacatttggagctggcgctgccctgcagatcccctttgctatgcagatggcctaccggttcaacggcatcggagtgacccagaatgtgctgtacgagaaccagaagctgatcgccaaccagttcaacagcgccatcggcaagatccaggacagcctgagcagcacagcaagcgccctgggaaagctgcaggacgtggtcaaccagaatgcccaggcactgaacaccctggtcaagcagctgtctagcaacttcggcgccatcagctctgtgctgaacgatatcctgagcagactggacaaagttgaggccgaggtgcagatcgacagactgatcacaggcagactgcagagcctccagacatacgtgacccagcagctgatcagagccgccgagattagagcctctgccaatctggccgccaccaagatgtctgagtgtgtgctgggccagagcaagagagtggacttttgcggcaagggctaccacctgatgagcttccctcagtctgcccctcacggcgtggtgtttctgcacgtgacatatgtgcccgctcaagagaagaatttcaccaccgctccagccatctgccacgacggcaaagcccactttcctagagaaggcgtgttcgtgtccaacggcacccattggttcgtgacacagcggaacttctacgagccccagatcatcaccaccgacaacaccttcgtgtctggcaactgcgacgtcgtgatcggcattgtgaacaataccgtgtacgaccctctgcagcccgagctggacagcttcaaagaggaactggacaagtactttaagaaccacacaagccccgacgtggacctgggcgatatcagcggaatcaatgccagcgtcgtgaacatccagaaagagatcgaccggctgaacgaggtggccaagaatttaaatgagagcctgatcgacctgcaagaactggggaagtacgagcaaggcggcggaggaacaggcggaggctatattcctgaggctcccagagatggccaggcctacgttagaaaggatggcgagtgggtgctgctgtccacctttctgggaagatctctggaagtgctgtttcaaggccctggccaccaccatcatcaccatcaccacagcgcttggagccatcctcagttcgagaaaggcggtggaagcggaggcggaggttctggcggatctgcttggtcacacccacagtttgagaagtgatga

SEQ ID NO: 54 - DNA, 3897 bp, synthetic construct
  source 1..3897: mol_type = other DNA
atggattggacctggcggttcctgtttgtggtggctgctgctacaggcgtgcagagcgtgaacctgaccaccagaacacagctgcctccagcctacaccaacagcttcaccagaggcgtgtactaccccgacaaggtgttcagatccagcgtgctgcactctacccaggacctgttcctgcctttcttcagcaacgtgacctggttccacgccatccacgtgtccggcaccaatggcaccaagagattcgacaaccccgtgctgcccttcaacgacggggtgtactttgccagcaccgagaagtccaacatcatcagaggctggatcttcggcaccacactggacagcaagacccagagcctgctgatcgtgaacaacgccaccaacgtggtcatcaaagtgtgcgagttccagttctgcaacgaccccttcctgggcgtctactaccacaagaacaacaagagctggatggaaagcgagttccgggtgtacagcagcgccaacaactgcaccttcgagtacgtgtcccagcctttcctgatggacctggaaggcaagcagggcaacttcaagaacctgcgcgagttcgtgttcaagaacatcgacggctacttcaagatctacagcaagcacacccctatcaacctcgtgcgggatctgcctcagggcttctctgctctggaacccctggtggatctgcccatcggcatcaacatcacccggtttcagacactgctggccctgcacagaagctacctgacacctggcgatagcagctctggatggacagctggcgccgctgcctactatgtgggatacctgcagcctcggaccttcctgctgaagtacaacgagaacggcaccatcaccgacgccgtggattgtgctctggatcctctgagcgagacaaagtgcaccctgaagtccttcaccgtggaaaagggcatctaccagaccagcaacttccgggtgcagcccaccgaatccatcgtgcggttccccaatatcaccaatctgtgccccttcggcgaggtgttcaatgccaccagattcgcctctgtgtacgcctggaaccggaagcggatcagcaattgcgtggccgactactccgtgctgtacaactccgccagcttcagcaccttcaagtgctacggcgtgtcccctaccaagctgaacgacctgtgcttcacaaacgtgtacgccgacagcttcgtgatccggggagatgaagtgcggcagattgcccctggacagacacgcaagatcgccgactacaactacaagctgcccgacgacttcaccggctgtgtgattgcctggaacagcaacaacctggactccaaagtcggcggcaactacaattacctgtaccggctgttccggaagtccaatctgaagcccttcgagcgggacatctccaccgagatctatcaggccggcagcaccccttgtaacggcgtggaaggcttcaactgctacttcccactgcagtcctacggctttcagcccacaaatggcgtgggctaccagccttacagagtggtggtgctgagcttcgagctgctgcatgctcctgccacagtgtgcggccctaagaaaagcaccaatctcgtgaagaacaaatgcgtgaacttcaacttcaacggcctgaccggaaccggcgtgctgacagagagcaacaagaagttcctgccattccagcagttcggccgggatatcgccgataccacagatgccgtcagagatccccagacactggaaatcctggacatcaccccttgcagcttcggcggagtgtctgtgatcacccctggcaccaacaccagcaatcaggtggcagtgctgtaccaggacgtgaactgtaccgaagtgcccgtggccattcacgccgatcagctgacacctacatggcgggtgtactccaccggcagcaatgtgtttcagaccagagccggctgtctgatcggagccgagcacgtgaacaatagctacgagtgcgacatccccatcggcgctggcatctgcgcctcttaccagacacagacaaacagccctggcagcgcctcttctgtggccagccagagcatcattgcctacacaatgtctctgggcgccgagaacagcgtggcctactccaacaactctatcgctatccccaccaacttcaccatcagcgtgaccacagagatcctgcctgtgtccatgaccaagaccagcgtggactgcaccatgtacatctgcggcgattccaccgagtgctccaacctgctgctgcagtacggcagcttctgcacccagctgaatagagccctgaccgggatcgccgtggaacaggacaagaacacccaagaggtgttcgcccaagtgaagcagatctacaagacccctcctatcaaggacttcggcggcttcaatttcagccagattctgcccgatcctagcaagcccagcaagcggagcttcatcgaggacctgctgttcaacaaagtgacactggccgacgccggcttcatcaagcagtatggcgattgtctgggcgacattgccgccagggatctgatttgcgcccagaagtttaacggactgacagtgctgcctcctctgctgaccgatgagatgatcgcccagtacacatctgccctgctggccggcacaatcacaagcggctggacatttggagctggcgctgccctgcagatcccctttgctatgcagatggcctaccggttcaacggcatcggagtgacccagaatgtgctgtacgagaaccagaagctgatcgccaaccagttcaacagcgccatcggcaagatccaggacagcctgagcagcacagcaagcgccctgggaaagctgcaggacgtggtcaaccagaatgcccaggcactgaacaccctggtcaagcagctgtctagcaacttcggcgccatcagctctgtgctgaacgatatcctgagcagactggacaaagttgaggccgaggtgcagatcgacagactgatcacaggcagactgcagagcctccagacatacgtgacccagcagctgatcagagccgccgagattagagcctctgccaatctggccgccaccaagatgtctgagtgtgtgctgggccagagcaagagagtggacttttgcggcaagggctaccacctgatgagcttccctcagtctgcccctcacggcgtggtgtttctgcacgtgacatatgtgcccgctcaagagaagaatttcaccaccgctccagccatctgccacgacggcaaagcccactttcctagagaaggcgtgttcgtgtccaacggcacccattggttcgtgacacagcggaacttctacgagccccagatcatcaccaccgacaacaccttcgtgtctggcaactgcgacgtcgtgatcggcattgtgaacaataccgtgtacgaccctctgcagcccgagctggacagcttcaaagaggaactggacaagtactttaagaaccacacaagccccgacgtggacctgggcgatatcagcggaatcaatgccagcgtcgtgaacatccagaaagagatcgaccggctgaacgaggtggccaagaatttaaatgagagcctgatcgacctgcaagaactggggaagtacgagcaaggcggcggaggaacaggcggaggctatattcctgaggctcccagagatggccaggcctacgttagaaaggatggcgagtgggtgctgctgtccacctttctgggaagatctctggaagtgctgtttcaaggccctggccaccaccatcatcaccatcaccacagcgcttggagccatcctcagttcgagaaaggcggtggaagcggaggcggaggttctggcggatctgcttggtcacacccacagtttgagaagtgatga

SEQ ID NO: 55 - DNA, 3897 bp, synthetic construct
  source 1..3897: mol_type = other DNA
atggattggacctggcggttcctgtttgtggtggctgctgctacaggcgtgcagagcgtgaacctgaccaccagaacacagctgcctccagcctacaccaacagcttcaccagaggcgtgtactaccccgacaaggtgttcagatccagcgtgctgcactctacccaggacctgttcctgcctttcttcagcaacgtgacctggttccacgccatccacgtgtccggcaccaatggcaccaagagattcgacaaccccgtgctgcccttcaacgacggggtgtactttgccagcaccgagaagtccaacatcatcagaggctggatcttcggcaccacactggacagcaagacccagagcctgctgatcgtgaacaacgccaccaacgtggtcatcaaagtgtgcgagttccagttctgcaacgaccccttcctgggcgtctactaccacaagaacaacaagagctggatggaaagcgagttccgggtgtacagcagcgccaacaactgcaccttcgagtacgtgtcccagcctttcctgatggacctggaaggcaagcagggcaacttcaagaacctgcgcgagttcgtgttcaagaacatcgacggctacttcaagatctacagcaagcacacccctatcaacctcgtgcgggatctgcctcagggcttctctgctctggaacccctggtggatctgcccatcggcatcaacatcacccggtttcagacactgctggccctgcacagaagctacctgacacctggcgatagcagctctggatggacagctggcgccgctgcctactatgtgggatacctgcagcctcggaccttcctgctgaagtacaacgagaacggcaccatcaccgacgccgtggattgtgctctggatcctctgagcgagacaaagtgcaccctgaagtccttcaccgtggaaaagggcatctaccagaccagcaacttccgggtgcagcccaccgaatccatcgtgcggttccccaatatcaccaatctgtgccccttcggcgaggtgttcaatgccaccagattcgcctctgtgtacgcctggaaccggaagcggatcagcaattgcgtggccgactactccgtgctgtacaactccgccagcttcagcaccttcaagtgctacggcgtgtcccctaccagactgaacgacctgtgcttcacaaacgtgtacgccgacagcttcgtgatccggggagatgaagtgcggcagattgcccctggacagacaggcaagatcgccgactacaactacaagctgcccgacgacttcaccggctgtgtgattgcctggaacagcaacaacctggactccaaagtcggcggcaactacaattacctgtaccggctgttccggaagtccaatctgaagcccttcgagcgggacatctccaccgagatctatcaggccggcagcaccccttgtaacggcgtggaaggcttcaactgctacttcccactgcagtcctacggctttcagcccacaaatggcgtgggctaccagccttacagagtggtggtgctgagcttcgagctgctgcatgctcctgccacagtgtgcggccctaagaaaagcaccaatctcgtgaagaacaaatgcgtgaacttcaacttcaacggcctgaccggaaccggcgtgctgacagagagcaacaagaagttcctgccattccagcagttcggccgggatatcgccgataccacagatgccgtcagagatccccagacactggaaatcctggacatcaccccttgcagcttcggcggagtgtctgtgatcacccctggcaccaacaccagcaatcaggtggcagtgctgtaccaggacgtgaactgtaccgaagtgcccgtggccattcacgccgatcagctgacacctacatggcgggtgtactccaccggcagcaatgtgtttcagaccagagccggctgtctgatcggagccgagcacgtgaacaatagctacgagtgcgacatccccatcggcgctggcatctgcgcctcttaccagacacagacaaacagccctggcagcgcctcttctgtggccagccagagcatcattgcctacacaatgtctctgggcgccgagaacagcgtggcctactccaacaactctatcgctatccccaccaacttcaccatcagcgtgaccacagagatcctgcctgtgtccatgaccaagaccagcgtggactgcaccatgtacatctgcggcgattccaccgagtgctccaacctgctgctgcagtacggcagcttctgcacccagctgaatagagccctgaccgggatcgccgtggaacaggacaagaacacccaagaggtgttcgcccaagtgaagcagatctacaagacccctcctatcaaggacttcggcggcttcaatttcagccagattctgcccgatcctagcaagcccagcaagcggagcttcatcgaggacctgctgttcaacaaagtgacactggccgacgccggcttcatcaagcagtatggcgattgtctgggcgacattgccgccagggatctgatttgcgcccagaagtttaacggactgacagtgctgcctcctctgctgaccgatgagatgatcgcccagtacacatctgccctgctggccggcacaatcacaagcggctggacatttggagctggcgctgccctgcagatcccctttgctatgcagatggcctaccggttcaacggcatcggagtgacccagaatgtgctgtacgagaaccagaagctgatcgccaaccagttcaacagcgccatcggcaagatccaggacagcctgagcagcacagcaagcgccctgggaaagctgcaggacgtggtcaaccagaatgcccaggcactgaacaccctggtcaagcagctgtctagcaacttcggcgccatcagctctgtgctgaacgatatcctgagcagactggacaaagttgaggccgaggtgcagatcgacagactgatcacaggcagactgcagagcctccagacatacgtgacccagcagctgatcagagccgccgagattagagcctctgccaatctggccgccaccaagatgtctgagtgtgtgctgggccagagcaagagagtggacttttgcggcaagggctaccacctgatgagcttccctcagtctgcccctcacggcgtggtgtttctgcacgtgacatatgtgcccgctcaagagaagaatttcaccaccgctccagccatctgccacgacggcaaagcccactttcctagagaaggcgtgttcgtgtccaacggcacccattggttcgtgacacagcggaacttctacgagccccagatcatcaccaccgacaacaccttcgtgtctggcaactgcgacgtcgtgatcggcattgtgaacaataccgtgtacgaccctctgcagcccgagctggacagcttcaaagaggaactggacaagtactttaagaaccacacaagccccgacgtggacctgggcgatatcagcggaatcaatgccagcgtcgtgaacatccagaaagagatcgaccggctgaacgaggtggccaagaatttaaatgagagcctgatcgacctgcaagaactggggaagtacgagcaaggcggcggaggaacaggcggaggctatattcctgaggctcccagagatggccaggcctacgttagaaaggatggcgagtgggtgctgctgtccacctttctgggaagatctctggaagtgctgtttcaaggccctggccaccaccatcatcaccatcaccacagcgcttggagccatcctcagttcgagaaaggcggtggaagcggaggcggaggttctggcggatctgcttggtcacacccacagtttgagaagtgatga

SEQ ID NO: 56 - DNA, 3897 bp, synthetic construct
  source 1..3897: mol_type = other DNA
atggattggacctggcggttcctgtttgtggtggctgctgctacaggcgtgcagagcgtgaacctgaccaccagaacacagctgcctccagcctacaccaacagcttcaccagaggcgtgtactaccccgacaaggtgttcagatccagcgtgctgcactctacccaggacctgttcctgcctttcttcagcaacgtgacctggttccacgccatccacgtgtccggcaccaatggcaccaagagattcgacaaccccgtgctgcccttcaacgacggggtgtactttgccagcaccgagaagtccaacatcatcagaggctggatcttcggcaccacactggacagcaagacccagagcctgctgatcgtgaacaacgccaccaacgtggtcatcaaagtgtgcgagttccagttctgcaacgaccccttcctgggcgtctactaccacaagaacaacaagagctggatggaaagcgagttccgggtgtacagcagcgccaacaactgcaccttcgagtacgtgtcccagcctttcctgatggacctggaaggcaagcagggcaacttcaagaacctgcgcgagttcgtgttcaagaacatcgacggctacttcaagatctacagcaagcacacccctatcaacctcgtgcgggatctgcctcagggcttctctgctctggaacccctggtggatctgcccatcggcatcaacatcacccggtttcagacactgctggccctgcacagaagctacctgacacctggcgatagcagctctggatggacagctggcgccgctgcctactatgtgggatacctgcagcctcggaccttcctgctgaagtacaacgagaacggcaccatcaccgacgccgtggattgtgctctggatcctctgagcgagacaaagtgcaccctgaagtccttcaccgtggaaaagggcatctaccagaccagcaacttccgggtgcagcccaccgaatccatcgtgcggttccccaatatcaccaatctgtgccccttcggcgaggtgttcaatgccaccagattcgcctctgtgtacgcctggaaccggaagcggatcagcaattgcgtggccgactactccgtgctgtacaactccgccagcttcagcaccttcaagtgctacggcgtgtcccctaccaagctgaacgacctgtgcttcacaaacgtgtacgccgacagcttcgtgatccggggagatgaagtgcggcagattgcccctggacagacaggcaagatcgccgactacaactacaagctgcccgacgacttcaccggctgtgtgattgcctggaacagcaacaacctggactccaaagtcggcggcaactacaattacctgtaccggctgttccggaagtccaatctgaagcccttcgagcgggacatctccaccgagatctatcaggccggcagcaccccttgtaacggcgtggaaggcttcaactgctacttcccactgcagtcctacggctttcagcccacaaatggcgtgggctaccagccttacagagtggtggtgctgagcttcgagctgctgcatgctcctgccacagtgtgcggccctaagaaaagcaccaatctcgtgaagaacaaatgcgtgaacttcaacttcaacggcctgaccggaaccggcgtgctgacagagagcaacaagaagttcctgccattccagcagttcggccgggatatcgccgataccacagatgccgtcagagatccccagacactggaaatcctggacatcaccccttgcagcttcggcggagtgtctgtgatcacccctggcaccaacaccagcaatcaggtggcagtgctgtaccaggacgtgaactgtaccgaagtgcccgtggccattcacgccgatcagctgacacctacatggcgggtgtactccaccggcagcaatgtgtttcagaccagagccggctgtctgatcggagccgagcacgtgaacaatagctacgagtgcgacatccccatcggcgctggcatctgcgcctcttaccagacacagacaaacagccctggcagcgcctcttctgtggccagccagagcatcattgcctacacaatgtctctgggcgccgagaacagcgtggcctactccaacaactctatcgctatccccaccaacttcaccatcagcgtgaccacagagatcctgcctgtgtccatgaccaagaccagcgtggactgcaccatgtacatctgcggcgattccaccgagtgctccaacctgctgctgcagtacggcagcttctgcacccagctgaatagagccctgaccgggatcgccgtggaacaggacaagaacacccaagaggtgttcgcccaagtgaagcagatctacaagacccctcctatcaaggacttcggcggcttcaatttcagccagattctgcccgatcctagcaagcccagcaagcggagcttcatcgaggacctgctgttcaacaaagtgacactggccgacgccggcttcatcaagcagtatggcgattgtctgggcgacattgccgccagggatctgatttgcgcccagaagtttaacggactgacagtgctgcctcctctgctgaccgatgagatgatcgcccagtacacatctgccctgctggccggcacaatcacaagcggctggacatttggagctggcgctgccctgcagatcccctttgctatgcagatggcctaccggttcaacggcatcggagtgacccagaatgtgctgtacgagaaccagaagctgatcgccaaccagttcaacagcgccatcggcaagatccaggacagcctgagcagcacagcaagcgccctgggaaagctgcaggacgtggtcaaccagaatgcccaggcactgaacaccctggtcaagcagctgtctagcaacttcggcgccatcagctctgtgctgaacgatatcctgagcagactggacaaatgggaggccgaggtgcagatcgacagactgatcacaggcagactgcagagcctccagacatacgtgacccagcagctgatcagagccgccgagattagagcctctgccaatctggccgccaccaagatgtctgagtgtgtgctgggccagagcaagagagtggacttttgcggcaagggctaccacctgatgagcttccctcagtctgcccctcacggcgtggtgtttctgcacgtgacatatgtgcccgctcaagagaagaatttcaccaccgctccagccatctgccacgacggcaaagcccactttcctagagaaggcgtgttcgtgtccaacggcacccattggttcgtgacacagcggaacttctacgagccccagatcatcaccaccgacaacaccttcgtgtctggcaactgcgacgtcgtgatcggcattgtgaacaataccgtgtacgaccctctgcagcccgagctggacagcttcaaagaggaactggacaagtactttaagaaccacacaagccccgacgtggacctgggcgatatcagcggaatcaatgccagcgtcgtgaacatccagaaagagatcgaccggctgaacgaggtggccaagaatttaaatgagagcctgatcgacctgcaagaactggggaagtacgagcaaggcggcggaggaacaggcggaggctatattcctgaggctcccagagatggccaggcctacgttagaaaggatggcgagtgggtgctgctgtccacctttctgggaagatctctggaagtgctgtttcaaggccctggccaccaccatcatcaccatcaccacagcgcttggagccatcctcagttcgagaaaggcggtggaagcggaggcggaggttctggcggatctgcttggtcacacccacagtttgagaagtgatga

SEQ ID NO: 57 - DNA, 3897 bp, synthetic construct
  source 1..3897: mol_type = other DNA
atggattggacctggcggttcctgtttgtggtggctgctgctacaggcgtgcagagcgtgaacctgaccaccagaacacagctgcctccagcctacaccaacagcttcaccagaggcgtgtactaccccgacaaggtgttcagatccagcgtgctgcactctacccaggacctgttcctgcctttcttcagcaacgtgacctggttccacgccatccacgtgtccggcaccaatggcaccaagagattcgacaaccccgtgctgcccttcaacgacggggtgtactttgccagcaccgagaagtccaacatcatcagaggctggatcttcggcaccacactggacagcaagacccagagcctgctgatcgtgaacaacgccaccaacgtggtcatcaaagtgtgcgagttccagttctgcaacgaccccttcctgggcgtctactaccacaagaacaacaagagctggatggaaagcgagttccgggtgtacagcagcgccaacaactgcaccttcgagtacgtgtcccagcctttcctgatggacctggaaggcaagcagggcaacttcaagaacctgcgcgagttcgtgttcaagaacatcgacggctacttcaagatctacagcaagcacacccctatcaacctcgtgcgggatctgcctcagggcttctctgctctggaacccctggtggatctgcccatcggcatcaacatcacccggtttcagacactgctggccctgcacagaagctacctgacacctggcgatagcagctctggatggacagctggcgccgctgcctactatgtgggatacctgcagcctcggaccttcctgctgaagtacaacgagaacggcaccatcaccgacgccgtggattgtgctctggatcctctgagcgagacaaagtgcaccctgaagtccttcaccgtggaaaagggcatctaccagaccagcaacttccgggtgcagcccaccgaatccatcgtgcggttccccaatatcaccaatctgtgccccttcggcgaggtgttcaatgccaccagattcgcctctgtgtacgcctggaaccggaagcggatcagcaattgcgtggccgactactccgtgctgtacaactccgccagcttcagcaccttcaagtgctacggcgtgtcccctaccaagctgaacgacctgtgcttcacaaacgtgtacgccgacagcttcgtgatccggggagatgaagtgcggcagattgcccctggacagacaggcaagatcgccgactacaactacaagctgcccatcgacttcaccggctgtgtgattgcctggaacagcaacaacctggactccaaagtcggcggcaactacaattacctgtaccggctgttccggaagtccaatctgaagcccttcgagcgggacatctccaccgagatctatcaggccggcagcaccccttgtaacggcgtggaaggcttcaactgctacttcccactgcagtcctacggctttcagcccacaaatggcgtgggctaccagccttacagagtggtggtgctgagcttcgagctgctgcatgctcctgccacagtgtgcggccctaagaaaagcaccaatctcgtgaagaacaaatgcgtgaacttcaacttcaacggcctgaccggaaccggcgtgctgacagagagcaacaagaagttcctgccattccagcagttcggccgggatatcgccgataccacagatgccgtcagagatccccagacactggaaatcctggacatcaccccttgcagcttcggcggagtgtctgtgatcacccctggcaccaacaccagcaatcaggtggcagtgctgtaccaggacgtgaactgtaccgaagtgcccgtggccattcacgccgatcagctgacacctacatggcgggtgtactccaccggcagcaatgtgtttcagaccagagccggctgtctgatcggagccgagcacgtgaacaatagctacgagtgcgacatccccatcggcgctggcatctgcgcctcttaccagacacagacaaacagccctggcagcgcctcttctgtggccagccagagcatcattgcctacacaatgtctctgggcgccgagaacagcgtggcctactccaacaactctatcgctatccccaccaacttcaccatcagcgtgaccacagagatcctgcctgtgtccatgaccaagaccagcgtggactgcaccatgtacatctgcggcgattccaccgagtgctccaacctgctgctgcagtacggcagcttctgcacccagctgaatagagccctgaccgggatcgccgtggaacaggacaagaacacccaagaggtgttcgcccaagtgaagcagatctacaagacccctcctatcaaggacttcggcggcttcaatttcagccagattctgcccgatcctagcaagcccagcaagcggagcttcatcgaggacctgctgttcaacaaagtgacactggccgacgccggcttcatcaagcagtatggcgattgtctgggcgacattgccgccagggatctgatttgcgcccagaagtttaacggactgacagtgctgcctcctctgctgaccgatgagatgatcgcccagtacacatctgccctgctggccggcacaatcacaagcggctggacatttggagctggcgctgccctgcagatcccctttgctatgcagatggcctaccggttcaacggcatcggagtgacccagaatgtgctgtacgagaaccagaagctgatcgccaaccagttcaacagcgccatcggcaagatccaggacagcctgagcagcacagcaagcgccctgggaaagctgcaggacgtggtcaaccagaatgcccaggcactgaacaccctggtcaagcagctgtctagcaacttcggcgccatcagctctgtgctgaacgatatcctgagcagactggacaaagttgaggccgaggtgcagatcgacagactgatcacaggcagactgcagagcctccagacatacgtgacccagcagctgatcagagccgccgagattagagcctctgccaatctggccgccaccaagatgtctgagtgtgtgctgggccagagcaagagagtggacttttgcggcaagggctaccacctgatgagcttccctcagtctgcccctcacggcgtggtgtttctgcacgtgacatatgtgcccgctcaagagaagaatttcaccaccgctccagccatctgccacgacggcaaagcccactttcctagagaaggcgtgttcgtgtccaacggcacccattggttcgtgacacagcggaacttctacgagccccagatcatcaccaccgacaacaccttcgtgtctggcaactgcgacgtcgtgatcggcattgtgaacaataccgtgtacgaccctctgcagcccgagctggacagcttcaaagaggaactggacaagtactttaagaaccacacaagccccgacgtggacctgggcgatatcagcggaatcaatgccagcgtcgtgaacatccagaaagagatcgaccggctgaacgaggtggccaagaatttaaatgagagcctgatcgacctgcaagaactggggaagtacgagcaaggcggcggaggaacaggcggaggctatattcctgaggctcccagagatggccaggcctacgttagaaaggatggcgagtgggtgctgctgtccacctttctgggaagatctctggaagtgctgtttcaaggccctggccaccaccatcatcaccatcaccacagcgcttggagccatcctcagttcgagaaaggcggtggaagcggaggcggaggttctggcggatctgcttggtcacacccacagtttgagaagtgatga

SEQ ID NO: 58 - DNA, 3897 bp, synthetic construct
  source 1..3897: mol_type = other DNA
atggattggacctggcggttcctgtttgtggtggctgctgctacaggcgtgcagagcgtgaacctgaccaccagaacacagctgcctccagcctacaccaacagcttcaccagaggcgtgtactaccccgacaaggtgttcagatccagcgtgctgcactctacccaggacctgttcctgcctttcttcagcaacgtgacctggttccacgccatccacgtgtccggcaccaatggcaccaagagattcgacaaccccgtgctgcccttcaacgacggggtgtactttgccagcaccgagaagtccaacatcatcagaggctggatcttcggcaccacactggacagcaagacccagagcctgctgatcgtgaacaacgccaccaacgtggtcatcaaagtgtgcgagttccagttctgcaacgaccccttcctgggcgtctactaccacaagaacaacaagagctggatggaaagcgagttccgggtgtacagcagcgccaacaactgcaccttcgagtacgtgtcccagcctttcctgatggacctggaaggcaagcagggcaacttcaagaacctgcgcgagttcgtgttcaagaacatcgacggctacttcaagatctacagcaagcacacccctatcaacctcgtgcgggatctgcctcagggcttctctgctctggaacccctggtggatctgcccatcggcatcaacatcacccggtttcagacactgctggccctgcacagaagctacctgacacctggcgatagcagctctggatggacagctggcgccgctgcctactatgtgggatacctgcagcctcggaccttcctgctgaagtacaacgagaacggcaccatcaccgacgccgtggattgtgctctggatcctctgagcgagacaaagtgcaccctgaagtccttcaccgtggaaaagggcatctaccagaccagcaacttccgggtgcagcccaccgaatccatcgtgcggttccccaatatcaccaatctgtgccccttcggcgaggtgttcaatgccaccagattcgcctctgtgtacgcctggaaccggaagcggatcagcaattgcgtggccgactactccgtgctgtacaactccgccagcttcagcaccttcaagtgctacggcgtgtcccctaccaagctgaacgacctgtgcttcacaaacgtgtacgccgacagcttcgtgatccggggagatgaagtgcggcagattgcccctggacagacaggcaagatcgcccgttacaactacaagctgcccgacgacttcaccggctgtgtgattgcctggaacagcaacaacctggactccaaagtcggcggcaactacaattacctgtaccggctgttccggaagtccaatctgaagcccttcgagcgggacatctccaccgagatctatcaggccggcagcaccccttgtaacggcgtggaaggcttcaactgctacttcccactgcagtcctacggctttcagcccacaaatggcgtgggctaccagccttacagagtggtggtgctgagcttcgagctgctgcatgctcctgccacagtgtgcggccctaagaaaagcaccaatctcgtgaagaacaaatgcgtgaacttcaacttcaacggcctgaccggaaccggcgtgctgacagagagcaacaagaagttcctgccattccagcagttcggccgggatatcgccgataccacagatgccgtcagagatccccagacactggaaatcctggacatcaccccttgcagcttcggcggagtgtctgtgatcacccctggcaccaacaccagcaatcaggtggcagtgctgtaccaggacgtgaactgtaccgaagtgcccgtggccattcacgccgatcagctgacacctacatggcgggtgtactccaccggcagcaatgtgtttcagaccagagccggctgtctgatcggagccgagcacgtgaacaatagctacgagtgcgacatccccatcggcgctggcatctgcgcctcttaccagacacagacaaacagccctggcagcgcctcttctgtggccagccagagcatcattgcctacacaatgtctctgggcgccgagaacagcgtggcctactccaacaactctatcgctatccccaccaacttcaccatcagcgtgaccacagagatcctgcctgtgtccatgaccaagaccagcgtggactgcaccatgtacatctgcggcgattccaccgagtgctccaacctgctgctgcagtacggcagcttctgcacccagctgaatagagccctgaccgggatcgccgtggaacaggacaagaacacccaagaggtgttcgcccaagtgaagcagatctacaagacccctcctatcaaggacttcggcggcttcaatttcagccagattctgcccgatcctagcaagcccagcaagcggagcttcatcgaggacctgctgttcaacaaagtgacactggccgacgccggcttcatcaagcagtatggcgattgtctgggcgacattgccgccagggatctgatttgcgcccagaagtttaacggactgacagtgctgcctcctctgctgaccgatgagatgatcgcccagtacacatctgccctgctggccggcacaatcacaagcggctggacatttggagctggcgctgccctgcagatcccctttgctatgcagatggcctaccggttcaacggcatcggagtgacccagaatgtgctgtacgagaaccagaagctgatcgccaaccagttcaacagcgccatcggcaagatccaggacagcctgagcagcacagcaagcgccctgggaaagctgcaggacgtggtcaaccagaatgcccaggcactgaacaccctggtcaagcagctgtctagcaacttcggcgccatcagctctgtgctgaacgatatcctgagcagactggacaaagttgaggccgaggtgcagatcgacagactgatcacaggcagactgcagagcctccagacatacgtgacccagcagctgatcagagccgccgagattagagcctctgccaatctggccgccaccaagatgtctgagtgtgtgctgggccagagcaagagagtggacttttgcggcaagggctaccacctgatgagcttccctcagtctgcccctcacggcgtggtgtttctgcacgtgacatatgtgcccgctcaagagaagaatttcaccaccgctccagccatctgccacgacggcaaagcccactttcctagagaaggcgtgttcgtgtccaacggcacccattggttcgtgacacagcggaacttctacgagccccagatcatcaccaccgacaacaccttcgtgtctggcaactgcgacgtcgtgatcggcattgtgaacaataccgtgtacgaccctctgcagcccgagctggacagcttcaaagaggaactggacaagtactttaagaaccacacaagccccgacgtggacctgggcgatatcagcggaatcaatgccagcgtcgtgaacatccagaaagagatcgaccggctgaacgaggtggccaagaatttaaatgagagcctgatcgacctgcaagaactggggaagtacgagcaaggcggcggaggaacaggcggaggctatattcctgaggctcccagagatggccaggcctacgttagaaaggatggcgagtgggtgctgctgtccacctttctgggaagatctctggaagtgctgtttcaaggccctggccaccaccatcatcaccatcaccacagcgcttggagccatcctcagttcgagaaaggcggtggaagcggaggcggaggttctggcggatctgcttggtcacacccacagtttgagaagtgatga

SEQ ID NO: 59 - DNA, 3897 bp, synthetic construct
  source 1..3897: mol_type = other DNA
atggattggacctggcggttcctgtttgtggtggctgctgctacaggcgtgcagagcgtgaacctgaccaccagaacacagctgcctccagcctacaccaacagcttcaccagaggcgtgtactaccccgacaaggtgttcagatccagcgtgctgcactctacccaggacctgttcctgcctttcttcagcaacgtgacctggttccacgccatccacgtgtccggcaccaatggcaccaagagattcgacaaccccgtgctgcccttcaacgacggggtgtactttgccagcaccgagaagtccaacatcatcagaggctggatcttcggcaccacactggacagcaagacccagagcctgctgatcgtgaacaacgccaccaacgtggtcatcaaagtgtgcgagttccagttctgcaacgaccccttcctgggcgtctactaccacaagaacaacaagagctggatggaaagcgagttccgggtgtacagcagcgccaacaactgcaccttcgagtacgtgtcccagcctttcctgatggacctggaaggcaagcagggcaacttcaagaacctgcgcgagttcgtgttcaagaacatcgacggctacttcaagatctacagcaagcacacccctatcaacctcgtgcgggatctgcctcagggcttctctgctctggaacccctggtggatctgcccatcggcatcaacatcacccggtttcagacactgctggccctgcacagaagctacctgacacctggcgatagcagctctggatggacagctggcgccgctgcctactatgtgggatacctgcagcctcggaccttcctgctgaagtacaacgagaacggcaccatcaccgacgccgtggattgtgctctggatcctctgagcgagacaaagtgcaccctgaagtccttcaccgtggaaaagggcatctaccagaccagcaacttccgggtgcagcccaccgaatccatcgtgcggttccccaatatcaccaatctgtgccccttcggcgaggtgttcaatgccaccagattcgcctctgtgtacgcctggaaccggaagcggatcagcaattgcgtggccgactactccgtgctgtacaactcctggagcttcagcaccttcaagtgctacggcgtgtcccctaccaagctgaacgacctgtgcttcacaaacgtgtacgccgacagcttcgtgatccggggagatgaagtgcggcagattgcccctggacagacaggcaagatcgccgactacaactacaagctgcccgacgacttcaccggctgtgtgattgcctggaacagcaacaacctggactccaaagtcggcggcaactacaattacctgtaccggctgttccggaagtccaatctgaagcccttcgagcgggacatctccaccgagatctatcaggccggcagcaccccttgtaacggcgtggaaggcttcaactgctacttcccactgcagtcctacggctttcagcccacaaatggcgtgggctaccagccttacagagtggtggtgctgagcttcgagctgctgcatgctcctgccacagtgtgcggccctaagaaaagcaccaatctcgtgaagaacaaatgcgtgaacttcaacttcaacggcctgaccggaaccggcgtgctgacagagagcaacaagaagttcctgccattccagcagttcggccgggatatcgccgataccacagatgccgtcagagatccccagacactggaaatcctggacatcaccccttgcagcttcggcggagtgtctgtgatcacccctggcaccaacaccagcaatcaggtggcagtgctgtaccaggacgtgaactgtaccgaagtgcccgtggccattcacgccgatcagctgacacctacatggcgggtgtactccaccggcagcaatgtgtttcagaccagagccggctgtctgatcggagccgagcacgtgaacaatagctacgagtgcgacatccccatcggcgctggcatctgcgcctcttaccagacacagacaaacagccctggcagcgcctcttctgtggccagccagagcatcattgcctacacaatgtctctgggcgccgagaacagcgtggcctactccaacaactctatcgctatccccaccaacttcaccatcagcgtgaccacagagatcctgcctgtgtccatgaccaagaccagcgtggactgcaccatgtacatctgcggcgattccaccgagtgctccaacctgctgctgcagtacggcagcttctgcacccagctgaatagagccctgaccgggatcgccgtggaacaggacaagaacacccaagaggtgttcgcccaagtgaagcagatctacaagacccctcctatcaaggacttcggcggcttcaatttcagccagattctgcccgatcctagcaagcccagcaagcggagcttcatcgaggacctgctgttcaacaaagtgacactggccgacgccggcttcatcaagcagtatggcgattgtctgggcgacattgccgccagggatctgatttgcgcccagaagtttaacggactgacagtgctgcctcctctgctgaccgatgagatgatcgcccagtacacatctgccctgctggccggcacaatcacaagcggctggacatttggagctggcgctgccctgcagatcccctttgctatgcagatggcctaccggttcaacggcatcggagtgacccagaatgtgctgtacgagaaccagaagctgatcgccaaccagttcaacagcgccatcggcaagatccaggacagcctgagcagcacagcaagcgccctgggaaagctgcaggacgtggtcaaccagaatgcccaggcactgaacaccctggtcaagcagctgtctagcaacttcggcgccatcagctctgtgctgaacgatatcctgagcagactggacaaagttgaggccgaggtgcagatcgacagactgatcacaggcagactgcagagcctccagacatacgtgacccagcagctgatcagagccgccgagattagagcctctgccaatctggccgccaccaagatgtctgagtgtgtgctgggccagagcaagagagtggacttttgcggcaagggctaccacctgatgagcttccctcagtctgcccctcacggcgtggtgtttctgcacgtgacatatgtgcccgctcaagagaagaatttcaccaccgctccagccatctgccacgacggcaaagcccactttcctagagaaggcgtgttcgtgtccaacggcacccattggttcgtgacacagcggaacttctacgagccccagatcatcaccaccgacaacaccttcgtgtctggcaactgcgacgtcgtgatcggcattgtgaacaataccgtgtacgaccctctgcagcccgagctggacagcttcaaagaggaactggacaagtactttaagaaccacacaagccccgacgtggacctgggcgatatcagcggaatcaatgccagcgtcgtgaacatccagaaagagatcgaccggctgaacgaggtggccaagaatttaaatgagagcctgatcgacctgcaagaactggggaagtacgagcaaggcggcggaggaacaggcggaggctatattcctgaggctcccagagatggccaggcctacgttagaaaggatggcgagtgggtgctgctgtccacctttctgggaagatctctggaagtgctgtttcaaggccctggccaccaccatcatcaccatcaccacagcgcttggagccatcctcagttcgagaaaggcggtggaagcggaggcggaggttctggcggatctgcttggtcacacccacagtttgagaagtgatga

SEQ ID NO: 60 - DNA, 3897 bp, synthetic construct
  source 1..3897: mol_type = other DNA
atggattggacctggcggttcctgtttgtggtggctgctgctacaggcgtgcagagcgtgaacctgaccaccagaacacagctgcctccagcctacaccaacagcttcaccagaggcgtgtactaccccgacaaggtgttcagatccagcgtgctgcactctacccaggacctgttcctgcctttcttcagcaacgtgacctggttccacgccatccacgtgtccggcaccaatggcaccaagagattcgacaaccccgtgctgcccttcaacgacggggtgtactttgccagcaccgagaagtccaacatcatcagaggctggatcttcggcaccacactggacagcaagacccagagcctgctgatcgtgaacaacgccaccaacgtggtcatcaaagtgtgcgagttccagttctgcaacgaccccttcctgggcgtctactaccacaagaacaacaagagctggatggaaagcgagttccgggtgtacagcagcgccaacaactgcaccttcgagtacgtgtcccagcctttcctgatggacctggaaggcaagcagggcaacttcaagaacctgcgcgagttcgtgttcaagaacatcgacggctacttcaagatctacagcaagcacacccctatcaacctcgtgcgggatctgcctcagggcttctctgctctggaacccctggtggatctgcccatcggcatcaacatcacccggtttcagacactgctggccctgcacagaagctacctgacacctggcgatagcagctctggatggacagctggcgccgctgcctactatgtgggatacctgcagcctcggaccttcctgctgaagtacaacgagaacggcaccatcaccgacgccgtggattgtgctctggatcctctgagcgagacaaagtgcaccctgaagtccttcaccgtggaaaagggcatctaccagaccagcaacttccgggtgcagcccaccgaatccatcgtgcggttccccaatatcaccaatctgtgccccttcggcgaggtgttcaatgccaccagattcgcctctgtgtacgcctggaaccggaagcggatcagcaattgcgtggccgactactccgtgctgtacaactccgccagcttcagcaccttcaagtgctacggcgtgtcccctaccaagctgaacgacctgtgcttcacaaacgtgtacgccgacagcttcgtgatccggggagatgaagtgcggcagattgcccctggacagacaggcaagatcgcctactacaactacaagctgcccgacgacttcaccggctgtgtgattgcctggaacagcaacaacctggactccaaagtcggcggcaactacaattacctgtaccggctgttccggaagtccaatctgaagcccttcgagcgggacatctccaccgagatctatcaggccggcagcaccccttgtaacggcgtggaaggcttcaactgctacttcccactgcagtcctacggctttcagcccacaaatggcgtgggctaccagccttacagagtggtggtgctgagcttcgagctgctgcatgctcctgccacagtgtgcggccctaagaaaagcaccaatctcgtgaagaacaaatgcgtgaacttcaacttcaacggcctgaccggaaccggcgtgctgacagagagcaacaagaagttcctgccattccagcagttcggccgggatatcgccgataccacagatgccgtcagagatccccagacactggaaatcctggacatcaccccttgcagcttcggcggagtgtctgtgatcacccctggcaccaacaccagcaatcaggtggcagtgctgtaccaggacgtgaactgtaccgaagtgcccgtggccattcacgccgatcagctgacacctacatggcgggtgtactccaccggcagcaatgtgtttcagaccagagccggctgtctgatcggagccgagcacgtgaacaatagctacgagtgcgacatccccatcggcgctggcatctgcgcctcttaccagacacagacaaacagccctggcagcgcctcttctgtggccagccagagcatcattgcctacacaatgtctctgggcgccgagaacagcgtggcctactccaacaactctatcgctatccccaccaacttcaccatcagcgtgaccacagagatcctgcctgtgtccatgaccaagaccagcgtggactgcaccatgtacatctgcggcgattccaccgagtgctccaacctgctgctgcagtacggcagcttctgcacccagctgaatagagccctgaccgggatcgccgtggaacaggacaagaacacccaagaggtgttcgcccaagtgaagcagatctacaagacccctcctatcaaggacttcggcggcttcaatttcagccagattctgcccgatcctagcaagcccagcaagcggagcttcatcgaggacctgctgttcaacaaagtgacactggccgacgccggcttcatcaagcagtatggcgattgtctgggcgacattgccgccagggatctgatttgcgcccagaagtttaacggactgacagtgctgcctcctctgctgaccgatgagatgatcgcccagtacacatctgccctgctggccggcacaatcacaagcggctggacatttggagctggcgctgccctgcagatcccctttgctatgcagatggcctaccggttcaacggcatcggagtgacccagaatgtgctgtacgagaaccagaagctgatcgccaaccagttcaacagcgccatcggcaagatccaggacagcctgagcagcacagcaagcgccctgggaaagctgcaggacgtggtcaaccagaatgcccaggcactgaacaccctggtcaagcagctgtctagcaacttcggcgccatcagctctgtgctgaacgatatcctgagcagactggacaaagttgaggccgaggtgcagatcgacagactgatcacaggcagactgcagagcctccagacatacgtgacccagcagctgatcagagccgccgagattagagcctctgccaatctggccgccaccaagatgtctgagtgtgtgctgggccagagcaagagagtggacttttgcggcaagggctaccacctgatgagcttccctcagtctgcccctcacggcgtggtgtttctgcacgtgacatatgtgcccgctcaagagaagaatttcaccaccgctccagccatctgccacgacggcaaagcccactttcctagagaaggcgtgttcgtgtccaacggcacccattggttcgtgacacagcggaacttctacgagccccagatcatcaccaccgacaacaccttcgtgtctggcaactgcgacgtcgtgatcggcattgtgaacaataccgtgtacgaccctctgcagcccgagctggacagcttcaaagaggaactggacaagtactttaagaaccacacaagccccgacgtggacctgggcgatatcagcggaatcaatgccagcgtcgtgaacatccagaaagagatcgaccggctgaacgaggtggccaagaatttaaatgagagcctgatcgacctgcaagaactggggaagtacgagcaaggcggcggaggaacaggcggaggctatattcctgaggctcccagagatggccaggcctacgttagaaaggatggcgagtgggtgctgctgtccacctttctgggaagatctctggaagtgctgtttcaaggccctggccaccaccatcatcaccatcaccacagcgcttggagccatcctcagttcgagaaaggcggtggaagcggaggcggaggttctggcggatctgcttggtcacacccacagtttgagaagtgatga

SEQ ID NO: 61 - DNA, 3897 bp, synthetic construct
  source 1..3897: mol_type = other DNA
atggattggacctggcggttcctgtttgtggtggctgctgctacaggcgtgcagagcgtgaacctgaccaccagaacacagctgcctccagcctacaccaacagcttcaccagaggcgtgtactaccccgacaaggtgttcagatccagcgtgctgcactctacccaggacctgttcctgcctttcttcagcaacgtgacctggttccacgccatccacgtgtccggcaccaatggcaccaagagattcgacaaccccgtgctgcccttcaacgacggggtgtactttgccagcaccgagaagtccaacatcatcagaggctggatcttcggcaccacactggacagcaagacccagagcctgctgatcgtgaacaacgccaccaacgtggtcatcaaagtgtgcgagttccagttctgcaacgaccccttcctgggcgtctactaccacaagaacaacaagagctggatggaaagcgagttccgggtgtacagcagcgccaacaactgcaccttcgagtacgtgtcccagcctttcctgatggacctggaaggcaagcagggcaacttcaagaacctgcgcgagttcgtgttcaagaacatcgacggctacttcaagatctacagcaagcacacccctatcaacctcgtgcgggatctgcctcagggcttctctgctctggaacccctggtggatctgcccatcggcatcaacatcacccggtttcagacactgctggccctgcacagaagctacctgacacctggcgatagcagctctggatggacagctggcgccgctgcctactatgtgggatacctgcagcctcggaccttcctgctgaagtacaacgagaacggcaccatcaccgacgccgtggattgtgctctggatcctctgagcgagacaaagtgcaccctgaagtccttcaccgtggaaaagggcatctaccagaccagcaacttccgggtgcagcccaccgaatccatcgtgcggttccccaatatcaccaatctgtgccccttcggcgaggtgttcaatgccaccagattcgcctctgtgtacgcctggaaccggaagcggatcagcaattgcgtggccgactactccgtgctgtacaactcctggagcttcagcaccttcaagtgctacggcgtgtcccctaccaagctgaacgacctgtgcttcacaaacgtgtacgccgacagcttcgtgatccggggagatgaagtgcggcagattgcccctggacagacaggcaagatcgccagatacaactacaagctgcccgacgacttcaccggctgtgtgattgcctggaacagcaacaacctggactccaaagtcggcggcaactacaattacctgtaccggctgttccggaagtccaatctgaagcccttcgagcgggacatctccaccgagatctatcaggccggcagcaccccttgtaacggcgtggaaggcttcaactgctacttcccactgcagtcctacggctttcagcccacaaatggcgtgggctaccagccttacagagtggtggtgctgagcttcgagctgctgcatgctcctgccacagtgtgcggccctaagaaaagcaccaatctcgtgaagaacaaatgcgtgaacttcaacttcaacggcctgaccggaaccggcgtgctgacagagagcaacaagaagttcctgccattccagcagttcggccgggatatcgccgataccacagatgccgtcagagatccccagacactggaaatcctggacatcaccccttgcagcttcggcggagtgtctgtgatcacccctggcaccaacaccagcaatcaggtggcagtgctgtaccaggacgtgaactgtaccgaagtgcccgtggccattcacgccgatcagctgacacctacatggcgggtgtactccaccggcagcaatgtgtttcagaccagagccggctgtctgatcggagccgagcacgtgaacaatagctacgagtgcgacatccccatcggcgctggcatctgcgcctcttaccagacacagacaaacagccctggcagcgcctcttctgtggccagccagagcatcattgcctacacaatgtctctgggcgccgagaacagcgtggcctactccaacaactctatcgctatccccaccaacttcaccatcagcgtgaccacagagatcctgcctgtgtccatgaccaagaccagcgtggactgcaccatgtacatctgcggcgattccaccgagtgctccaacctgctgctgcagtacggcagcttctgcacccagctgaatagagccctgaccgggatcgccgtggaacaggacaagaacacccaagaggtgttcgcccaagtgaagcagatctacaagacccctcctatcaaggacttcggcggcttcaatttcagccagattctgcccgatcctagcaagcccagcaagcggagcttcatcgaggacctgctgttcaacaaagtgacactggccgacgccggcttcatcaagcagtatggcgattgtctgggcgacattgccgccagggatctgatttgcgcccagaagtttaacggactgacagtgctgcctcctctgctgaccgatgagatgatcgcccagtacacatctgccctgctggccggcacaatcacaagcggctggacatttggagctggcgctgccctgcagatcccctttgctatgcagatggcctaccggttcaacggcatcggagtgacccagaatgtgctgtacgagaaccagaagctgatcgccaaccagttcaacagcgccatcggcaagatccaggacagcctgagcagcacagcaagcgccctgggaaagctgcaggacgtggtcaaccagaatgcccaggcactgaacaccctggtcaagcagctgtctagcaacttcggcgccatcagctctgtgctgaacgatatcctgagcagactggacaaagttgaggccgaggtgcagatcgacagactgatcacaggcagactgcagagcctccagacatacgtgacccagcagctgatcagagccgccgagattagagcctctgccaatctggccgccaccaagatgtctgagtgtgtgctgggccagagcaagagagtggacttttgcggcaagggctaccacctgatgagcttccctcagtctgcccctcacggcgtggtgtttctgcacgtgacatatgtgcccgctcaagagaagaatttcaccaccgctccagccatctgccacgacggcaaagcccactttcctagagaaggcgtgttcgtgtccaacggcacccattggttcgtgacacagcggaacttctacgagccccagatcatcaccaccgacaacaccttcgtgtctggcaactgcgacgtcgtgatcggcattgtgaacaataccgtgtacgaccctctgcagcccgagctggacagcttcaaagaggaactggacaagtactttaagaaccacacaagccccgacgtggacctgggcgatatcagcggaatcaatgccagcgtcgtgaacatccagaaagagatcgaccggctgaacgaggtggccaagaatttaaatgagagcctgatcgacctgcaagaactggggaagtacgagcaaggcggcggaggaacaggcggaggctatattcctgaggctcccagagatggccaggcctacgttagaaaggatggcgagtgggtgctgctgtccacctttctgggaagatctctggaagtgctgtttcaaggccctggccaccaccatcatcaccatcaccacagcgcttggagccatcctcagttcgagaaaggcggtggaagcggaggcggaggttctggcggatctgcttggtcacacccacagtttgagaagtgatga

SEQ ID NO: 62 - DNA, 3897 bp, synthetic construct
  source 1..3897: mol_type = other DNA
atggattggacctggcggttcctgtttgtggtggctgctgctacaggcgtgcagagcgtgaacctgaccaccagaacacagctgcctccagcctacaccaacagcttcaccagaggcgtgtactaccccgacaaggtgttcagatccagcgtgctgcactctacccaggacctgttcctgcctttcttcagcaacgtgacctggttccacgccatccacgtgtccggcaccaatggcaccaagagattcgacaaccccgtgctgcccttcaacgacggggtgtactttgccagcaccgagaagtccaacatcatcagaggctggatcttcggcaccacactggacagcaagacccagagcctgctgatcgtgaacaacgccaccaacgtggtcatcaaagtgtgcgagttccagttctgcaacgaccccttcctgggcgtctactaccacaagaacaacaagagctggatggaaagcgagttccgggtgtacagcagcgccaacaactgcaccttcgagtacgtgtcccagcctttcctgatggacctggaaggcaagcagggcaacttcaagaacctgcgcgagttcgtgttcaagaacatctttggctacttcaagatctacagcaagcacacccctatcaacctcgtgcgggatctgcctcagggcttctctgctctggaacccctggtggatctgcccatccttatcaacatcacccggtttcagacactgctggccctgcacagaagctacctgacacctggcgatagcagctctggatggacagctggcgccgctgcctactatgtgggatacctgcagcctcggaccttcctgctgaagtacaacgagaacggcaccatcaccgacgccgtggattgtgctctggatcctctgagcgagacaaagtgcaccctgaagtccttcaccgtggaaaagggcatctaccagaccagcaacttccgggtgcagcccaccgaatccatcgtgcggttccccaatatcaccaatctgtgccccttcggcgaggtgttcaatgccaccagattcgcctctgtgtacgcctggaaccggaagcggatcagcaattgcgtggccgactactccgtgctgtacaactcctggagcttcagcaccttcaagtgctacggcgtgtcccctaccaagctgaacgacctgtgcttcacacaggtgtacgccgacagcttcgtgatccggggagatgaagtgcggcagattgcccctggacagacaggcaagatcgccagatacaactacaagctgcccgacgacttcaccggctgtgtgattgcctggaacagcaacaacctggactccaaagtcggcggcaactacaattacctgtaccggctgttccggaagtccaatctgaagcccttcgagcgggacatctccaccgagatctatcaggccggcagcaccccttgtaacggcgtggaaggcttcaactgctacttcccactgcagtcctacggctttcagcccacaaatggcgtgggctaccagccttacagagtggtggtgctgagcttcgagctgctgcatgctcctgccacagtgtgcggccctaagaaaagcaccaatctcgtgaagaacaaatgcgtgaacttcaacttcaacggcctgaccggaaccggcgtgctgacagagagcaacaagaagttcctgccattccagcagttcggccgggatatcgccgataccacagatgccgtcagagatccccagacactggaaatcctggacatcaccccttgcagcttcggcggagtgtctgtgatcacccctggcaccaacaccagcaatcaggtggcagtgctgtaccaggacgtgaactgtaccgaagtgcccgtggccattcacgccgatcagctgacacctacatggcgggtgtactccaccggcagcaatgtgtttcagaccagagccggctgtctgatcggagccgagcacgtgaacaatagctacgagtgcgacatccccatcggcgctggcatctgcgcctcttaccagacacagacaaacagccctggcagcgcctcttctgtggccagccagagcatcattgcctacacaatgtctctgggcgccgagaacagcgtggcctactccaacaactctatcgctatccccaccaacttcaccatcagcgtgaccacagagatcctgcctgtgtccatgaccaagaccagcgtggactgcaccatgtacatctgcggcgattccaccgagtgctccaacctgctgctgcagtacggcagcttctgcacccagctgaatagagccctgaccgggatcgccgtggaacaggacaagaacacccaagaggtgttcgcccaagtgaagcagatctacaagacccctcctatcaaggacttcggcggcttcaatttcagccagattctgcccgatcctagcaagcccagcaagcggagcttcatcgaggacctgctgttcaacaaagtgacactggccgacgccggcttcatcaagcagtatggcgattgtctgggcgacattgccgccagggatctgatttgcgcccagaagtttaacggactgacagtgctgcctcctctgctgaccgatgagatgatcgcccagtacacatctgccctgctggccggcacaatcacaagcggctggacatttggagctggcgctgccctgcagatcccctttgctatgcagatggcctaccggttcaacggcatcggagtgacccagaatgtgctgtacgagaaccagaagctgatcgccaaccagttcaacagcgccatcggcaagatccaggacagcctgagcagcacagcaagcgccctgggaaagctgcaggacgtggtcaaccagaatgcccaggcactgaacaccctggtcaagcagctgtctagcaacttcggcgccatcagctctgtgctgaacgatatcctgagcagactggacaaagttgaggccgaggtgcagatcgacagactgatcacaggcagactgcagagcctccagacatacgtgacccagcagctgatcagagccgccgagattagagcctctgccaatctggccgccaccaagatgtctgagtgtgtgctgggccagagcaagagagtggacttttgcggcaagggctaccacctgatgagcttccctcagtctgcccctcacggcgtggtgtttctgcacgtgacatatgtgcccgctcaagagaagaatttcaccaccgctccagccatctgccacgacggcaaagcccactttcctagagaaggcgtgttcgtgtccaacggcacccattggttcgtgacacagcggaacttctacgagccccagatcatcaccaccgacaacaccttcgtgtctggcaactgcgacgtcgtgatcggcattgtgaacaataccgtgtacgaccctctgcagcccgagctggacagcttcaaagaggaactggacaagtactttaagaaccacacaagccccgacgtggacctgggcgatatcagcggaatcaatgccagcgtcgtgaacatccagaaagagatcgaccggctgaacgaggtggccaagaatttaaatgagagcctgatcgacctgcaagaactggggaagtacgagcaaggcggcggaggaacaggcggaggctatattcctgaggctcccagagatggccaggcctacgttagaaaggatggcgagtgggtgctgctgtccacctttctgggaagatctctggaagtgctgtttcaaggccctggccaccaccatcatcaccatcaccacagcgcttggagccatcctcagttcgagaaaggcggtggaagcggaggcggaggttctggcggatctgcttggtcacacccacagtttgagaagtgatga

SEQ ID NO: 63 - DNA, 3894 bp, synthetic construct
  source 1..3894: mol_type = other DNA
atggattggacctggcggttcctgtttgtggtggctgctgctacaggcgtgcagagcgtgaacctgaccaccagaacacagctgcctccagcctacaccaacagcttcaccagaggcgtgtactaccccgacaaggtgttcagatccagcgtgctgcactctacccaggacctgttcctgcctttcttcagcaacgtgacctggttccacgccatccacgtgtccggcaccaatggcaccaagagattcgacaaccccgtgctgcccttcaacgacggggtgtactttgccagcaccgagaagtccaacatcatcagaggctggatcttcggcaccacactggacagcaagacccagagcctgctgatcgtgaacaacgccaccaacgtggtcatcaaagtgtgcgagttccagttctgcaacgaccccttcctgggcgtctactaccacaagaacaacaagagctggatggaaagcgagttccgggtgtacagcagcgccaacaactgcaccttcgagtacgtgtcccagcctttcctgatggacctggaaggcaagcagggcaacttcaagaacctgcgcgagttcgtgttcaagaacatcgacggctacttcaagatctacagcaagcacacccctatcaacctcgtgcgggatctgcctcagggcttctctgctctggaacccctggtggatctgcccatcggcatcaacatcacccggtttcagacactgctggccctgcacagaagctacctgacacctggcgatagcagctctggatggacagctggcgccgctgcctactatgtgggatacctgcagcctcggaccttcctgctgaagtacaacgagaacggcaccatcaccgacgccgtggattgtgctctggatcctctgagcgagacaaagtgcaccctgaagtccttcaccgtggaaaagggcatctaccagaccagcaacttccgggtgcagcccaccgaatccatcgtgcggttccccaatatcaccaatctgtgccccttcggcgaggtgttcaatgccaccagattcgcctctgtgtacgcctggaaccggaagcggatcagcaattgcgtggccgactactccgtgctgtacaactccgccagcttcagcaccttcaagtgctacggcgtgtcccctaccaagctgaacgacctgtgcttcacaaacgtgtacgccgacagcttcgtgatccggggagatgaagtgcggcagattgcccctggacagacaggcaagatcgccgactacaactacaagctgcccgacgacttcaccggctgtgtgattgcctggaacagcaacaacctggactccaaagtcggcggcaactacaattacctgtaccggctgttccggaagtccaatctgaagcccttcgagcgggacatctccaccgagatctatcaggccggcagcaccccttgtaacggcgtggaaggcttcaactgctacttcccactgcagtcctacggctttcagcccacaaatggcgtgggctaccagccttacagagtggtggtgctgagcttcgagctgctgcatgctcctgccacagtgtgcggccctaagaaaagcaccaatctcgtgaagaacaaatgcgtgaacttcaacttcaacggcctgaccggaaccggcgtgctgacagagagcaacaagaagttcctgccattccagcagttcggccgggatatcgccgataccacagatgccgtcagagatccccagacactggaaatcctggacatcaccccttgcagcttcggcggagtgtctgtgatcacccctggcaccaacaccagcaatcaggtggcagtgctgtaccaggacgtgaactgtaccgaagtgcccgtggccattcacgccgatcagctgacacctacatggcgggtgtactccaccggcagcaatgtgtttcagaccagagccggctgtctgatcggagccgagcacgtgaacaatagctacgagtgcgacatccccatcggcgctggcatctgcgcctcttaccagacacagacaaacagccctggcagcgcctcttctgtggccagccagagcatcattgcctacacaatgtctctgggcgccgagaacagcgtgcagtactccaacaactctatcgctatccccaccaacttcaccatcagcgtgaccacagagatcctgcctgtgtccatgaccaagaccagcgtggactgcaccatgtacatctgcggcgattccaccgagtgctccaacctgctgctgcagtacggcgagttctgcacccagctgaatagagccctgaccgggatcgccgtggaacaggacaagaacacccaagaggtgttcgcccaagtgaagcagatctacaagacccctcctatcaaggacttcggcggcttcaatttcagccagattctgcccgatcctagcaagcccagcaagcggagcttcatcgaggacctgctgttcaacaaagtgacactggccgacgccggcttcatcaagcagtatggcgattgtctgggcgacattgccgccagggataagatttgcgcccagaagtttaacggactgacagtgctgcctcctctgctgaccgatgagatgatcgcccagtacacatctgccctgctggccggcacaatcacaagcggctggacatttggagctggcgctgccctgcagatcccctttgctatgcagatggcctaccggttcaacggcatcggagtgacccagaatgtgctgtacgagaaccagaagctgatcgccaaccagttcaacagcgccatcggcaagatccaggacagcctgagcagcacagcaagcgccctgggaaagctgcaggacgtggtcaaccagaatgcccaggcactgaacaccctggagaagcagctgtctagcaacttcggcgccatcagctctgtgctgaacgatatcctgagcagactggaccctcctgaggccgaggtgcagatcgacagactgatcacaggcagactgcagagcctccagacatacgtgacccagcagctgatcagagccgccgagattagagcctctgccaatctggccgccaccaagatgcgtgagtgtgtgctgggccagagcaagagagtggacttttgcggcaagggctaccacctgatgagcttccctcagtctgcccctcacggcgtggtgtttctgcacgtgacatatgtgcccgctcaagagaagaatttcaccaccgctccagccatctgccacgacggcaaagcccactttcctagagaaggcgtgttcgtgtccaacggcacccattggttcgtgacacagcggaacttctacgagccccggatcatcaccaccgacaacaccttcgtgtctggcaactgcgacgtcgtgatcggcattgtgaacaataccgtgtacgaccctctgcagcccgagctggacagcttcaaagaggaactggacaagtactttaagaaccacacaagccccgacgtggacctgggcgatatcagcggaatcaatgccagcgtcgtgaacatccagaaagagatcgaccggctgaacgaggtggccaagaatttaaatgagagcctgatcgacctgcaagaactggggaagtacgagcaaggcggcggaggaacaggcggaggctatattcctgaggctcccagagatggccaggcctacgttagaaaggatggcgagtgggtgctgctgtccacctttctgggaagatctctggaagtgctgtttcaaggccctggccaccaccatcatcaccatcaccacagcgcttggagccatcctcagttcgagaaaggcggtggaagcggaggcggaggttctggcggatctgcttggtcacacccacagtttgagaagtga

SEQ ID NO: 64 - DNA, 3894 bp, synthetic construct
  source 1..3894: mol_type = other DNA
atggattggacctggcggttcctgtttgtggtggctgctgctacaggcgtgcagagcgtgaacctgaccaccagaacacagctgcctccagcctacaccaacagcttcaccagaggcgtgtactaccccgacaaggtgttcagatccagcgtgctgcactctacccaggacctgttcctgcctttcttcagcaacgtgacctggttccacgccatccacgtgtccggcaccaatggcaccaagagattcgacaaccccgtgctgcccttcaacgacggggtgtactttgccagcaccgagaagtccaacatcatcagaggctggatcttcggcaccacactggacagcaagacccagagcctgctgatcgtgaacaacgccaccaacgtggtcatcaaagtgtgcgagttccagttctgcaacgaccccttcctgggcgtctactaccacaagaacaacaagagctggatggaaagcgagttccgggtgtacagcagcgccaacaactgcaccttcgagtacgtgtcccagcctttcctgatggacctggaaggcaagcagggcaacttcaagaacctgcgcgagttcgtgttcaagaacatcgacggctacttcaagatctacagcaagcacacccctatcaacctcgtgcgggatctgcctcagggcttctctgctctggaacccctggtggatctgcccatcggcatcaacatcacccggtttcagacactgctggccctgcacagaagctacctgacacctggcgatagcagctctggatggacagctggcgccgctgcctactatgtgggatacctgcagcctcggaccttcctgctgaagtacaacgagaacggcaccatcaccgacgccgtggattgtgctctggatcctctgagcgagacaaagtgcaccctgaagtccttcaccgtggaaaagggcatctaccagaccagcaacttccgggtgcagcccaccgaatccatcgtgcggttccccaatatcaccaatctgtgccccttcggcgaggtgttcaatgccaccagattcgcctctgtgtacgcctggaaccggaagcggatcagcaattgcgtggccgactactccgtgctgtacaactccgccagcttcagcaccttcaagtgctacggcgtgtcccctaccaagctgaacgacctgtgcttcacaaacgtgtacgccgacagcttcgtgatccggggagatgaagtgcggcagattgcccctggacagacaggcaagatcgccgactacaactacaagctgcccgacgacttcaccggctgtgtgattgcctggaacagcaacaacctggactccaaagtcggcggcaactacaattacctgtaccggctgttccggaagtccaatctgaagcccttcgagcgggacatctccaccgagatctatcaggccggcagcaccccttgtaacggcgtggaaggcttcaactgctacttcccactgcagtcctacggctttcagcccacaaatggcgtgggctaccagccttacagagtggtggtgctgagcttcgagctgctgcatgctcctgccacagtgtgcggccctaagaaaagcaccaatctcgtgaagaacaaatgcgtgaacttcaacttcaacggcctgaccggaaccggcgtgctgacagagagcaacaagaagttcctgccattccagcagttcggccgggatatcgccgataccacagatgccgtcagagatccccagacactggaaatcctggacatcaccccttgcagcttcggcggagtgtctgtgatcacccctggcaccaacaccagcaatcaggtggcagtgctgtaccaggacgtgaactgtaccgaagtgcccgtggccattcacgccgatcagctgacacctacatggcgggtgtactccaccggcagcaatgtgtttcagaccagagccggctgtctgatcggagccgagcacgtgaacaatagctacgagtgcgacatccccatcggcgctggcatctgcgcctcttaccagacacagacaaacagccctggcagcgcctcttctgtggccagccagagcatcattgcctacacaatgtctctgggcgccgagaacagcgtggcctactccaacaactctatcgctatccccaccaacttcaccatcagcgtgaccacagagatcctgcctgtgtccatgaccaagaccagcgtggactgcaccatgtacatctgcggcgattccaccgagtgctccaacctgctgctgaagtacggcagcttctgcacccagctgaatagagccctgaccgggatcgccgtggaacaggacaagaacacccaagaggtgttcgcccaagtgaagcagatctacaagacccctcctatcaaggacttcggcggcttcaatttcagccagattctgcccgatcctagcaagcccagcaagcggagcttcatcgaggacctgctgttcaacaaagtgacactggccgacgccggcttcatcaagcagtatggcgattgtctgggcgacattgccgccagggataagatttgcgcccagaagtttaacggactgacagtgctgcctcctctgctgaccgatgagatgatcgcccagtacacatctgccctgctggccggcacaatcacaagcggctggacatttggagctggcaatgccctgcagatcccctttgctatgcagatggcctaccggttcaacggcatcggagtgacccagaatgtgctgtacgagaaccagaagctgatcgccaaccagttcaacagcgccatcggcaagatccaggacagcctgagcagcacagcaagcgccctgggaaggctgcaggacgtggtcaaccagaatgcccaggcactgaacaccctggtcaagcagctgtctagcaacttcggcgccatcagctctgtgctgaacgatatcctgagcagactggaccctcctgaggccgaggtgcagatcgacagactgatcacaggcagactgcagagcctccagacatacgtgacccagcagctgatcagagccgccgagattagagcctctgccaatctggccgccaccaagatgtctgagtgtgtgctgggccagagcaagagagtggacttttgcggcaggggctaccacctgatgagcttccctcagtctgcccctcacggcgtggtgtttctgcacgtgacatatgtgcccgctcaagagaagaatttcaccaccgctccagccatctgccacgacggcaaagcccactttcctagagaaggcgtgttcgtgtccaacggcacccattggttcgtgacacagcggaacttctacgagccccagatcatcaccaccgacaacaccttcgtgtctggcaactgcgacgtcgtgatcggcattgtgaacaataccgtgtacgaccctctgcagcccgagctggacagcttcaaagaggaactggacaagtactttaagaaccacacaagccccgacgtggacctgggcgatatcagcggaatcaatgccagcgtcgtgaacatccagaaagagatcgaccggctgaacgaggtggccaagaatttaaatgagagcctgatcgacctgcaagaactggggaagtacgagcaaggcggcggaggaacaggcggaggctatattcctgaggctcccagagatggccaggcctacgttagaaaggatggcgagtgggtgctgctgtccacctttctgggaagatctctggaagtgctgtttcaaggccctggccaccaccatcatcaccatcaccacagcgcttggagccatcctcagttcgagaaaggcggtggaagcggaggcggaggttctggcggatctgcttggtcacacccacagtttgagaagtga

SEQ ID NO: 65 - DNA, 3894 bp, synthetic construct
  source 1..3894: mol_type = other DNA
atggattggacctggcggttcctgtttgtggtggctgctgctacaggcgtgcagagcgtgaacctgaccaccagaacacagctgcctccagcctacaccaacagcttcaccagaggcgtgtactaccccgacaaggtgttcagatccagcgtgctgcactctacccaggacctgttcctgcctttcttcagcaacgtgacctggttccacgccatccacgtgtccggcaccaatggcaccaagagattcgacaaccccgtgctgcccttcaacgacggggtgtactttgccagcaccgagaagtccaacatcatcagaggctggatcttcggcaccacactggacagcaagacccagagcctgctgatcgtgaacaacgccaccaacgtggtcatcaaagtgtgcgagttccagttctgcaacgaccccttcctgggcgtctactaccacaagaacaacaagagctggatggaaagcgagttccgggtgtacagcagcgccaacaactgcaccttcgagtacgtgtcccagcctttcctgatggacctggaaggcaagcagggcaacttcaagaacctgcgcgagttcgtgttcaagaacatcgacggctacttcaagatctacagcaagcacacccctatcaacctcgtgcgggatctgcctcagggcttctctgctctggaacccctggtggatctgcccatcggcatcaacatcacccggtttcagacactgctggccctgcacagaagctacctgacacctggcgatagcagctctggatggacagctggcgccgctgcctactatgtgggatacctgcagcctcggaccttcctgctgaagtacaacgagaacggcaccatcaccgacgccgtggattgtgctctggatcctctgagcgagacaaagtgcaccctgaagtccttcaccgtggaaaagggcatctaccagaccagcaacttccgggtgcagcccaccgaatccatcgtgcggttccccaatatcaccaatctgtgccccttcggcgaggtgttcaatgccaccagattcgcctctgtgtacgcctggaaccggaagcggatcagcaattgcgtggccgactactccgtgctgtacaactccgccagcttcagcaccttcaagtgctacggcgtgtcccctaccaagctgaacgacctgtgcttcacaaacgtgtacgccgacagcttcgtgatccggggagatgaagtgcggcagattgcccctggacagacaggcaagatcgccgactacaactacaagctgcccgacgacttcaccggctgtgtgattgcctggaacagcaacaacctggactccaaagtcggcggcaactacaattacctgtaccggctgttccggaagtccaatctgaagcccttcgagcgggacatctccaccgagatctatcaggccggcagcaccccttgtaacggcgtggaaggcttcaactgctacttcccactgcagtcctacggctttcagcccacaaatggcgtgggctaccagccttacagagtggtggtgctgagcttcgagctgctgcatgctcctgccacagtgtgcggccctaagaaaagcaccaatctcgtgaagaacaaatgcgtgaacttcaacttcaacggcctgaccggaaccggcgtgctgacagagagcaacaagaagttcctgccattccagcagttcggccgggatatcgccgataccacagatgccgtcagagatccccagacactggaaatcctggacatcaccccttgcagcttcggcggagtgtctgtgatcacccctggcaccaacaccagcaatcaggtggcagtgctgtaccaggacgtgaactgtaccgaagtgcccgtggccattcacgccgatcagctgacacctacatggcgggtgtactccaccggcagcaatgtgtttcagaccagagccggctgtctgatcggagccgagcacgtgaacaatagctacgagtgcgacatccccatcggcgctggcatctgcgcctcttaccagacacagacaaacagccctggcagcgcctcttctgtggccagccagagcatcattgcctacacaatgtctctgggcgccgagaacagcgtggcctactccaacaactctatcgctatccccaccaacttcaccatcagcgtgaccacagagatcctgcctgtgtccatgaccaagaccagcgtggactgcaccatgtacatctgcggcgattccaccgagtgctccaacctgctgctgcagtacggcgaattctgcacccagctgaatagagccctgaccgggatcgccgtggaacaggacaagaacacccaagaggtgttcgcccaagtgaagcagatctacaagacccctcctatcaaggacttcggcggcttcaatttcagccagattctgcccgatcctagcaagcccagcaagcggagcttcatcgaggacctgctgttcaacaaagtgacactggccgacgccggcttcatcaagcagtatggcgattgtctgggcgacattgccgccagggataagatttgcgcccagaagtttaacggactgacagtgctgcctcctctgctgaccgatgagatgatcgcccagtacacatctgccctgctggccggcacaatcacaagcggctggacatttggagctggcgctgccctgcagatcccctttgctatgcagatggcctaccggttcaacggcatcggagtgacccagaatgtgctgtacgagaaccagaagctgatcgccaaccagttcaacagcgccatcggcaagatccaggacagcctgagcagcacagcaagcgccctgggaaagctgcaggacgtggtcaaccagaatgcccaggcactgaacaccctggagaagcagctgtctagcaacttcggcgccatcagctctgtgctgaacgatatcctgagcagactggaccctcctgaggccgaggtgcagatcgacagactgatcacaggcagactgcagagcctccagacatacgtgacccagcagctgatcagagccgccgagattagagcctctgccaatctggccgccaccaagatgtctgagtgtgtgctgggccagagcaagagagtggacttttgcggcaagggctaccacctgatgagcttccctcagtctgcccctcacggcgtggtgtttctgcacgtgacatatgtgcccgctcaagagaagaatttcaccaccgctccagccatctgccacgacggcaaagcccactttcctagagaaggcgtgttcgtgtccaacggcacccattggttcgtgacacagcggaacttctacgagccccagatcatcaccaccgacaacaccttcgtgtctggcaactgcgacgtcgtgatcggcattgtgaacaataccgtgtacgaccctctgcagcccgagctggacagcttcaaagaggaactggacaagtactttaagaaccacacaagccccgacgtggacctgggcgatatcagcggaatcaatgccagcgtcgtgaacatccagaaagagatcgaccggctgaacgaggtggccaagaatttaaatgagagcctgatcgacctgcaagaactggggaagtacgagcaaggcggcggaggaacaggcggaggctatattcctgaggctcccagagatggccaggcctacgttagaaaggatggcgagtgggtgctgctgtccacctttctgggaagatctctggaagtgctgtttcaaggccctggccaccaccatcatcaccatcaccacagcgcttggagccatcctcagttcgagaaaggcggtggaagcggaggcggaggttctggcggatctgcttggtcacacccacagtttgagaagtga

SEQ ID NO: 66 - DNA, 3894 bp, synthetic construct
  source 1..3894: mol_type = other DNA
atggattggacctggcggttcctgtttgtggtggctgctgctacaggcgtgcagagcgtgaacctgaccaccagaacacagctgcctccagcctacaccaacagcttcaccagaggcgtgtactaccccgacaaggtgttcagatccagcgtgctgcactctacccaggacctgttcctgcctttcttcagcaacgtgacctggttccacgccatccacgtgtccggcaccaatggcaccaagagattcgacaaccccgtgctgcccttcaacgacggggtgtactttgccagcaccgagaagtccaacatcatcagaggctggatcttcggcaccacactggacagcaagacccagagcctgctgatcgtgaacaacgccaccaacgtggtcatcaaagtgtgcgagttccagttctgcaacgaccccttcctgggcgtctactaccacaagaacaacaagagctggatggaaagcgagttccgggtgtacagcagcgccaacaactgcaccttcgagtacgtgtcccagcctttcctgatggacctggaaggcaagcagggcaacttcaagaacctgcgcgagttcgtgttcaagaacatcgacggctacttcaagatctacagcaagcacacccctatcaacctcgtgcgggatctgcctcagggcttctctgctctggaacccctggtggatctgcccatcggcatcaacatcacccggtttcagacactgctggccctgcacagaagctacctgacacctggcgatagcagctctggatggacagctggcgccgctgcctactatgtgggatacctgcagcctcggaccttcctgctgaagtacaacgagaacggcaccatcaccgacgccgtggattgtgctctggatcctctgagcgagacaaagtgcaccctgaagtccttcaccgtggaaaagggcatctaccagaccagcaacttccgggtgcagcccaccgaatccatcgtgcggttccccaatatcaccaatctgtgccccttcggcgaggtgttcaatgccaccagattcgcctctgtgtacgcctggaaccggaagcggatcagcaattgcgtggccgactactccgtgctgtacaactccgccagcttcagcaccttcaagtgctacggcgtgtcccctaccaagctgaacgacctgtgcttcacaaacgtgtacgccgacagcttcgtgatccggggagatgaagtgcggcagattgcccctggacagacaggcaagatcgccgactacaactacaagctgcccgacgacttcaccggctgtgtgattgcctggaacagcaacaacctggactccaaagtcggcggcaactacaattacctgtaccggctgttccggaagtccaatctgaagcccttcgagcgggacatctccaccgagatctatcaggccggcagcaccccttgtaacggcgtggaaggcttcaactgctacttcccactgcagtcctacggctttcagcccacaaatggcgtgggctaccagccttacagagtggtggtgctgagcttcgagctgctgcatgctcctgccacagtgtgcggccctaagaaaagcaccaatctcgtgaagaacaaatgcgtgaacttcaacttcaacggcctgaccggaaccggcgtgctgacagagagcaacaagaagttcctgccattccagcagttcggccgggatatcgccgataccacagatgccgtcagagatccccagacactggaaatcctggacatcaccccttgcagcttcggcggagtgtctgtgatcacccctggcaccaacaccagcaatcaggtggcagtgctgtaccaggacgtgaactgtaccgaagtgcccgtggccattcacgccgatcagctgacacctacatggcgggtgtactccaccggcagcaatgtgtttcagaccagagccggctgtctgatcggagccgagcacgtgaacaatagctacgagtgcgacatccccatcggcgctggcatctgcgcctcttaccagacacagacaaacagccctggcagcgcctcttctgtggccagccagagcatcattgcctacacaatgtctctgggcgccgagaacagcgtggcctactccaacaactctatcgctatccccaccaacttcaccatcagcgtgaccacagagatcctgcctgtgtccatgaccaagaccagcgtggactgcaccatgtacatctgcggcgattccaccgagtgctccaacctgctgctgaagtacggcagcttctgcacccagctgaatagagccctgaccgggatcgccgtggaacaggacaagaacacccaagaggtgttcgcccaagtgaagcagatctacaagacccctcctatcaaggacttcggcggcttcaatttcagccagattctgcccgatcctagcaagcccagcaagcggagcttcatcgaggacctgctgttcaacaaagtgacactggccgacgccggcttcatcaagcagtatggcgattgtctgggcgacattgccgccagggatctgattcaggcccagaagtttaacggactgacagtgctgcctcctctgctgaccgatgagatgatcgcccagtacacatctgccctgctggccggcacaatcacaagcggctggacatttggagctggcgctgccctgcagatcccctttgctatgcagatggcctaccggttcaacggcatcggagtgacccagaatgtgctgtacgagaaccagaagctgatcgccaaccagttcaacagcgccatcggcaagatccaggacagcctgagcagcacagcaagcgccctgggaaagctgcaggacgtggtcaaccagaatgcccaggcactgaacgagctggtcaagcagctgtctagcaacttcggcgccatcagctctgtgctgaacgatatcctgagcagactggaccctcctgaggccgaggtgcagatcgacagactgatcacaggcagactgcagagcctccagacatacgtgacccagcagctgatcagagccgccgagattagagcctctgccaatctggccgccaccaagatgtctgagtgtgtgctgggccagagcaagagagtggacttttgcggcaagggctaccacctgatgagcttccctcagtctgcccctcacggcgtggtgtttctgcacgtgacatatgtgcccgctcaagagaagaatttcaccaccgctccagccatctgccacgacggcaaagcccactttcctagagaaggcgtgttcgtgtccaacggcacccattggttcgtgacacagcggaacttctacgagccccagatcatcaccaccgacaacaccttcgtgtctggcaactgcgacgtcgtgatcggcattgtgaacaataccgtgtacgaccctctgcagcccgagctggacagcttcaaagaggaactggacaagtactttaagaaccacacaagccccgacgtggacctgggcgatatcagcggaatcaatgccagcgtcgtgaacatccagaaagagatcgaccggctgaacgaggtggccaagaatttaaatgagagcctgatcgacctgcaagaactggggaagtacgagcaaggcggcggaggaacaggcggaggctatattcctgaggctcccagagatggccaggcctacgttagaaaggatggcgagtgggtgctgctgtccacctttctgggaagatctctggaagtgctgtttcaaggccctggccaccaccatcatcaccatcaccacagcgcttggagccatcctcagttcgagaaaggcggtggaagcggaggcggaggttctggcggatctgcttggtcacacccacagtttgagaagtga

SEQ ID NO: 67 - DNA, 3894 bp, synthetic construct
  source 1..3894: mol_type = other DNA
atggattggacctggcggttcctgtttgtggtggctgctgctacaggcgtgcagagcgtgaacctgaccaccagaacacagctgcctccagcctacaccaacagcttcaccagaggcgtgtactaccccgacaaggtgttcagatccagcgtgctgcactctacccaggacctgttcctgcctttcttcagcaacgtgacctggttccacgccatccacgtgtccggcaccaatggcaccaagagattcgacaaccccgtgctgcccttcaacgacggggtgtactttgccagcaccgagaagtccaacatcatcagaggctggatcttcggcaccacactggacagcaagacccagagcctgctgatcgtgaacaacgccaccaacgtggtcatcaaagtgtgcgagttccagttctgcaacgaccccttcctgggcgtctactaccacaagaacaacaagagctggatggaaagcgagttccgggtgtacagcagcgccaacaactgcaccttcgagtacgtgtcccagcctttcctgatggacctggaaggcaagcagggcaacttcaagaacctgcgcgagttcgtgttcaagaacatcgacggctacttcaagatctacagcaagcacacccctatcaacctcgtgcgggatctgcctcagggcttctctgctctggaacccctggtggatctgcccatcggcatcaacatcacccggtttcagacactgctggccctgcacagaagctacctgacacctggcgatagcagctctggatggacagctggcgccgctgcctactatgtgggatacctgcagcctcggaccttcctgctgaagtacaacgagaacggcaccatcaccgacgccgtggattgtgctctggatcctctgagcgagacaaagtgcaccctgaagtccttcaccgtggaaaagggcatctaccagaccagcaacttccgggtgcagcccaccgaatccatcgtgcggttccccaatatcaccaatctgtgccccttcggcgaggtgttcaatgccaccagattcgcctctgtgtacgcctggaaccggaagcggatcagcaattgcgtggccgactactccgtgctgtacaactccgccagcttcagcaccttcaagtgctacggcgtgtcccctaccaagctgaacgacctgtgcttcacaaacgtgtacgccgacagcttcgtgatccggggagatgaagtgcggcagattgcccctggacagacaggcaagatcgccgactacaactacaagctgcccgacgacttcaccggctgtgtgattgcctggaacagcaacaacctggactccaaagtcggcggcaactacaattacctgtaccggctgttccggaagtccaatctgaagcccttcgagcgggacatctccaccgagatctatcaggccggcagcaccccttgtaacggcgtggaaggcttcaactgctacttcccactgcagtcctacggctttcagcccacaaatggcgtgggctaccagccttacagagtggtggtgctgagcttcgagctgctgcatgctcctgccacagtgtgcggccctaagaaaagcaccaatctcgtgaagaacaaatgcgtgaacttcaacttcaacggcctgaccggaaccggcgtgctgacagagagcaacaagaagttcctgccattccagcagttcggccgggatatcgccgataccacagatgccgtcagagatccccagacactggaaatcctggacatcaccccttgcagcttcggcggagtgtctgtgatcacccctggcaccaacaccagcaatcaggtggcagtgctgtaccaggacgtgaactgtaccgaagtgcccgtggccattcacgccgatcagctgacacctacatggcgggtgtactccaccggcagcaatgtgtttcagaccagagccggctgtctgatcggagccgagcacgtgaacaatagctacgagtgcgacatccccatcggcgctggcatctgcgcctcttaccagacacagacaaacagccctggcagcgcctcttctgtggccagccagagcatcattgcctacacaatgtctctgggcgccgagaacagcgtgcaatactccaacaactctatcgctatccccaccaacttcaccatcagcgtgaccacagagatcctgcctgtgtccatgaccaagaccagcgtggactgcaccatgtacatctgcggcgattccaccgagtgctccaacctgctgctgcagtacggcagcttctgcacccagctgaatagagccctgaccgggatcgccgtggaacaggacaagaacacccaagaggtgttcgcccaagtgaagcagatctacaagacccctcctatcaaggacttcggcggcttcaatttcagccagattctgcccgatcctagcaagcccagcaagcggagcttcatcgaggacctgctgttcaacaaagtgacactggccgacgccggcttcatcaagcagtatggcgattgtctgggcgacattgccgccagggatctgatttgcgcccagaagtttaacggactgacagtgctgcctcctctgctgaccgatgagatgatcgcccagtacacatctgccctgctggccggcacaatcacaagcggctggacatttggagctggcgctgccctgcagatcccctttgctatgcagatggcctaccggttcaacggcatcggagtgacccagaatgtgctgtacgagaaccagaagctgatcgccaaccagttcaacagcgccatcggcaagatccaggacagcctgagcagcacagcaagcgccctgggaaagctgcaggacgtggtcaaccagaatgcccaggcactgaacaccctggtcaagcagctgtctagcaacttcggcgccatcagctctgtgctgaacgatatcctgagcagactggaccctcctgaggccgaggtgcagatcgacagactgatcacaggcagactgcagagcctccagacatacgtgacccagcagctgatcagagccgccgagattagagcctctgccaatctggccgccaccaagatgcgtgagtgtgtgctgggccagagcaagagagtggacttttgcggcaagggctaccacctgatgagcttccctcagtctgcccctcacggcgtggtgtttctgcacgtgacatatgtgcccgctcaagagaagaatttcaccaccgctccagccatctgccacgacggcaaagcccactttcctagagaaggcgtgttcgtgtccaacggcacccattggttcgtgacacagcggaacttctacgagccccgtatcatcaccaccgacaacaccttcgtgtctggcaactgcgacgtcgtgatcggcattgtgaacaataccgtgtacgaccctctgcagcccgagctggacagcttcaaagaggaactggacaagtactttaagaaccacacaagccccgacgtggacctgggcgatatcagcggaatcaatgccagcgtcgtgaacatccagaaagagatcgaccggctgaacgaggtggccaagaatttaaatgagagcctgatcgacctgcaagaactggggaagtacgagcaaggcggcggaggaacaggcggaggctatattcctgaggctcccagagatggccaggcctacgttagaaaggatggcgagtgggtgctgctgtccacctttctgggaagatctctggaagtgctgtttcaaggccctggccaccaccatcatcaccatcaccacagcgcttggagccatcctcagttcgagaaaggcggtggaagcggaggcggaggttctggcggatctgcttggtcacacccacagtttgagaagtga

SEQ ID NO: 68 - DNA, 3894 bp, synthetic construct
  source 1..3894: mol_type = other DNA
atggattggacctggcggttcctgtttgtggtggctgctgctacaggcgtgcagagcgtgaacctgaccaccagaacacagctgcctccagcctacaccaacagcttcaccagaggcgtgtactaccccgacaaggtgttcagatccagcgtgctgcactctacccaggacctgttcctgcctttcttcagcaacgtgacctggttccacgccatccacgtgtccggcaccaatggcaccaagagattcgacaaccccgtgctgcccttcaacgacggggtgtactttgccagcaccgagaagtccaacatcatcagaggctggatcttcggcaccacactggacagcaagacccagagcctgctgatcgtgaacaacgccaccaacgtggtcatcaaagtgtgcgagttccagttctgcaacgaccccttcctgggcgtctactaccacaagaacaacaagagctggatggaaagcgagttccgggtgtacagcagcgccaacaactgcaccttcgagtacgtgtcccagcctttcctgatggacctggaaggcaagcagggcaacttcaagaacctgcgcgagttcgtgttcaagaacatcgacggctacttcaagatctacagcaagcacacccctatcaacctcgtgcgggatctgcctcagggcttctctgctctggaacccctggtggatctgcccatcggcatcaacatcacccggtttcagacactgctggccctgcacagaagctacctgacacctggcgatagcagctctggatggacagctggcgccgctgcctactatgtgggatacctgcagcctcggaccttcctgctgaagtacaacgagaacggcaccatcaccgacgccgtggattgtgctctggatcctctgagcgagacaaagtgcaccctgaagtccttcaccgtggaaaagggcatctaccagaccagcaacttccgggtgcagcccaccgaatccatcgtgcggttccccaatatcaccaatctgtgccccttcggcgaggtgttcaatgccaccagattcgcctctgtgtacgcctggaaccggaagcggatcagcaattgcgtggccgactactccgtgctgtacaactccgccagcttcagcaccttcaagtgctacggcgtgtcccctaccaagctgaacgacctgtgcttcacaaacgtgtacgccgacagcttcgtgatccggggagatgaagtgcggcagattgcccctggacagacaggcaagatcgccgactacaactacaagctgcccgacgacttcaccggctgtgtgattgcctggaacagcaacaacctggactccaaagtcggcggcaactacaattacctgtaccggctgttccggaagtccaatctgaagcccttcgagcgggacatctccaccgagatctatcaggccggcagcaccccttgtaacggcgtggaaggcttcaactgctacttcccactgcagtcctacggctttcagcccacaaatggcgtgggctaccagccttacagagtggtggtgctgagcttcgagctgctgcatgctcctgccacagtgtgcggccctaagaaaagcaccaatctcgtgaagaacaaatgcgtgaacttcaacttcaacggcctgaccggaaccggcgtgctgacagagagcaacaagaagttcctgccattccagcagttcggccgggatatcgccgataccacagatgccgtcagagatccccagacactggaaatcctggacatcaccccttgcagcttcggcggagtgtctgtgatcacccctggcaccaacaccagcaatcaggtggcagtgctgtaccaggacgtgaactgtaccgaagtgcccgtggccattcacgccgatcagctgacacctacatggcgggtgtactccaccggcagcaatgtgtttcagaccagagccggctgtctgatcggagccgagcacgtgaacaatagctacgagtgcgacatccccatcggcgctggcatctgcgcctcttaccagacacagacaaacagccctggcagcgcctcttctgtggccagccagagcatcattgcctacacaatgtctctgggcgccgagaacagcgtggcctactccaacaactctatcgctatccccaccaacttcaccatcagcgtgaccacagagatcctgcctgtgtccatgaccaagaccagcgtggactgcaccatgtacatctgcggcgattccaccgagtgctccaacctgctgctgcagtacggcgagttctgcacccagctgaatagagccctgaccgggatcgccgtggaacaggacaagaacacccaagaggtgttcgcccaagtgaagcagatctacaagacccctcctatcaaggacttcggcggcttcaatttcagccagattctgcccgatcctagcaagcccagcaagcggagcttcatcgaggacctgctgttcaacaaagtgacactggccgacgccggcttcatcaagcagtatggcgattgtctgggcgacattgccgccagggatctgatttgcgcccagaagtttaacggactgacagtgctgcctcctctgctgaccgatgagatgatcgcccagtacacatctgccctgctggccggcacaatcacaagcggctggacatttggagctggcgctgccctgcagatcccctttgctatgcagatggcctaccggttcaacggcatcggagtgcggcagaatgtgctgtacgagaaccagaagctgatcgccaaccagttcaacagcgccatcggcaagatccaggacagcctgagcagcacagcaagcgccctgggaagactgcaggacgtggtcaaccagaatgcccaggcactgaacaccctggtcaagcagctgtctagcaacttcggcgccatcagctctgtgctgaacgatatcctgagcagactggaccctcctgaggccgaggtgcagatcgacagactgatcacaggcagactgcagagcctccagacatacgtgacccagcagctgatcagagccgccgagattagagcctctgccaatctggccgccaccaagatgtctgagtgtgtgctgggccagagcaagagagtggacttttgcggcaagggctaccacctgatgagcttccctcagtctgcccctcacggcgtggtgtttctgcacgtgacatatgtgcccgctcaagagaagaatttcaccaccgctccagccatctgccacgacggcaaagcccactttcctagagaaggcgtgttcgtgtccaacggcacccattggttcgtgacacagcggaacttctacgagccccagatcatcaccaccgacaacaccttcgtgtctggcaactgcgacgtcgtgatcggcattgtgaacaataccgtgtacgaccctctgcagcccgagctggacagcttcaaagaggaactggacaagtactttaagaaccacacaagccccgacgtggacctgggcgatatcagcggaatcaatgccagcgtcgtgaacatccagaaagagatcgaccggctgaacgaggtggccaagaatttaaatgagagcctgatcgacctgcaagaactggggaagtacgagcaaggcggcggaggaacaggcggaggctatattcctgaggctcccagagatggccaggcctacgttagaaaggatggcgagtgggtgctgctgtccacctttctgggaagatctctggaagtgctgtttcaaggccctggccaccaccatcatcaccatcaccacagcgcttggagccatcctcagttcgagaaaggcggtggaagcggaggcggaggttctggcggatctgcttggtcacacccacagtttgagaagtga

SEQ ID NO: 69 - DNA, 3894 bp, synthetic construct
  source 1..3894: mol_type = other DNA
atggattggacctggcggttcctgtttgtggtggctgctgctacaggcgtgcagagcgtgaacctgaccaccagaacacagctgcctccagcctacaccaacagcttcaccagaggcgtgtactaccccgacaaggtgttcagatccagcgtgctgcactctacccaggacctgttcctgcctttcttcagcaacgtgacctggttccacgccatccacgtgtccggcaccaatggcaccaagagattcgacaaccccgtgctgcccttcaacgacggggtgtactttgccagcaccgagaagtccaacatcatcagaggctggatcttcggcaccacactggacagcaagacccagagcctgctgatcgtgaacaacgccaccaacgtggtcatcaaagtgtgcgagttccagttctgcaacgaccccttcctgggcgtctactaccacaagaacaacaagagctggatggaaagcgagttccgggtgtacagcagcgccaacaactgcaccttcgagtacgtgtcccagcctttcctgatggacctggaaggcaagcagggcaacttcaagaacctgcgcgagttcgtgttcaagaacatcgacggctacttcaagatctacagcaagcacacccctatcaacctcgtgcgggatctgcctcagggcttctctgctctggaacccctggtggatctgcccatcggcatcaacatcacccggtttcagacactgctggccctgcacagaagctacctgacacctggcgatagcagctctggatggacagctggcgccgctgcctactatgtgggatacctgcagcctcggaccttcctgctgaagtacaacgagaacggcaccatcaccgacgccgtggattgtgctctggatcctctgagcgagacaaagtgcaccctgaagtccttcaccgtggaaaagggcatctaccagaccagcaacttccgggtgcagcccaccgaatccatcgtgcggttccccaatatcaccaatctgtgccccttcggcgaggtgttcaatgccaccagattcgcctctgtgtacgcctggaaccggaagcggatcagcaattgcgtggccgactactccgtgctgtacaactccgccagcttcagcaccttcaagtgctacggcgtgtcccctaccaagctgaacgacctgtgcttcacaaacgtgtacgccgacagcttcgtgatccggggagatgaagtgcggcagattgcccctggacagacaggcaagatcgccgactacaactacaagctgcccgacgacttcaccggctgtgtgattgcctggaacagcaacaacctggactccaaagtcggcggcaactacaattacctgtaccggctgttccggaagtccaatctgaagcccttcgagcgggacatctccaccgagatctatcaggccggcagcaccccttgtaacggcgtggaaggcttcaactgctacttcccactgcagtcctacggctttcagcccacaaatggcgtgggctaccagccttacagagtggtggtgctgagcttcgagctgctgcatgctcctgccacagtgtgcggccctaagaaaagcaccaatctcgtgaagaacaaatgcgtgaacttcaacttcaacggcctgaccggaaccggcgtgctgacagagagcaacaagaagttcctgccattccagcagttcggccgggatatcgccgataccacagatgccgtcagagatccccagacactggaaatcctggacatcaccccttgcagcttcggcggagtgtctgtgatcacccctggcaccaacaccagcaatcaggtggcagtgctgtaccaggacgtgaactgtaccgaagtgcccgtggccattcacgccgatcagctgacacctacatggcgggtgtactccaccggcagcaatgtgtttcagaccagagccggctgtctgatcggagccgagcacgtgaacaatagctacgagtgcgacatccccatcggcgctggcatctgcgcctcttaccagacacagacaaacagccctggcagcgcctcttctgtggccagccagagcatcattgcctacacaatgtctctgggcgccgagaacagcgtggcctactccaacaactctatcgctatccccaccaacttcaccatcagcgtgaccacagagatcctgcctgtgtccatgaccaagaccagcgtggactgcaccatgtacatctgcggcgattccaccgagtgctccaacctgctgctgcagtacggcagcttctgcacccagctgaatagagccctgaccgggatcgccgtggaacaggacaagaacacccaagaggtgttcgcccaagtgaagcagatctacaagacccctcctatcaaggacttcggcggcttcaatttcagccagattctgcccgatcctagcaagcccagcaagcggagcttcatcgaggacctgctgttcaacaaagtgacactggccgacgccggcttcatcaagcagtatggcgattgtctgggcgacattgccgccagggataagatttgcgcccagaagtttaacggactgacagtgctgcctcctctgctgaccgatgagatgatcgcccagtacacatctgccctgctggccggcacaatcacaagcggctggacatttggagctggcgctgccctgcagatcccctttgctatgcagatggcctaccggttcaacggcatcggagtgacccagaatgtgctgtacgagaaccagaagctgatcgccaaccagttcaacagcgccatcggcaagatccaggacagcctgagcagcacagcaagcgccctgggaaagctgcaggacgtggtcaaccagaatgcccaggcactgaacaccctggtcaagcagctgtctagcaacttcggcgccatcagctctgtgctgaacgatatcctgagcagactggaccctcctgaggccgaggtgcagatcgacagactgatcacaggcagactgcagagcctccagacatacgtgacccagcagctgatcagagccgccgagattagagcctctgccaatctggccgccaccaagatgtctgagtgtgtgctgggccagagcaagagagtggacttttgcggcaagggctaccacctgatgagcttccctcagtctgcccctcacggcgtggtgtttctgcacgtgacatatgtgcccgctcaagagaagaatttcaccaccgctccagccatctgccacgacggcaaagcccactttcctagagaaggcgtgttcgtgtccaacggcacccattggttcgtgacacagcggaacttctacgagccccagatcatcaccaccgacaacaccttcgtgtctggcaactgcgacgtcgtgatcggcattgtgaacaataccgtgtacgaccctctgcagcccgagctggacagcttcaaagaggaactggacaagtactttaagaaccacacaagccccgacgtggacctgggcgatatcagcggaatcaatgccagcgtcgtgaacatccagaaagagatcgaccggctgaacgaggtggccaagaatttaaatgagagcctgatcgacctgcaagaactggggaagtacgagcaaggcggcggaggaacaggcggaggctatattcctgaggctcccagagatggccaggcctacgttagaaaggatggcgagtgggtgctgctgtccacctttctgggaagatctctggaagtgctgtttcaaggccctggccaccaccatcatcaccatcaccacagcgcttggagccatcctcagttcgagaaaggcggtggaagcggaggcggaggttctggcggatctgcttggtcacacccacagtttgagaagtga

SEQ ID NO: 70 - DNA, 3897 bp, synthetic construct
  source 1..3897: mol_type = other DNA
atggattggacctggcggttcctgtttgtggtggctgctgctacaggcgtgcagagcgtgaacctgaccaccagaacacagctgcctccagcctacaccaacagcttcaccagaggcgtgtactaccccgacaaggtgttcagatccagcgtgctgcactctacccaggacctgttcctgcctttcttcagcaacgtgacctggttccacgccatccacgtgtccggcaccaatggcaccaagagattcgacaaccccgtgctgcccttcaacgacggggtgtactttgccagcaccgagaagtccaacatcatcagaggctggatcttcggcaccacactggacagcaagacccagagcctgctgatcgtgaacaacgccaccaacgtggtcatcaaagtgtgcgagttccagttctgcaacgaccccttcctgggcgtctactaccacaagaacaacaagagctggatggaaagcgagttccgggtgtacagcagcgccaacaactgcaccttcgagtacgtgtcccagcctttcctgatggacctggaaggcaagcagggcaacttcaagaacctgcgcgagttcgtgttcaagaacatcgacggctacttcaagatctacagcaagcacacccctatcaacctcgtgcgggatctgcctcagggcttctctgctctggaacccctggtggatctgcccatcggcatcaacatcacccggtttcagacactgctggccctgcacagaagctacctgacacctggcgatagcagctctggatggacagctggcgccgctgcctactatgtgggatacctgcagcctcggaccttcctgctgaagtacaacgagaacggcaccatcaccgacgccgtggattgtgctctggatcctctgagcgagacaaagtgcaccctgaagtccttcaccgtggaaaagggcatctaccagaccagcaacttccgggtgcagcccaccgaatccatcgtgcggttccccaatatcaccaatctgtgccccttcggcgaggtgttcaatgccaccagattcgcctctgtgtacgcctggaaccggaagcggatcagcaattgcgtggccgactactccgtgctgtacaactccgccagcttcagcaccttcaagtgctacggcgtgtcccctaccaagctgaacgacctgtgcttcacaaacgtgtacgccgacagcttcgtgatccggggagatgaagtgcggcagattgcccctggacagacaggcaagatcgccgactacaactacaagctgcccgacgacttcaccggctgtgtgattgcctggaacagcaacaacctggactccaaagtcggcggcaactacaattacctgtaccggctgttccggaagtccaatctgaagcccttcgagcgggacatctccaccgagatctatcaggccggcagcaccccttgtaacggcgtggaaggcttcaactgctacttcccactgcagtcctacggctttcagcccacaaatggcgtgggctaccagccttacagagtggtggtgctgagcttcgagctgctgcatgctcctgccacagtgtgcggccctaagaaaagcaccaatctcgtgaagaacaaatgcgtgaacttcaacttcaacggcctgaccggaaccggcgtgctgacagagagcaacaagaagttcctgccattccagcagttcggccgggatatcgccgataccacagatgccgtcagagatccccagacactggaaatcctggacatcaccccttgcagcttcggcggagtgtctgtgatcacccctggcaccaacaccagcaatcaggtggcagtgctgtaccaggacgtgaactgtaccgaagtgcccgtggccattcacgccgatcagctgacacctacatggcgggtgtactccaccggcagcaatgtgtttcagaccagagccggctgtctgatcggagccgagcacgtgaacaatagctacgagtgcgacatccccatcggcgctggcatctgcgcctcttaccagacacagacaaacagccctggcagcgcctcttctgtggccagccagagcatcattgcctacacaatgtctctgggcgccgagaacagcgtggcctactccaacaactctatcgctatccccaccaacttcaccatcagcgtgaccacagagatcctgcctgtgtccatgaccaagaccagcgtggactgcaccatgtacatctgcggcgattccaccgagtgctccaacctgctgctgcagtacggcagcttctgcacccagctgaatagagccctgaccgggatcgccgtggaacaggacaagaacacccaagaggtgttcgcccaagtgaagcagatctacaagacccctcctatcaaggacttcggcggcttcaatttcagccagattctgcccgatcctagcaagcccagcaagcggagcttcatcgaggacctgctgttcaacaaagtgacactggccgacgccggcttcatcaagcagtatggcgattgtctgggcgacattgccgccagggatctgatttgcgcccagaagtttaacggactgacagtgctgcctcctctgctgaccgatgagatgatcgcccagtacacatctgccctgctggccggcacaatcacaagcggctggacatttggagctggcgctgccctgcagatcccctttgctatgcagatggcctaccggttcaacggcatcggagtgacccagaatgtgctgtacgagaaccagaagctgatcgccaaccagttcaacagcgccatcggcaagatccaggacagcctgagcagcacagcaagcgccctgggaaagctgcaggacgtggtcaaccagaatgcccaggcactgaacgagctggtcaagcagctgtctagcaacttcggcgccatcagctctgtgctgaacgatatcctgagcagactggaccctcctgaggccgaggtgcagatcgacagactgatcacaggcagactgcagagcctccagacatacgtgacccagcagctgatcagagccgccgagattagagcctctgccaatctggccgccaccaagatgtctgagtgtgtgctgggccagagcaagagagtggacttttgcggcaagggctaccacctgatgagcttccctcagtctgcccctcacggcgtggtgtttctgcacgtgacatatgtgcccgctcaagagaagaatttcaccaccgctccagccatctgccacgacggcaaagcccactttcctagagaaggcgtgttcgtgtccaacggcacccattggttcgtgacacagcggaacttctacgagccccagatcatcaccaccgacaacaccttcgtgtctggcaactgcgacgtcgtgatcggcattgtgaacaataccgtgtacgaccctctgcagcccgagctggacagcttcaaagaggaactggacaagtactttaagaaccacacaagccccgacgtggacctgggcgatatcagcggaatcaatgccagcgtcgtgaacatccagaaagagatcgaccggctgaacgaggtggccaagaatttaaatgagagcctgatcgacctgcaagaactggggaagtacgagcaaggcggcggaggaacaggcggaggctatattcctgaggctcccagagatggccaggcctacgttagaaaggatggcgagtgggtgctgctgtccacctttctgggaagatctctggaagtgctgtttcaaggccctggccaccaccatcatcaccatcaccacagcgcttggagccatcctcagttcgagaaaggcggtggaagcggaggcggaggttctggcggatctgcttggtcacacccacagtttgagaagtgatga

SEQ ID NO: 71 - protein, 6 aa, synthetic construct
LVPRGS

SEQ ID NO: 72 - protein, 7 aa, synthetic construct
ENLYFQG

SEQ ID NO: 73 - protein, 7 aa, synthetic construct
ENLYFQS

SEQ ID NO: 74 - protein, 4 aa, synthetic construct
IEGR

SEQ ID NO: 75 - protein, 4 aa, synthetic construct
IDGR

SEQ ID NO: 76 - protein, 8 aa, synthetic construct
LEVLFQGP

SEQ ID NO: 77 - protein, 1273 aa, synthetic construct
MFVFLVLLPLVSSQCVNLTTRTQLPPAYTNSFTRGVYYPDKVFRSSVLHSTQDLFLPFFSNVTWFHAIHVSGTNGTKRFDNPVLPFNDGVYFASTEKSNIIRGWIFGTTLDSKTQSLLIVNNATNVVIKVCEFQFCNDPFLGVYYHKNNKSWMESEFRVYSSANNCTFEYVSQPFLMDLEGKQGNFKNLREFVFKNIDGYFKIYSKHTPINLVRDLPQGFSALEPLVDLPIGINITRFQTLLALHRSYLTPGDSSSGWTAGAAAYYVGYLQPRTFLLKYNENGTITDAVDCALDPLSETKCTLKSFTVEKGIYQTSNFRVQPTESIVRFPNITNLCPFGEVFNATRFASVYAWNRKRISNCVADYSVLYNSASFSTFKCYGVSPTKLNDLCFTNVYADSFVIRGDEVRQIAPGQTGKIADYNYKLPDDFTGCVIAWNSNNLDSKVGGNYNYLYRLFRKSNLKPFERDISTEIYQAGSTPCNGVEGFNCYFPLQSYGFQPTNGVGYQPYRVVVLSFELLHAPATVCGPKKSTNLVKNKCVNFNFNGLTGTGVLTESNKKFLPFQQFGRDIADTTDAVRDPQTLEILDITPCSFGGVSVITPGTNTSNQVAVLYQDVNCTEVPVAIHADQLTPTWRVYSTGSNVFQTRAGCLIGAEHVNNSYECDIPIGAGICASYQTQTNSPRRARSVASQSIIAYTMSLGAENSVAYSNNSIAIPTNFTISVTTEILPVSMTKTSVDCTMYICGDSTECSNLLLQYGSFCTQLNRALTGIAVEQDKNTQEVFAQVKQIYKTPPIKDFGGFNFSQILPDPSKPSKRSFIEDLLFNKVTLADAGFIKQYGDCLGDIAARDLICAQKFNGLTVLPPLLTDEMIAQYTSALLAGTITSGWTFGAGAALQIPFAMQMAYRFNGIGVTQNVLYENQKLIANQFNSAIGKIQDSLSSTASALGKLQDVVNQNAQALNTLVKQLSSNFGAISSVLNDILSRLDKVEAEVQIDRLITGRLQSLQTYVTQQLIRAAEIRASANLAATKMSECVLGQSKRVDFCGKGYHLMSFPQSAPHGVVFLHVTYVPAQEKNFTTAPAICHDGKAHFPREGVFVSNGTHWFVTQRNFYEPQIITTDNTFVSGNCDVVIGIVNNTVYDPLQPELDSFKEELDKYFKNHTSPDVDLGDISGINASVVNIQKEIDRLNEVAKNLNESLIDLQELGKYEQYIKWPWYIWLGFIAGLIAIVMVTIMLCCMTSCCSCLKGCCSCGSCCKFDEDDSEPVLKGVKLHYT

SEQ ID NO: 78 - protein, 1258 aa, synthetic construct
VNLTTRTQLPPAYTNSFTRGVYYPDKVFRSSVLHSTQDLFLPFFSNVTWFHAIHVSGTNGTKRFDNPVLPFNDGVYFASTEKSNIIRGWIFGTTLDSKTQSLLIVNNATNVVIKVCEFQFCNDPFLGVYYHKNNKSWMESEFRVYSSANNCTFEYVSQPFLMDLEGKQGNFKNLREFVFKNIDGYFKIYSKHTPINLVRDLPQGFSALEPLVDLPIGINITRFQTLLALHRSYLTPGDSSSGWTAGAAAYYVGYLQPRTFLLKYNENGTITDAVDCALDPLSETKCTLKSFTVEKGIYQTSNFRVQPTESIVRFPNITNLCPFGEVFNATRFASVYAWNRKRISNCVADYSVLYNSASFSTFKCYGVSPTKLNDLCFTNVYADSFVIRGDEVRQIAPGQTGKIADYNYKLPDDFTGCVIAWNSNNLDSKVGGNYNYLYRLFRKSNLKPFERDISTEIYQAGSTPCNGVEGFNCYFPLQSYGFQPTNGVGYQPYRVVVLSFELLHAPATVCGPKKSTNLVKNKCVNFNFNGLTGTGVLTESNKKFLPFQQFGRDIADTTDAVRDPQTLEILDITPCSFGGVSVITPGTNTSNQVAVLYQDVNCTEVPVAIHADQLTPTWRVYSTGSNVFQTRAGCLIGAEHVNNSYECDIPIGAGICASYQTQTNSPRRARSVASQSIIAYTMSLGAENSVAYSNNSIAIPTNFTISVTTEILPVSMTKTSVDCTMYICGDSTECSNLLLQYGSFCTQLNRALTGIAVEQDKNTQEVFAQVKQIYKTPPIKDFGGFNFSQILPDPSKPSKRSFIEDLLFNKVTLADAGFIKQYGDCLGDIAARDLICAQKFNGLTVLPPLLTDEMIAQYTSALLAGTITSGWTFGAGAALQIPFAMQMAYRFNGIGVTQNVLYENQKLIANQFNSAIGKIQDSLSSTASALGKLQDVVNQNAQALNTLVKQLSSNFGAISSVLNDILSRLDKVEAEVQIDRLITGRLQSLQTYVTQQLIRAAEIRASANLAATKMSECVLGQSKRVDFCGKGYHLMSFPQSAPHGVVFLHVTYVPAQEKNFTTAPAICHDGKAHFPREGVFVSNGTHWFVTQRNFYEPQIITTDNTFVSGNCDVVIGIVNNTVYDPLQPELDSFKEELDKYFKNHTSPDVDLGDISGINASVVNIQKEIDRLNEVAKNLNESLIDLQELGKYEQYIKWPWYIWLGFIAGLIAIVMVTIMLCCMTSCCSCLKGCCSCGSCCKFDEDDSEPVLKGVKLHYT

SEQ ID NO: 79 - protein, 12 aa, synthetic construct
GGGGTGGGRSGS

SEQ ID NO: 80 - protein, 5 aa, synthetic construct
RRARS

SEQ ID NO: 81 - protein, 7 aa, synthetic construct
GGSSGGS

SEQ ID NO: 82 - protein, 14 aa, synthetic construct
SGGTSGSTSGTGST

SEQ ID NO: 83 - protein, 15 aa, synthetic construct
AGSSTGSSTGPGSTT

SEQ ID NO: 84 - protein, 7 aa, synthetic construct
GGSGGAP

SEQ ID NO: 85 - protein, 8 aa, synthetic construct
GGGVEGGG

SEQ ID NO: 86 - protein, 10 aa, synthetic construct
PKPSTPPGSS

SEQ ID NO: 87 - protein, 11 aa, synthetic construct
APAETKAEPMT

SEQ ID NO: 88 - protein, 5 aa, synthetic construct
AAALE

SEQ ID NO: 89 - protein, 29 aa, synthetic construct
WSHPQFEKGGGSGGGGSGGSAWSHPQFEK

SEQ ID NO: 90 - DNA, 26 bp, synthetic construct
  source 1..26: mol_type = other DNA
acactagccatccttactgcgcttcg

SEQ ID NO: 91 - DNA, 23 bp, synthetic construct
  source 1..23: mol_type = other DNA
cgatctcttgtagatctgttctc

SEQ ID NO: 92 - DNA, 26 bp, synthetic construct
  source 1..26: mol_type = other DNA
acactagccatccttactgcgcttcg

SEQ ID NO: 93 - DNA, 23 bp, synthetic construct
  source 1..23: mol_type = other DNA
atattgcagcagtacgcacacaa

SEQ ID NO: 94 - DNA, 26 bp, synthetic construct
  source 1..26: mol_type = other DNA
acaggtacgttaatagttaatagcgt

SEQ ID NO: 95 - DNA, 22 bp, synthetic construct
  source 1..22: mol_type = other DNA
atattgcagcagtacgcacaca

SEQ ID NO: 96 - protein, 5 aa, synthetic construct
HHHHH

SEQ ID NO: 97 - protein, 10 aa, synthetic construct
EQKLISEEDL

SEQ ID NO: 98 - protein, 8 aa, synthetic construct
DYKDDDDK

SEQ ID NO: 99 - protein, 9 aa, synthetic construct
YPYDVPDYA

SEQ ID NO: 100 - protein, 5 aa, synthetic construct
RYIRS

SEQ ID NO: 101 - protein, 4 aa, synthetic construct
FHHT

SEQ ID NO: 102 - protein, 17 aa, synthetic construct
WEAAAREACCRECCARA

SEQ ID NO: 103 - protein, 1227 aa, synthetic construct
VNLTTRTQLPPAYTNSFTRGVYYPDKVFRSSVLHSTQDLFLPFFSNVTWFHAIHVSGTNGTKRFDNPVLPFNDGVYFASTEKSNIIRGWIFGTTLDSKTQSLLIVNNATNVVIKVCEFQFCNDPFLGVYYHKNNKSWMESEFRVYSSANNCTFEYVSQPFLMDLEGKQGNFKNLREFVFKNIDGYFKIYSKHTPINLVRDLPQGFSALEPLVDLPIGINITRFQTLLALHRSYLTPGDSSSGWTAGAAAYYVGYLQPRTFLLKYNENGTITDAVDCALDPLSETKCTLKSFTVEKGIYQTSNFRVQPTESIVRFPNITNLCPFGEVFNATRFASVYAWNRKRISNCVADYSVLYNSASFSTFKCYGVSPTKLNDLCFTNVYADSFVIRGDEVRQIAPGQTGKIADYNYKLPDDFTGCVIAWNSNNLDSKVGGNYNYLYRLFRKSNLKPFERDISTEIYQAGSTPCNGVEGFNCYFPLQSYGFQPTNGVGYQPYRVVVLSFELLHAPATVCGPKKSTNLVKNKCVNFNFNGLTGTGVLTESNKKFLPFQQFGRDIADTTDAVRDPQTLEILDITPCSFGGVSVITPGTNTSNQVAVLYQDVNCTEVPVAIHADQLTPTWRVYSTGSNVFQTRAGCLIGAEHVNNSYECDIPIGAGICASYQTQTNSPGSASSVASQSIIAYTMSLGAENSVAYSNNSIAIPTNFTISVTTEILPVSMTKTSVDCTMYICGDSTECSNLLLQYGSFCTQLNRALTGIAVEQDKNTQEVFAQVKQIYKTPPIKDFGGFNFSQILPDPSKPSKRSFIEDLLFNKVTLADAGFIKQYGDCLGDIAARDLICAQKFNGLTVLPPLLTDEMIAQYTSALLAGTITSGWTFGAGAALQIPFAMQMAYRFNGIGVTQNVLYENQKLIANQFNSAIGKIQDSLSSTASALGKLQDVVNQNAQALNTLVKQLSSNFGAISSVLNDILSRLDKHEAEVQIDRLITGRLQSLQTYVTQQLIRAAEIRASANLAATKMSECVLGQSKRVDFCGKGYHLMSFPQSAPHGVVFLHVTYVPAQEKNFTTAPAICHDGKAHFPREGVFVSNGTHWFVTQRNFYEPQIITTDNTFVSGNCDVVIGIVNNTVYDPLQPELDSFKEELDKYFKNHTSPDVDLGDISGINASVVNIQKEIDRLNEVAKNLNESLIDLQELGKYEQGGGGTGGGYIPEAPRDGQAYVRKDGEWVLLSTFL

SEQ ID NO: 104 - protein, 1227 aa, synthetic construct
VNLTTRTQLPPAYTNSFTRGVYYPDKVFRSSVLHSTQDLFLPFFSNVTWFHAIHVSGTNGTKRFDNPVLPFNDGVYFASTEKSNIIRGWIFGTTLDSKTQSLLIVNNATNVVIKVCEFQFCNDPFLGVYYHKNNKSWMESEFRVYSSANNCTFEYVSQPFLMDLEGKQGNFKNLREFVFKNIDGYFKIYSKHTPINLVRDLPQGFSALEPLVDLPIGINITRFQTLLALHRSYLTPGDSSSGWTAGAAAYYVGYLQPRTFLLKYNENGTITDAVDCALDPLSETKCTLKSFTVEKGIYQTSNFRVQPTESIVRFPNITNLCPFGEVFNATRFASVYAWNRKRISNCVADYSVLYNSASFSTFKCYGVSPTKLNDLCFTNVYADSFVIRGDEVRQIAPGQTGKIADYNYKLPDDFTGCVIAWNSNNLDSKVGGNYNYLYRLFRKSNLKPFERDISTEIYQAGSTPCNGVEGFNCYFPLQSYGFQPTNGVGYQPYRVVVLSFELLHAPATVCGPKKSTNLVKNKCVNFNFNGLTGTGVLTESNKKFLPFQQFGRDIADTTDAVRDPQTLEILDITPCSFGGVSVITPGTNTSNQVAVLYQDVNCTEVPVAIHADQLTPTWRVYSTGSNVFQTRAGCLIGAEHVNNSYECDIPIGAGICASYQTQTNSPGSASSVASQSIIAYTMSLGAENSVAYSNNSIAIPTNFTISVTTEILPVSMTKTSVDCTMYICGDSTECSNLLLQYGSFCTQLNRALTGIAVEQDKNTQEVFAQVKQIYKTPPIKDFGGFNFSQILPDPSKPSKRSFIEDLLFNKVTLADAGFIKQYGDCLGDIAARDLICAQKFNGLTVLPPLLTDEMIAQYTSALLAGTITSGWTFGAGAALQIPFAMQMAYRFNGIGVTQNVLYENQKLIANQFNSAIGKIQDSLSSTASALGKLQDVVNQNAQALNTLVKQLSSNFGAISSVLNDILSRLLKVEAEVQIDRLITGRLQSLQTYVTQQLIRAAEIRASANLAATKMSECVLGQSKRVDFCGKGYHLMSFPQSAPHGVVFLHVTYVPAQEKNFTTAPAICHDGKAHFPREGVFVSNGTHWFVTQRNFYEPQIITTDNTFVSGNCDVVIGIVNNTVYDPLQPELDSFKEELDKYFKNHTSPDVDLGDISGINASVVNIQKEIDRLNEVAKNLNESLIDLQELGKYEQGGGGTGGGYIPEAPRDGQAYVRKDGEWVLLSTFL

SEQ ID NO: 105 - protein, 1227 aa, synthetic construct
VNLTTRTQLPPAYTNSFTRGVYYPDKVFRSSVLHSTQDLFLPFFSNVTWFHAIHVSGTNGTKRFDNPVLPFNDGVYFASTEKSNIIRGWIFGTTLDSKTQSLLIVNNATNVVIKVCEFQFCNDPFLGVYYHKNNKSWMESEFRVYSSANNCTFEYVSQPFLMDLEGKQGNFKNLREFVFKNIDGYFKIYSKHTPINLVRDLPQGFSALEPLVDLPIGINITRFQTLLALHRSYLTPGDSSSGWTAGAAAYYVGYLQPRTFLLKYNENGTITDAVDCALDPLSETKCTLKSFTVEKGIYQTSNFRVQPTESIVRFPNITNLCPFGEVFNATRFASVYAWNRKRISNCVADYSVLYNSASFSTFKCYGVSPTKLNDLCFTNVYADSFVIRGDEVRQIAPGQTGKIADYNYKLPDDFTGCVIAWNSNNLDSKVGGNYNYLYRLFRKSNLKPFERDISTEIYQAGSTPCNGVEGFNCYFPLQSYGFQPTNGVGYQPYRVVVLSFELLHAPATVCGPKKSTNLVKNKCVNFNFNGLTGTGVLTESNKKFLPFQQFGRDIADTTDAVRDPQTLEILDITPCSFGGVSVITPGTNTSNQVAVLYQDVNCTEVPVAIHADQLTPTWRVYSTGSNVFQTRAGCLIGAEHVNNSYECDIPIGAGICASYQTQTNSPGSASSVASQSIIAYTMSLGAENSVAYSNNSIAIPTNFTISVTTEILPVSMTKTSVDCTMYICGDSTECSNLLLQYGSFCTQLNRALTGIAVEQDKNTQEVFAQVKQIYKTPPIKDFGGFNFSQILPDPSKPSKRSFIEDLLFNKVTLADAGFIKQYGDCLGDIAARDLICAQKFNGLTVLPPLLTDEMIAQYTSALLAGTITSGWTFGAGAALQIPFAMQMAYRFNGIGVTQNVLYENQKLIANQFNSAIGKIQDSLSSTASALGKLQDVVNQNAQALNTLVKQLSSNFGAISSVLNDILFRLDKVEAEVQIDRLITGRLQSLQTYVTQQLIRAAEIRASANLAATKMSECVLGQSKRVDFCGKGYHLMSFPQSAPHGVVFLHVTYVPAQEKNFTTAPAICHDGKAHFPREGVFVSNGTHWFVTQRNFYEPQIITTDNTFVSGNCDVVIGIVNNTVYDPLQPELDSFKEELDKYFKNHTSPDVDLGDISGINASVVNIQKEIDRLNEVAKNLNESLIDLQELGKYEQGGGGTGGGYIPEAPRDGQAYVRKDGEWVLLSTFL

SEQ ID NO: 106 - protein, 1227 aa, synthetic construct
VNLTTRTQLPPAYTNSFTRGVYYPDKVFRSSVLHSTQDLFLPFFSNVTWFHAIHVSGTNGTKRFDNPVLPFNDGVYFASTEKSNIIRGWIFGTTLDSKTQSLLIVNNATNVVIKVCEFQFCNDPFLGVYYHKNNKSWMESEFRVYSSANNCTFEYVSQPFLMDLEGKQGNFKNLREFVFKNIDGYFKIYSKHTPINLVRDLPQGFSALEPLVDLPIGINITRFQTLLALHRSYLTPGDSSSGWTAGAAAYYVGYLQPRTFLLKYNENGTITDAVDCALDPLSETKCTLKSFTVEKGIYQTSNFRVQPTESIVRFPNITNLCPFGEVFNATRFASVYAWNRKRISNCVADYSVLYNSASFSTFKCYGVSPTKLNDLCFTNVYADSFVIRGDEVRQIAPGQTGKIADYNYKLPDDFTGCVIAWNSNNLDSKVGGNYNYLYRLFRKSNLKPFERDISTEIYQAGSTPCNGVEGFNCYFPLQSYGFQPTNGVGYQPYRVVVLSFEYLHAPATVCGPKKSTNLVKNKCVNFNFNGLTGTGVLTESNKKFLPFQQFGRDIADTTDAVRDPQTLEILDITPCSFGGVSVITPGTNTSNQVAVLYQDVNCTEVPVAIHADQLTPTWRVYSTGSNVFQTRAGCLIGAEHVNNSYECDIPIGAGICASYQTQTNSPGSASSVASQSIIAYTMSLGAENSVAYSNNSIAIPTNFTISVTTEILPVSMTKTSVDCTMYICGDSTECSNLLLQYGSFCTQLNRALTGIAVEQDKNTQEVFAQVKQIYKTPPIKDFGGFNFSQILPDPSKPSKRSFIEDLLFNKVTLADAGFIKQYGDCLGDIAARDLICAQKFNGLTVLPPLLTDEMIAQYTSALLAGTITSGWTFGAGAALQIPFAMQMAYRFNGIGVTQNVLYENQKLIANQFNSAIGKIQDSLSSTASALGKLQDVVNQNAQALNTLVKQLSSNFGAISSVLNDILSRLDKVEAEVQIDRLITGRLQSLQTYVTQQLIRAAEIRASANLAATKMSECVLGQSKRVDFCGKGYHLMSFPQSAPHGVVFLHVTYVPAQEKNFTTAPAICHDGKAHFPREGVFVSNGTHWFVTQRNFYEPQIITTDNTFVSGNCDVVIGIVNNTVYDPLQPELDSFKEELDKYFKNHTSPDVDLGDISGINASVVNIQKEIDRLNEVAKNLNESLIDLQELGKYEQGGGGTGGGYIPEAPRDGQAYVRKDGEWVLLSTFL

SEQ ID NO: 107 - protein, 1227 aa, synthetic construct
VNLTTRTQLPPAYTNSFTRGVYYPDKVFRSSVLHSTQDLFLPFFSNVTWFHAIHVSGTNGTKRFDNPVLPFNDGVYFASTEKSNIIRGWIFGTTLDSKTQSLLIVNNATNVVIKVCEFQFCNDPFLGVYYHKNNKSWMESEFRVYSSANNCTFEYVSQPFLMDLEGKQGNFKNLREFVFKNIDGYFKIYSKHTPINLVRDLPQGFSALEPLVDLPIGINITRFQTLLALHRSYLTPGDSSSGWTAGAAAYYVGYLQPRTFLLKYNENGTITDAVDCALDPLSETKCTLKSFTVEKGIYQTSNFRVQPTESIVRFPNITNLCPFGEVFNATRFASVYAWNRKRISNCVADYSVLYNSASFSTFKCYGVSPTKLNDLCFTNVYADSFVIRGDEVRQIAPGQTRKIADYNYKLPDDFTGCVIAWNSNNLDSKVGGNYNYLYRLFRKSNLKPFERDISTEIYQAGSTPCNGVEGFNCYFPLQSYGFQPTNGVGYQPYRVVVLSFELLHAPATVCGPKKSTNLVKNKCVNFNFNGLTGTGVLTESNKKFLPFQQFGRDIADTTDAVRDPQTLEILDITPCSFGGVSVITPGTNTSNQVAVLYQDVNCTEVPVAIHADQLTPTWRVYSTGSNVFQTRAGCLIGAEHVNNSYECDIPIGAGICASYQTQTNSPGSASSVASQSIIAYTMSLGAENSVAYSNNSIAIPTNFTISVTTEILPVSMTKTSVDCTMYICGDSTECSNLLLQYGSFCTQLNRALTGIAVEQDKNTQEVFAQVKQIYKTPPIKDFGGFNFSQILPDPSKPSKRSFIEDLLFNKVTLADAGFIKQYGDCLGDIAARDLICAQKFNGLTVLPPLLTDEMIAQYTSALLAGTITSGWTFGAGAALQIPFAMQMAYRFNGIGVTQNVLYENQKLIANQFNSAIGKIQDSLSSTASALGKLQDVVNQNAQALNTLVKQLSSNFGAISSVLNDILSRLDKVEAEVQIDRLITGRLQSLQTYVTQQLIRAAEIRASANLAATKMSECVLGQSKRVDFCGKGYHLMSFPQSAPHGVVFLHVTYVPAQEKNFTTAPAICHDGKAHFPREGVFVSNGTHWFVTQRNFYEPQIITTDNTFVSGNCDVVIGIVNNTVYDPLQPELDSFKEELDKYFKNHTSPDVDLGDISGINASVVNIQKEIDRLNEVAKNLNESLIDLQELGKYEQGGGGTGGGYIPEAPRDGQAYVRKDGEWVLLSTFL

SEQ ID NO: 108 - protein, 1227 aa, synthetic construct
VNLTTRTQLPPAYTNSFTRGVYYPDKVFRSSVLHSTQDLFLPFFSNVTWFHAIHVSGTNGTKRFDNPVLPFNDGVYFASTEKSNIIRGWIFGTTLDSKTQSLLIVNNATNVVIKVCEFQFCNDPFLGVYYHKNNKSWMESEFRVYSSANNCTFEYVSQPFLMDLEGKQGNFKNLREFVFKNIDGYFKIYSKHTPINLVRDLPQGFSALEPLVDLPIGINITRFQTLLALHRSYLTPGDSSSGWTAGAAAYYVGYLQPRTFLLKYNENGTITDAVDCALDPLSETKCTLKSFTVEKGIYQTSNFRVQPTESIVRFPNITNLCPFGEVFNATRFASVYAWNRKRISNCVADYSVLYNSASFSTFKCYGVSPTRLNDLCFTNVYADSFVIRGDEVRQIAPGQTGKIADYNYKLPDDFTGCVIAWNSNNLDSKVGGNYNYLYRLFRKSNLKPFERDISTEIYQAGSTPCNGVEGFNCYFPLQSYGFQPTNGVGYQPYRVVVLSFELLHAPATVCGPKKSTNLVKNKCVNFNFNGLTGTGVLTESNKKFLPFQQFGRDIADTTDAVRDPQTLEILDITPCSFGGVSVITPGTNTSNQVAVLYQDVNCTEVPVAIHADQLTPTWRVYSTGSNVFQTRAGCLIGAEHVNNSYECDIPIGAGICASYQTQTNSPGSASSVASQSIIAYTMSLGAENSVAYSNNSIAIPTNFTISVTTEILPVSMTKTSVDCTMYICGDSTECSNLLLQYGSFCTQLNRALTGIAVEQDKNTQEVFAQVKQIYKTPPIKDFGGFNFSQILPDPSKPSKRSFIEDLLFNKVTLADAGFIKQYGDCLGDIAARDLICAQKFNGLTVLPPLLTDEMIAQYTSALLAGTITSGWTFGAGAALQIPFAMQMAYRFNGIGVTQNVLYENQKLIANQFNSAIGKIQDSLSSTASALGKLQDVVNQNAQALNTLVKQLSSNFGAISSVLNDILSRLDKVEAEVQIDRLITGRLQSLQTYVTQQLIRAAEIRASANLAATKMSECVLGQSKRVDFCGKGYHLMSFPQSAPHGVVFLHVTYVPAQEKNFTTAPAICHDGKAHFPREGVFVSNGTHWFVTQRNFYEPQIITTDNTFVSGNCDVVIGIVNNTVYDPLQPELDSFKEELDKYFKNHTSPDVDLGDISGINASVVNIQKEIDRLNEVAKNLNESLIDLQELGKYEQGGGGTGGGYIPEAPRDGQAYVRKDGEWVLLSTFL

SEQ ID NO: 109 - protein, 1227 aa, synthetic construct
VNLTTRTQLPPAYTNSFTRGVYYPDKVFRSSVLHSTQDLFLPFFSNVTWFHAIHVSGTNGTKRFDNPVLPFNDGVYFASTEKSNIIRGWIFGTTLDSKTQSLLIVNNATNVVIKVCEFQFCNDPFLGVYYHKNNKSWMESEFRVYSSANNCTFEYVSQPFLMDLEGKQGNFKNLREFVFKNIDGYFKIYSKHTPINLVRDLPQGFSALEPLVDLPIGINITRFQTLLALHRSYLTPGDSSSGWTAGAAAYYVGYLQPRTFLLKYNENGTITDAVDCALDPLSETKCTLKSFTVEKGIYQTSNFRVQPTESIVRFPNITNLCPFGEVFNATRFASVYAWNRKRISNCVADYSVLYNSASFSTFKCYGVSPTKLNDLCFTNVYADSFVIRGDEVRQIAPGQTGKIADYNYKLPDDFTGCVIAWNSNNLDSKVGGNYNYLYRLFRKSNLKPFERDISTEIYQAGSTPCNGVEGFNCYFPLQSYGFQPTNGVGYQPYRVVVLSFELLHAPATVCGPKKSTNLVKNKCVNFNFNGLTGTGVLTESNKKFLPFQQFGRDIADTTDAVRDPQTLEILDITPCSFGGVSVITPGTNTSNQVAVLYQDVNCTEVPVAIHADQLTPTWRVYSTGSNVFQTRAGCLIGAEHVNNSYECDIPIGAGICASYQTQTNSPGSASSVASQSIIAYTMSLGAENSVAYSNNSIAIPTNFTISVTTEILPVSMTKTSVDCTMYICGDSTECSNLLLQYGSFCTQLNRALTGIAVEQDKNTQEVFAQVKQIYKTPPIKDFGGFNFSQILPDPSKPSKRSFIEDLLFNKVTLADAGFIKQYGDCLGDIAARDLICAQKFNGLTVLPPLLTDEMIAQYTSALLAGTITSGWTFGAGAALQIPFAMQMAYRFNGIGVTQNVLYENQKLIANQFNSAIGKIQDSLSSTASALGKLQDVVNQNAQALNTLVKQLSSNFGAISSVLNDILSRLDKWEAEVQIDRLITGRLQSLQTYVTQQLIRAAEIRASANLAATKMSECVLGQSKRVDFCGKGYHLMSFPQSAPHGVVFLHVTYVPAQEKNFTTAPAICHDGKAHFPREGVFVSNGTHWFVTQRNFYEPQIITTDNTFVSGNCDVVIGIVNNTVYDPLQPELDSFKEELDKYFKNHTSPDVDLGDISGINASVVNIQKEIDRLNEVAKNLNESLIDLQELGKYEQGGGGTGGGYIPEAPRDGQAYVRKDGEWVLLSTFL

SEQ ID NO: 110 - protein, 1227 aa, synthetic construct
VNLTTRTQLPPAYTNSFTRGVYYPDKVFRSSVLHSTQDLFLPFFSNVTWFHAIHVSGTNGTKRFDNPVLPFNDGVYFASTEKSNIIRGWIFGTTLDSKTQSLLIVNNATNVVIKVCEFQFCNDPFLGVYYHKNNKSWMESEFRVYSSANNCTFEYVSQPFLMDLEGKQGNFKNLREFVFKNIDGYFKIYSKHTPINLVRDLPQGFSALEPLVDLPIGINITRFQTLLALHRSYLTPGDSSSGWTAGAAAYYVGYLQPRTFLLKYNENGTITDAVDCALDPLSETKCTLKSFTVEKGIYQTSNFRVQPTESIVRFPNITNLCPFGEVFNATRFASVYAWNRKRISNCVADYSVLYNSASFSTFKCYGVSPTKLNDLCFTNVYADSFVIRGDEVRQIAPGQTGKIADYNYKLPIDFTGCVIAWNSNNLDSKVGGNYNYLYRLFRKSNLKPFERDISTEIYQAGSTPCNGVEGFNCYFPLQSYGFQPTNGVGYQPYRVVVLSFELLHAPATVCGPKKSTNLVKNKCVNFNFNGLTGTGVLTESNKKFLPFQQFGRDIADTTDAVRDPQTLEILDITPCSFGGVSVITPGTNTSNQVAVLYQDVNCTEVPVAIHADQLTPTWRVYSTGSNVFQTRAGCLIGAEHVNNSYECDIPIGAGICASYQTQTNSPGSASSVASQSIIAYTMSLGAENSVAYSNNSIAIPTNFTISVTTEILPVSMTKTSVDCTMYICGDSTECSNLLLQYGSFCTQLNRALTGIAVEQDKNTQEVFAQVKQIYKTPPIKDFGGFNFSQILPDPSKPSKRSFIEDLLFNKVTLADAGFIKQYGDCLGDIAARDLICAQKFNGLTVLPPLLTDEMIAQYTSALLAGTITSGWTFGAGAALQIPFAMQMAYRFNGIGVTQNVLYENQKLIANQFNSAIGKIQDSLSSTASALGKLQDVVNQNAQALNTLVKQLSSNFGAISSVLNDILSRLDKVEAEVQIDRLITGRLQSLQTYVTQQLIRAAEIRASANLAATKMSECVLGQSKRVDFCGKGYHLMSFPQSAPHGVVFLHVTYVPAQEKNFTTAPAICHDGKAHFPREGVFVSNGTHWFVTQRNFYEPQIITTDNTFVSGNCDVVIGIVNNTVYDPLQPELDSFKEELDKYFKNHTSPDVDLGDISGINASVVNIQKEIDRLNEVAKNLNESLIDLQELGKYEQGGGGTGGGYIPEAPRDGQAYVRKDGEWVLLSTFL

SEQ ID NO: 111 - protein, 1227 aa, synthetic construct
VNLTTRTQLPPAYTNSFTRGVYYPDKVFRSSVLHSTQDLFLPFFSNVTWFHAIHVSGTNGTKRFDNPVLPFNDGVYFASTEKSNIIRGWIFGTTLDSKTQSLLIVNNATNVVIKVCEFQFCNDPFLGVYYHKNNKSWMESEFRVYSSANNCTFEYVSQPFLMDLEGKQGNFKNLREFVFKNIDGYFKIYSKHTPINLVRDLPQGFSALEPLVDLPIGINITRFQTLLALHRSYLTPGDSSSGWTAGAAAYYVGYLQPRTFLLKYNENGTITDAVDCALDPLSETKCTLKSFTVEKGIYQTSNFRVQPTESIVRFPNITNLCPFGEVFNATRFASVYAWNRKRISNCVADYSVLYNSASFSTFKCYGVSPTKLNDLCFTNVYADSFVIRGDEVRQIAPGQTGKIARYNYKLPDDFTGCVIAWNSNNLDSKVGGNYNYLYRLFRKSNLKPFERDISTEIYQAGSTPCNGVEGFNCYFPLQSYGFQPTNGVGYQPYRVVVLSFELLHAPATVCGPKKSTNLVKNKCVNFNFNGLTGTGVLTESNKKFLPFQQFGRDIADTTDAVRDPQTLEILDITPCSFGGVSVITPGTNTSNQVAVLYQDVNCTEVPVAIHADQLTPTWRVYSTGSNVFQTRAGCLIGAEHVNNSYECDIPIGAGICASYQTQTNSPGSASSVASQSIIAYTMSLGAENSVAYSNNSIAIPTNFTISVTTEILPVSMTKTSVDCTMYICGDSTECSNLLLQYGSFCTQLNRALTGIAVEQDKNTQEVFAQVKQIYKTPPIKDFGGFNFSQILPDPSKPSKRSFIEDLLFNKVTLADAGFIKQYGDCLGDIAARDLICAQKFNGLTVLPPLLTDEMIAQYTSALLAGTITSGWTFGAGAALQIPFAMQMAYRFNGIGVTQNVLYENQKLIANQFNSAIGKIQDSLSSTASALGKLQDVVNQNAQALNTLVKQLSSNFGAISSVLNDILSRLDKVEAEVQIDRLITGRLQSLQTYVTQQLIRAAEIRASANLAATKMSECVLGQSKRVDFCGKGYHLMSFPQSAPHGVVFLHVTYVPAQEKNFTTAPAICHDGKAHFPREGVFVSNGTHWFVTQRNFYEPQIITTDNTFVSGNCDVVIGIVNNTVYDPLQPELDSFKEELDKYFKNHTSPDVDLGDISGINASVVNIQKEIDRLNEVAKNLNESLIDLQELGKYEQGGGGTGGGYIPEAPRDGQAYVRKDGEWVLLSTFL

SEQ ID NO: 112 - protein, 1227 aa, synthetic construct
VNLTTRTQLPPAYTNSFTRGVYYPDKVFRSSVLHSTQDLFLPFFSNVTWFHAIHVSGTNGTKRFDNPVLPFNDGVYFASTEKSNIIRGWIFGTTLDSKTQSLLIVNNATNVVIKVCEFQFCNDPFLGVYYHKNNKSWMESEFRVYSSANNCTFEYVSQPFLMDLEGKQGNFKNLREFVFKNIDGYFKIYSKHTPINLVRDLPQGFSALEPLVDLPIGINITRFQTLLALHRSYLTPGDSSSGWTAGAAAYYVGYLQPRTFLLKYNENGTITDAVDCALDPLSETKCTLKSFTVEKGIYQTSNFRVQPTESIVRFPNITNLCPFGEVFNATRFASVYAWNRKRISNCVADYSVLYNSWSFSTFKCYGVSPTKLNDLCFTNVYADSFVIRGDEVRQIAPGQTGKIADYNYKLPDDFTGCVIAWNSNNLDSKVGGNYNYLYRLFRKSNLKPFERDISTEIYQAGSTPCNGVEGFNCYFPLQSYGFQPTNGVGYQPYRVVVLSFELLHAPATVCGPKKSTNLVKNKCVNFNFNGLTGTGVLTESNKKFLPFQQFGRDIADTTDAVRDPQTLEILDITPCSFGGVSVITPGTNTSNQVAVLYQDVNCTEVPVAIHADQLTPTWRVYSTGSNVFQTRAGCLIGAEHVNNSYECDIPIGAGICASYQTQTNSPGSASSVASQSIIAYTMSLGAENSVAYSNNSIAIPTNFTISVTTEILPVSMTKTSVDCTMYICGDSTECSNLLLQYGSFCTQLNRALTGIAVEQDKNTQEVFAQVKQIYKTPPIKDFGGFNFSQILPDPSKPSKRSFIEDLLFNKVTLADAGFIKQYGDCLGDIAARDLICAQKFNGLTVLPPLLTDEMIAQYTSALLAGTITSGWTFGAGAALQIPFAMQMAYRFNGIGVTQNVLYENQKLIANQFNSAIGKIQDSLSSTASALGKLQDVVNQNAQALNTLVKQLSSNFGAISSVLNDILSRLDKVEAEVQIDRLITGRLQSLQTYVTQQLIRAAEIRASANLAATKMSECVLGQSKRVDFCGKGYHLMSFPQSAPHGVVFLHVTYVPAQEKNFTTAPAICHDGKAHFPREGVFVSNGTHWFVTQRNFYEPQIITTDNTFVSGNCDVVIGIVNNTVYDPLQPELDSFKEELDKYFKNHTSPDVDLGDISGINASVVNIQKEIDRLNEVAKNLNESLIDLQELGKYEQGGGGTGGGYIPEAPRDGQAYVRKDGEWVLLSTFL

SEQ ID NO: 113 - protein, 1227 aa, synthetic construct
VNLTTRTQLPPAYTNSFTRGVYYPDKVFRSSVLHSTQDLFLPFFSNVTWFHAIHVSGTNGTKRFDNPVLPFNDGVYFASTEKSNIIRGWIFGTTLDSKTQSLLIVNNATNVVIKVCEFQFCNDPFLGVYYHKNNKSWMESEFRVYSSANNCTFEYVSQPFLMDLEGKQGNFKNLREFVFKNIDGYFKIYSKHTPINLVRDLPQGFSALEPLVDLPIGINITRFQTLLALHRSYLTPGDSSSGWTAGAAAYYVGYLQPRTFLLKYNENGTITDAVDCALDPLSETKCTLKSFTVEKGIYQTSNFRVQPTESIVRFPNITNLCPFGEVFNATRFASVYAWNRKRISNCVADYSVLYNSASFSTFKCYGVSPTKLNDLCFTNVYADSFVIRGDEVRQIAPGQTGKIAYYNYKLPDDFTGCVIAWNSNNLDSKVGGNYNYLYRLFRKSNLKPFERDISTEIYQAGSTPCNGVEGFNCYFPLQSYGFQPTNGVGYQPYRVVVLSFELLHAPATVCGPKKSTNLVKNKCVNFNFNGLTGTGVLTESNKKFLPFQQFGRDIADTTDAVRDPQTLEILDITPCSFGGVSVITPGTNTSNQVAVLYQDVNCTEVPVAIHADQLTPTWRVYSTGSNVFQTRAGCLIGAEHVNNSYECDIPIGAGICASYQTQTNSPGSASSVASQSIIAYTMSLGAENSVAYSNNSIAIPTNFTISVTTEILPVSMTKTSVDCTMYICGDSTECSNLLLQYGSFCTQLNRALTGIAVEQDKNTQEVFAQVKQIYKTPPIKDFGGFNFSQILPDPSKPSKRSFIEDLLFNKVTLADAGFIKQYGDCLGDIAARDLICAQKFNGLTVLPPLLTDEMIAQYTSALLAGTITSGWTFGAGAALQIPFAMQMAYRFNGIGVTQNVLYENQKLIANQFNSAIGKIQDSLSSTASALGKLQDVVNQNAQALNTLVKQLSSNFGAISSVLNDILSRLDKVEAEVQIDRLITGRLQSLQTYVTQQLIRAAEIRASANLAATKMSECVLGQSKRVDFCGKGYHLMSFPQSAPHGVVFLHVTYVPAQEKNFTTAPAICHDGKAHFPREGVFVSNGTHWFVTQRNFYEPQIITTDNTFVSGNCDVVIGIVNNTVYDPLQPELDSFKEELDKYFKNHTSPDVDLGDISGINASVVNIQKEIDRLNEVAKNLNESLIDLQELGKYEQGGGGTGGGYIPEAPRDGQAYVRKDGEWVLLSTFL

SEQ ID NO: 114 - protein, 1227 aa, synthetic construct
VNLTTRTQLPPAYTNSFTRGVYYPDKVFRSSVLHSTQDLFLPFFSNVTWFHAIHVSGTNGTKRFDNPVLPFNDGVYFASTEKSNIIRGWIFGTTLDSKTQSLLIVNNATNVVIKVCEFQFCNDPFLGVYYHKNNKSWMESEFRVYSSANNCTFEYVSQPFLMDLEGKQGNFKNLREFVFKNIDGYFKIYSKHTPINLVRDLPQGFSALEPLVDLPIGINITRFQTLLALHRSYLTPGDSSSGWTAGAAAYYVGYLQPRTFLLKYNENGTITDAVDCALDPLSETKCTLKSFTVEKGIYQTSNFRVQPTESIVRFPNITNLCPFGEVFNATRFASVYAWNRKRISNCVADYSVLYNSWSFSTFKCYGVSPTKLNDLCFTNVYADSFVIRGDEVRQIAPGQTGKIARYNYKLPDDFTGCVIAWNSNNLDSKVGGNYNYLYRLFRKSNLKPFERDISTEIYQAGSTPCNGVEGFNCYFPLQSYGFQPTNGVGYQPYRVVVLSFELLHAPATVCGPKKSTNLVKNKCVNFNFNGLTGTGVLTESNKKFLPFQQFGRDIADTTDAVRDPQTLEILDITPCSFGGVSVITPGTNTSNQVAVLYQDVNCTEVPVAIHADQLTPTWRVYSTGSNVFQTRAGCLIGAEHVNNSYECDIPIGAGICASYQTQTNSPGSASSVASQSIIAYTMSLGAENSVAYSNNSIAIPTNFTISVTTEILPVSMTKTSVDCTMYICGDSTECSNLLLQYGSFCTQLNRALTGIAVEQDKNTQEVFAQVKQIYKTPPIKDFGGFNFSQILPDPSKPSKRSFIEDLLFNKVTLADAGFIKQYGDCLGDIAARDLICAQKFNGLTVLPPLLTDEMIAQYTSALLAGTITSGWTFGAGAALQIPFAMQMAYRFNGIGVTQNVLYENQKLIANQFNSAIGKIQDSLSSTASALGKLQDVVNQNAQALNTLVKQLSSNFGAISSVLNDILSRLDKVEAEVQIDRLITGRLQSLQTYVTQQLIRAAEIRASANLAATKMSECVLGQSKRVDFCGKGYHLMSFPQSAPHGVVFLHVTYVPAQEKNFTTAPAICHDGKAHFPREGVFVSNGTHWFVTQRNFYEPQIITTDNTFVSGNCDVVIGIVNNTVYDPLQPELDSFKEELDKYFKNHTSPDVDLGDISGINASVVNIQKEIDRLNEVAKNLNESLIDLQELGKYEQGGGGTGGGYIPEAPRDGQAYVRKDGEWVLLSTFL

SEQ ID NO: 115 - protein, 1227 aa, synthetic construct
VNLTTRTQLPPAYTNSFTRGVYYPDKVFRSSVLHSTQDLFLPFFSNVTWFHAIHVSGTNGTKRFDNPVLPFNDGVYFASTEKSNIIRGWIFGTTLDSKTQSLLIVNNATNVVIKVCEFQFCNDPFLGVYYHKNNKSWMESEFRVYSSANNCTFEYVSQPFLMDLEGKQGNFKNLREFVFKNIFGYFKIYSKHTPINLVRDLPQGFSALEPLVDLPILINITRFQTLLALHRSYLTPGDSSSGWTAGAAAYYVGYLQPRTFLLKYNENGTITDAVDCALDPLSETKCTLKSFTVEKGIYQTSNFRVQPTESIVRFPNITNLCPFGEVFNATRFASVYAWNRKRISNCVADYSVLYNSWSFSTFKCYGVSPTKLNDLCFTQVYADSFVIRGDEVRQIAPGQTGKIARYNYKLPDDFTGCVIAWNSNNLDSKVGGNYNYLYRLFRKSNLKPFERDISTEIYQAGSTPCNGVEGFNCYFPLQSYGFQPTNGVGYQPYRVVVLSFELLHAPATVCGPKKSTNLVKNKCVNFNFNGLTGTGVLTESNKKFLPFQQFGRDIADTTDAVRDPQTLEILDITPCSFGGVSVITPGTNTSNQVAVLYQDVNCTEVPVAIHADQLTPTWRVYSTGSNVFQTRAGCLIGAEHVNNSYECDIPIGAGICASYQTQTNSPGSASSVASQSIIAYTMSLGAENSVAYSNNSIAIPTNFTISVTTEILPVSMTKTSVDCTMYICGDSTECSNLLLQYGSFCTQLNRALTGIAVEQDKNTQEVFAQVKQIYKTPPIKDFGGFNFSQILPDPSKPSKRSFIEDLLFNKVTLADAGFIKQYGDCLGDIAARDLICAQKFNGLTVLPPLLTDEMIAQYTSALLAGTITSGWTFGAGAALQIPFAMQMAYRFNGIGVTQNVLYENQKLIANQFNSAIGKIQDSLSSTASALGKLQDVVNQNAQALNTLVKQLSSNFGAISSVLNDILSRLDKVEAEVQIDRLITGRLQSLQTYVTQQLIRAAEIRASANLAATKMSECVLGQSKRVDFCGKGYHLMSFPQSAPHGVVFLHVTYVPAQEKNFTTAPAICHDGKAHFPREGVFVSNGTHWFVTQRNFYEPQIITTDNTFVSGNCDVVIGIVNNTVYDPLQPELDSFKEELDKYFKNHTSPDVDLGDISGINASVVNIQKEIDRLNEVAKNLNESLIDLQELGKYEQGGGGTGGGYIPEAPRDGQAYVRKDGEWVLLSTFL

SEQ ID NO: 116 - protein, 1227 aa, synthetic construct
VNLTTRTQLPPAYTNSFTRGVYYPDKVFRSSVLHSTQDLFLPFFSNVTWFHAIHVSGTNGTKRFDNPVLPFNDGVYFASTEKSNIIRGWIFGTTLDSKTQSLLIVNNATNVVIKVCEFQFCNDPFLGVYYHKNNKSWMESEFRVYSSANNCTFEYVSQPFLMDLEGKQGNFKNLREFVFKNIDGYFKIYSKHTPINLVRDLPQGFSALEPLVDLPIGINITRFQTLLALHRSYLTPGDSSSGWTAGAAAYYVGYLQPRTFLLKYNENGTITDAVDCALDPLSETKCTLKSFTVEKGIYQTSNFRVQPTESIVRFPNITNLCPFGEVFNATRFASVYAWNRKRISNCVADYSVLYNSASFSTFKCYGVSPTKLNDLCFTNVYADSFVIRGDEVRQIAPGQTGKIADYNYKLPDDFTGCVIAWNSNNLDSKVGGNYNYLYRLFRKSNLKPFERDISTEIYQAGSTPCNGVEGFNCYFPLQSYGFQPTNGVGYQPYRVVVLSFELLHAPATVCGPKKSTNLVKNKCVNFNFNGLTGTGVLTESNKKFLPFQQFGRDIADTTDAVRDPQTLEILDITPCSFGGVSVITPGTNTSNQVAVLYQDVNCTEVPVAIHADQLTPTWRVYSTGSNVFQTRAGCLIGAEHVNNSYECDIPIGAGICASYQTQTNSPGSASSVASQSIIAYTMSLGAENSVQYSNNSIAIPTNFTISVTTEILPVSMTKTSVDCTMYICGDSTECSNLLLQYGEFCTQLNRALTGIAVEQDKNTQEVFAQVKQIYKTPPIKDFGGFNFSQILPDPSKPSKRSFIEDLLFNKVTLADAGFIKQYGDCLGDIAARDKICAQKFNGLTVLPPLLTDEMIAQYTSALLAGTITSGWTFGAGAALQIPFAMQMAYRFNGIGVTQNVLYENQKLIANQFNSAIGKIQDSLSSTASALGKLQDVVNQNAQALNTLEKQLSSNFGAISSVLNDILSRLDPPEAEVQIDRLITGRLQSLQTYVTQQLIRAAEIRASANLAATKMRECVLGQSKRVDFCGKGYHLMSFPQSAPHGVVFLHVTYVPAQEKNFTTAPAICHDGKAHFPREGVFVSNGTHWFVTQRNFYEPRIITTDNTFVSGNCDVVIGIVNNTVYDPLQPELDSFKEELDKYFKNHTSPDVDLGDISGINASVVNIQKEIDRLNEVAKNLNESLIDLQELGKYEQGGGGTGGGYIPEAPRDGQAYVRKDGEWVLLSTFL

SEQ ID NO: 117 - protein, 1227 aa, synthetic construct
VNLTTRTQLPPAYTNSFTRGVYYPDKVFRSSVLHSTQDLFLPFFSNVTWFHAIHVSGTNGTKRFDNPVLPFNDGVYFASTEKSNIIRGWIFGTTLDSKTQSLLIVNNATNVVIKVCEFQFCNDPFLGVYYHKNNKSWMESEFRVYSSANNCTFEYVSQPFLMDLEGKQGNFKNLREFVFKNIDGYFKIYSKHTPINLVRDLPQGFSALEPLVDLPIGINITRFQTLLALHRSYLTPGDSSSGWTAGAAAYYVGYLQPRTFLLKYNENGTITDAVDCALDPLSETKCTLKSFTVEKGIYQTSNFRVQPTESIVRFPNITNLCPFGEVFNATRFASVYAWNRKRISNCVADYSVLYNSASFSTFKCYGVSPTKLNDLCFTNVYADSFVIRGDEVRQIAPGQTGKIADYNYKLPDDFTGCVIAWNSNNLDSKVGGNYNYLYRLFRKSNLKPFERDISTEIYQAGSTPCNGVEGFNCYFPLQSYGFQPTNGVGYQPYRVVVLSFELLHAPATVCGPKKSTNLVKNKCVNFNFNGLTGTGVLTESNKKFLPFQQFGRDIADTTDAVRDPQTLEILDITPCSFGGVSVITPGTNTSNQVAVLYQDVNCTEVPVAIHADQLTPTWRVYSTGSNVFQTRAGCLIGAEHVNNSYECDIPIGAGICASYQTQTNSPGSASSVASQSIIAYTMSLGAENSVAYSNNSIAIPTNFTISVTTEILPVSMTKTSVDCTMYICGDSTECSNLLLKYGSFCTQLNRALTGIAVEQDKNTQEVFAQVKQIYKTPPIKDFGGFNFSQILPDPSKPSKRSFIEDLLFNKVTLADAGFIKQYGDCLGDIAARDKICAQKFNGLTVLPPLLTDEMIAQYTSALLAGTITSGWTFGAGNALQIPFAMQMAYRFNGIGVTQNVLYENQKLIANQFNSAIGKIQDSLSSTASALGRLQDVVNQNAQALNTLVKQLSSNFGAISSVLNDILSRLDPPEAEVQIDRLITGRLQSLQTYVTQQLIRAAEIRASANLAATKMSECVLGQSKRVDFCGRGYHLMSFPQSAPHGVVFLHVTYVPAQEKNFTTAPAICHDGKAHFPREGVFVSNGTHWFVTQRNFYEPQIITTDNTFVSGNCDVVIGIVNNTVYDPLQPELDSFKEELDKYFKNHTSPDVDLGDISGINASVVNIQKEIDRLNEVAKNLNESLIDLQELGKYEQGGGGTGGGYIPEAPRDGQAYVRKDGEWVLLSTFL

SEQ ID NO: 118 - protein, 1226 aa, synthetic construct
NLTTRTQLPPAYTNSFTRGVYYPDKVFRSSVLHSTQDLFLPFFSNVTWFHAIHVSGTNGTKRFDNPVLPFNDGVYFASTEKSNIIRGWIFGTTLDSKTQSLLIVNNATNVVIKVCEFQFCNDPFLGVYYHKNNKSWMESEFRVYSSANNCTFEYVSQPFLMDLEGKQGNFKNLREFVFKNIDGYFKIYSKHTPINLVRDLPQGFSALEPLVDLPIGINITRFQTLLALHRSYLTPGDSSSGWTAGAAAYYVGYLQPRTFLLKYNENGTITDAVDCALDPLSETKCTLKSFTVEKGIYQTSNFRVQPTESIVRFPNITNLCPFGEVFNATRFASVYAWNRKRISNCVADYSVLYNSASFSTFKCYGVSPTKLNDLCFTNVYADSFVIRGDEVRQIAPGQTGKIADYNYKLPDDFTGCVIAWNSNNLDSKVGGNYNYLYRLFRKSNLKPFERDISTEIYQAGSTPCNGVEGFNCYFPLQSYGFQPTNGVGYQPYRVVVLSFELLHAPATVCGPKKSTNLVKNKCVNFNFNGLTGTGVLTESNKKFLPFQQFGRDIADTTDAVRDPQTLEILDITPCSFGGVSVITPGTNTSNQVAVLYQDVNCTEVPVAIHADQLTPTWRVYSTGSNVFQTRAGCLIGAEHVNNSYECDIPIGAGICASYQTQTNSPGSASSVASQSIIAYTMSLGAENSVAYSNNSIAIPTNFTISVTTEILPVSMTKTSVDCTMYICGDSTECSNLLLQYGEFCTQLNRALTGIAVEQDKNTQEVFAQVKQIYKTPPIKDFGGFNFSQILPDPSKPSKRSFIEDLLFNKVTLADAGFIKQYGDCLGDIAARDKICAQKFNGLTVLPPLLTDEMIAQYTSALLAGTITSGWTFGAGAALQIPFAMQMAYRFNGIGVTQNVLYENQKLIANQFNSAIGKIQDSLSSTASALGKLQDVVNQNAQALNTLEKQLSSNFGAISSVLNDILSRLDPPEAEVQIDRLITGRLQSLQTYVTQQLIRAAEIRASANLAATKMSECVLGQSKRVDFCGKGYHLMSFPQSAPHGVVFLHVTYVPAQEKNFTTAPAICHDGKAHFPREGVFVSNGTHWFVTQRNFYEPQIITTDNTFVSGNCDVVIGIVNNTVYDPLQPELDSFKEELDKYFKNHTSPDVDLGDISGINASVVNIQKEIDRLNEVAKNLNESLIDLQELGKYEQGGGGTGGGYIPEAPRDGQAYVRKDGEWVLLSTFL

SEQ ID NO: 119 - protein, 1227 aa, synthetic construct
VNLTTRTQLPPAYTNSFTRGVYYPDKVFRSSVLHSTQDLFLPFFSNVTWFHAIHVSGTNGTKRFDNPVLPFNDGVYFASTEKSNIIRGWIFGTTLDSKTQSLLIVNNATNVVIKVCEFQFCNDPFLGVYYHKNNKSWMESEFRVYSSANNCTFEYVSQPFLMDLEGKQGNFKNLREFVFKNIDGYFKIYSKHTPINLVRDLPQGFSALEPLVDLPIGINITRFQTLLALHRSYLTPGDSSSGWTAGAAAYYVGYLQPRTFLLKYNENGTITDAVDCALDPLSETKCTLKSFTVEKGIYQTSNFRVQPTESIVRFPNITNLCPFGEVFNATRFASVYAWNRKRISNCVADYSVLYNSASFSTFKCYGVSPTKLNDLCFTNVYADSFVIRGDEVRQIAPGQTGKIADYNYKLPDDFTGCVIAWNSNNLDSKVGGNYNYLYRLFRKSNLKPFERDISTEIYQAGSTPCNGVEGFNCYFPLQSYGFQPTNGVGYQPYRVVVLSFELLHAPATVCGPKKSTNLVKNKCVNFNFNGLTGTGVLTESNKKFLPFQQFGRDIADTTDAVRDPQTLEILDITPCSFGGVSVITPGTNTSNQVAVLYQDVNCTEVPVAIHADQLTPTWRVYSTGSNVFQTRAGCLIGAEHVNNSYECDIPIGAGICASYQTQTNSPGSASSVASQSIIAYTMSLGAENSVAYSNNSIAIPTNFTISVTTEILPVSMTKTSVDCTMYICGDSTECSNLLLKYGSFCTQLNRALTGIAVEQDKNTQEVFAQVKQIYKTPPIKDFGGFNFSQILPDPSKPSKRSFIEDLLFNKVTLADAGFIKQYGDCLGDIAARDLIQAQKFNGLTVLPPLLTDEMIAQYTSALLAGTITSGWTFGAGAALQIPFAMQMAYRFNGIGVTQNVLYENQKLIANQFNSAIGKIQDSLSSTASALGKLQDVVNQNAQALNELVKQLSSNFGAISSVLNDILSRLDPPEAEVQIDRLITGRLQSLQTYVTQQLIRAAEIRASANLAATKMSECVLGQSKRVDFCGKGYHLMSFPQSAPHGVVFLHVTYVPAQEKNFTTAPAICHDGKAHFPREGVFVSNGTHWFVTQRNFYEPQIITTDNTFVSGNCDVVIGIVNNTVYDPLQPELDSFKEELDKYFKNHTSPDVDLGDISGINASVVNIQKEIDRLNEVAKNLNESLIDLQELGKYEQGGGGTGGGYIPEAPRDGQAYVRKDGEWVLLSTFL

SEQ ID NO: 120 - protein, 1227 aa, synthetic construct
VNLTTRTQLPPAYTNSFTRGVYYPDKVFRSSVLHSTQDLFLPFFSNVTWFHAIHVSGTNGTKRFDNPVLPFNDGVYFASTEKSNIIRGWIFGTTLDSKTQSLLIVNNATNVVIKVCEFQFCNDPFLGVYYHKNNKSWMESEFRVYSSANNCTFEYVSQPFLMDLEGKQGNFKNLREFVFKNIDGYFKIYSKHTPINLVRDLPQGFSALEPLVDLPIGINITRFQTLLALHRSYLTPGDSSSGWTAGAAAYYVGYLQPRTFLLKYNENGTITDAVDCALDPLSETKCTLKSFTVEKGIYQTSNFRVQPTESIVRFPNITNLCPFGEVFNATRFASVYAWNRKRISNCVADYSVLYNSASFSTFKCYGVSPTKLNDLCFTNVYADSFVIRGDEVRQIAPGQTGKIADYNYKLPDDFTGCVIAWNSNNLDSKVGGNYNYLYRLFRKSNLKPFERDISTEIYQAGSTPCNGVEGFNCYFPLQSYGFQPTNGVGYQPYRVVVLSFELLHAPATVCGPKKSTNLVKNKCVNFNFNGLTGTGVLTESNKKFLPFQQFGRDIADTTDAVRDPQTLEILDITPCSFGGVSVITPGTNTSNQVAVLYQDVNCTEVPVAIHADQLTPTWRVYSTGSNVFQTRAGCLIGAEHVNNSYECDIPIGAGICASYQTQTNSPGSASSVASQSIIAYTMSLGAENSVQYSNNSIAIPTNFTISVTTEILPVSMTKTSVDCTMYICGDSTECSNLLLQYGSFCTQLNRALTGIAVEQDKNTQEVFAQVKQIYKTPPIKDFGGFNFSQILPDPSKPSKRSFIEDLLFNKVTLADAGFIKQYGDCLGDIAARDLICAQKFNGLTVLPPLLTDEMIAQYTSALLAGTITSGWTFGAGAALQIPFAMQMAYRFNGIGVTQNVLYENQKLIANQFNSAIGKIQDSLSSTASALGKLQDVVNQNAQALNTLVKQLSSNFGAISSVLNDILSRLDPPEAEVQIDRLITGRLQSLQTYVTQQLIRAAEIRASANLAATKMRECVLGQSKRVDFCGKGYHLMSFPQSAPHGVVFLHVTYVPAQEKNFTTAPAICHDGKAHFPREGVFVSNGTHWFVTQRNFYEPRIITTDNTFVSGNCDVVIGIVNNTVYDPLQPELDSFKEELDKYFKNHTSPDVDLGDISGINASVVNIQKEIDRLNEVAKNLNESLIDLQELGKYEQGGGGTGGGYIPEAPRDGQAYVRKDGEWVLLSTFL

SEQ ID NO: 121 - protein, 1227 aa, synthetic construct
VNLTTRTQLPPAYTNSFTRGVYYPDKVFRSSVLHSTQDLFLPFFSNVTWFHAIHVSGTNGTKRFDNPVLPFNDGVYFASTEKSNIIRGWIFGTTLDSKTQSLLIVNNATNVVIKVCEFQFCNDPFLGVYYHKNNKSWMESEFRVYSSANNCTFEYVSQPFLMDLEGKQGNFKNLREFVFKNIDGYFKIYSKHTPINLVRDLPQGFSALEPLVDLPIGINITRFQTLLALHRSYLTPGDSSSGWTAGAAAYYVGYLQPRTFLLKYNENGTITDAVDCALDPLSETKCTLKSFTVEKGIYQTSNFRVQPTESIVRFPNITNLCPFGEVFNATRFASVYAWNRKRISNCVADYSVLYNSASFSTFKCYGVSPTKLNDLCFTNVYADSFVIRGDEVRQIAPGQTGKIADYNYKLPDDFTGCVIAWNSNNLDSKVGGNYNYLYRLFRKSNLKPFERDISTEIYQAGSTPCNGVEGFNCYFPLQSYGFQPTNGVGYQPYRVVVLSFELLHAPATVCGPKKSTNLVKNKCVNFNFNGLTGTGVLTESNKKFLPFQQFGRDIADTTDAVRDPQTLEILDITPCSFGGVSVITPGTNTSNQVAVLYQDVNCTEVPVAIHADQLTPTWRVYSTGSNVFQTRAGCLIGAEHVNNSYECDIPIGAGICASYQTQTNSPGSASSVASQSIIAYTMSLGAENSVAYSNNSIAIPTNFTISVTTEILPVSMTKTSVDCTMYICGDSTECSNLLLQYGEFCTQLNRALTGIAVEQDKNTQEVFAQVKQIYKTPPIKDFGGFNFSQILPDPSKPSKRSFIEDLLFNKVTLADAGFIKQYGDCLGDIAARDLICAQKFNGLTVLPPLLTDEMIAQYTSALLAGTITSGWTFGAGAALQIPFAMQMAYRFNGIGVRQNVLYENQKLIANQFNSAIGKIQDSLSSTASALGRLQDVVNQNAQALNTLVKQLSSNFGAISSVLNDILSRLDPPEAEVQIDRLITGRLQSLQTYVTQQLIRAAEIRASANLAATKMSECVLGQSKRVDFCGKGYHLMSFPQSAPHGVVFLHVTYVPAQEKNFTTAPAICHDGKAHFPREGVFVSNGTHWFVTQRNFYEPQIITTDNTFVSGNCDVVIGIVNNTVYDPLQPELDSFKEELDKYFKNHTSPDVDLGDISGINASVVNIQKEIDRLNEVAKNLNESLIDLQELGKYEQGGGGTGGGYIPEAPRDGQAYVRKDGEWVLLSTFL

SEQ ID NO: 122 - protein, 1227 aa, synthetic construct
VNLTTRTQLPPAYTNSFTRGVYYPDKVFRSSVLHSTQDLFLPFFSNVTWFHAIHVSGTNGTKRFDNPVLPFNDGVYFASTEKSNIIRGWIFGTTLDSKTQSLLIVNNATNVVIKVCEFQFCNDPFLGVYYHKNNKSWMESEFRVYSSANNCTFEYVSQPFLMDLEGKQGNFKNLREFVFKNIDGYFKIYSKHTPINLVRDLPQGFSALEPLVDLPIGINITRFQTLLALHRSYLTPGDSSSGWTAGAAAYYVGYLQPRTFLLKYNENGTITDAVDCALDPLSETKCTLKSFTVEKGIYQTSNFRVQPTESIVRFPNITNLCPFGEVFNATRFASVYAWNRKRISNCVADYSVLYNSASFSTFKCYGVSPTKLNDLCFTNVYADSFVIRGDEVRQIAPGQTGKIADYNYKLPDDFTGCVIAWNSNNLDSKVGGNYNYLYRLFRKSNLKPFERDISTEIYQAGSTPCNGVEGFNCYFPLQSYGFQPTNGVGYQPYRVVVLSFELLHAPATVCGPKKSTNLVKNKCVNFNFNGLTGTGVLTESNKKFLPFQQFGRDIADTTDAVRDPQTLEILDITPCSFGGVSVITPGTNTSNQVAVLYQDVNCTEVPVAIHADQLTPTWRVYSTGSNVFQTRAGCLIGAEHVNNSYECDIPIGAGICASYQTQTNSPGSASSVASQSIIAYTMSLGAENSVAYSNNSIAIPTNFTISVTTEILPVSMTKTSVDCTMYICGDSTECSNLLLQYGSFCTQLNRALTGIAVEQDKNTQEVFAQVKQIYKTPPIKDFGGFNFSQILPDPSKPSKRSFIEDLLFNKVTLADAGFIKQYGDCLGDIAARDKICAQKFNGLTVLPPLLTDEMIAQYTSALLAGTITSGWTFGAGAALQIPFAMQMAYRFNGIGVTQNVLYENQKLIANQFNSAIGKIQDSLSSTASALGKLQDVVNQNAQALNTLVKQLSSNFGAISSVLNDILSRLDPPEAEVQIDRLITGRLQSLQTYVTQQLIRAAEIRASANLAATKMSECVLGQSKRVDFCGKGYHLMSFPQSAPHGVVFLHVTYVPAQEKNFTTAPAICHDGKAHFPREGVFVSNGTHWFVTQRNFYEPQIITTDNTFVSGNCDVVIGIVNNTVYDPLQPELDSFKEELDKYFKNHTSPDVDLGDISGINASVVNIQKEIDRLNEVAKNLNESLIDLQELGKYEQGGGGTGGGYIPEAPRDGQAYVRKDGEWVLLSTFL

SEQ ID NO: 123 - protein, 1227 aa, synthetic construct
VNLTTRTQLPPAYTNSFTRGVYYPDKVFRSSVLHSTQDLFLPFFSNVTWFHAIHVSGTNGTKRFDNPVLPFNDGVYFASTEKSNIIRGWIFGTTLDSKTQSLLIVNNATNVVIKVCEFQFCNDPFLGVYYHKNNKSWMESEFRVYSSANNCTFEYVSQPFLMDLEGKQGNFKNLREFVFKNIDGYFKIYSKHTPINLVRDLPQGFSALEPLVDLPIGINITRFQTLLALHRSYLTPGDSSSGWTAGAAAYYVGYLQPRTFLLKYNENGTITDAVDCALDPLSETKCTLKSFTVEKGIYQTSNFRVQPTESIVRFPNITNLCPFGEVFNATRFASVYAWNRKRISNCVADYSVLYNSASFSTFKCYGVSPTKLNDLCFTNVYADSFVIRGDEVRQIAPGQTGKIADYNYKLPDDFTGCVIAWNSNNLDSKVGGNYNYLYRLFRKSNLKPFERDISTEIYQAGSTPCNGVEGFNCYFPLQSYGFQPTNGVGYQPYRVVVLSFELLHAPATVCGPKKSTNLVKNKCVNFNFNGLTGTGVLTESNKKFLPFQQFGRDIADTTDAVRDPQTLEILDITPCSFGGVSVITPGTNTSNQVAVLYQDVNCTEVPVAIHADQLTPTWRVYSTGSNVFQTRAGCLIGAEHVNNSYECDIPIGAGICASYQTQTNSPGSASSVASQSIIAYTMSLGAENSVAYSNNSIAIPTNFTISVTTEILPVSMTKTSVDCTMYICGDSTECSNLLLQYGSFCTQLNRALTGIAVEQDKNTQEVFAQVKQIYKTPPIKDFGGFNFSQILPDPSKPSKRSFIEDLLFNKVTLADAGFIKQYGDCLGDIAARDLICAQKFNGLTVLPPLLTDEMIAQYTSALLAGTITSGWTFGAGAALQIPFAMQMAYRFNGIGVTQNVLYENQKLIANQFNSAIGKIQDSLSSTASALGKLQDVVNQNAQALNELVKQLSSNFGAISSVLNDILSRLDPPEAEVQIDRLITGRLQSLQTYVTQQLIRAAEIRASANLAATKMSECVLGQSKRVDFCGKGYHLMSFPQSAPHGVVFLHVTYVPAQEKNFTTAPAICHDGKAHFPREGVFVSNGTHWFVTQRNFYEPQIITTDNTFVSGNCDVVIGIVNNTVYDPLQPELDSFKEELDKYFKNHTSPDVDLGDISGINASVVNIQKEIDRLNEVAKNLNESLIDLQELGKYEQGGGGTGGGYIPEAPRDGQAYVRKDGEWVLLSTFL